European Patent Application EP 4 137 571 A1, published February 22, 2023. Title: Burden-addicted production strains. Applicant: Danmarks Tekniske Universitet. The sequence listing filed with the application follows.

SEQUENCE LISTING (230 sequences)

SEQ ID NO: 1 - DNA, 2179 bp, E. coli
  gene (1)..(2179): E. coli essential gene folP-glmM
  CDS (1)..(849): folP
atgaaactctttgcccagggtacttcactggaccttagccatcctcacgtaatggggatcctcaacgtcacgcctgattccttttcggatggtggcacgcataactcgctgatagatgcggtgaaacatgcgaatctgatgatcaatgctggcgcgacgatcattgacgttggtggcgagtccacgcgcccaggggcggcggaagttagcgttgaagaagagttgcaacgtgttattcctgtggttgaggcaattgctcaacgcttcgaagtctggatctcggtcgatacatccaaaccagaagtcatccgtgagtcagcgaaagttggcgctcacattattaatgatatccgctccctttccgaacctggcgctctggaggcggctgcagaaaccggtttaccggtttgtctgatgcatatgcagggaaatccaaaaaccatgcaggaagctccgaagtatgacgatgtctttgcagaagtgaatcgctactttattgagcaaatagcacgttgcgagcaggcgggtatcgcaaaagagaaattgttgctcgaccccggattcggtttcggtaaaaatctctcccataactattcattactggcgcgcctggctgaatttcaccatttcaacctgccgctgttggtgggtatgtcacgaaaatcgatgattgggcagctgctgaacgtggggccgtccgagcgcctgagcggtagtctggcctgtgcggtcattgccgcaatgcaaggcgcgcacatcattcgtgttcatgacgtcaaagaaaccgtagaagcgatgcgggtggtggaagccactctgtctgcaaaggaaaacaaacgctatgagtaatcgtaaatatttcggtaccgatgggattcgtggtcgtgtaggggatgcgccgatcacacctgattttgtgcttaagctgggttgggccgcgggtaaagtgctggcgcgccacggctcccgtaagatcattattggtaaagacacgcgtatttctggctatatgctggagtcagcactggaagcgggtctggcggcagcgggcctttccgcactcttcactggcccgatgccaacaccggccgtggcttatctgacgcgtaccttccgcgcagaggccggaattgtgatatctgcatcgcataacccgttctacgataatggcattaaattcttctctatcgacggcaccaaactgccggatgcggtagaagaggccatcgaagcggaaatggaaaaggagatcagctgcgttgattcggcagaactgggtaaagccagccgtatcgttgatgccgcgggtcgctatatcgagttttgcaaagccacgttcccgaacgaacttagcctcagtgaactgaagattgtggtggattgtgcaaacggtgcgacttatcacatcgcgccgaacgtgctgcgcgaactgggggcgaacgttatcgctatcggttgtgagccaaacggtgtaaacatcaatgccgaagtgggggctaccgacgttcgcgcgctccaggctcgtgtgctggctgaaaaagcggatctcggtattgccttcgacggcgatggcgatcgcgtgattatggttgaccatgaaggcaataaagtcgatggcgatcagatcatgtatatcatcgcgcgtgaaggtcttcgtcagggccagctgcgtggtggcgctgtgggtacattgatgagcaacatggggcttgaactggcgctgaaacagttaggaattccatttgcgcgcgcgaaagtgggtgaccgctacgtactggaaaaaatgcaggagaaaggctggcgtatcggtgcagagaattccggtcatgtgatcctgctggataaaactactaccggtgacggcatcgttgctggcttgcaggtgctggcggctatggcacgtaaccatatgagcctgcacgacctttgcagcggcatgaaaatgttcccgcagattctggttaacgtacgttacaccgcaggtagcggcgatccacttgagcatgagtcagttaaagccgtgaccgcagaggttgaagctgcgctgggcaaccgtggacgcgtgttgctgcgtaaatccggcaccgaaccgttaattcgcgtgatggtggaaggcgaagacgaagcgcaggtgactgaatttgcacaccgcatcgccgatgcagtaaaagccgtttaa

SEQ ID NO: 2 - protein, 282 aa, E. coli
MKLFAQGTSLDLSHPHVMGILNVTPDSFSDGGTHNSLIDAVKHANLMINAGATIIDVGGESTRPGAAEVSVEEELQRVIPVVEAIAQRFEVWISVDTSKPEVIRESAKVGAHIINDIRSLSEPGALEAAAETGLPVCLMHMQGNPKTMQEAPKYDDVFAEVNRYFIEQIARCEQAGIAKEKLLLDPGFGFGKNLSHNYSLLARLAEFHHFNLPLLVGMSRKSMIGQLLNVGPSERLSGSLACAVIAAMQGAHIIRVHDVKETVEAMRVVEATLSAKENKRYE

SEQ ID NO: 3 - DNA, 1338 bp, E. coli
  CDS (1)..(1338): E. coli essential gene glmM
atgagtaatcgtaaatatttcggtaccgatgggattcgtggtcgtgtaggggatgcgccgatcacacctgattttgtgcttaagctgggttgggccgcgggtaaagtgctggcgcgccacggctcccgtaagattattattggtaaagacacgcgtatttctggctatatgctggagtcagcactggaagcgggtctggcggcagcgggcctttccgcactcttcactggcccgatgccaacaccggccgtggcttatctgacgcgtaccttccgcgcagaggccggaattgtgatatctgcatcgcataacccgttctacgataatggcattaaattcttctctatcgacggcaccaaactgccggatgcggtagaagaggccatcgaagcggaaatggaaaaggagatcagctgcgttgattcggcagaactgggtaaagccagccgtatcgttgatgccgcgggtcgctatatcgagttttgcaaagccacgttcccgaacgaacttagcctcagtgaactgaagattgtggtggattgtgcaaacggtgcgacttatcacatcgcgccgaacgtgctgcgcgaactgggggcgaacgttatcgctatcggttgtgagccaaacggtgtaaacatcaatgccgaagtgggggctaccgacgttcgcgcgctccaggctcgtgtgctggctgaaaaagcggatctcggtattgccttcgacggcgatggcgatcgcgtgattatggttgaccatgaaggcaataaagtcgatggcgatcagatcatgtatatcatcgcgcgtgaaggtcttcgtcagggccagctgcgtggtggcgctgtgggtacattgatgagcaacatggggcttgaactggcgctgaaacagttaggaattccatttgcgcgcgcgaaagtgggtgaccgctacgtactggaaaaaatgcaggagaaaggctggcgtatcggtgcagagaattccggtcatgtgatcctgctggataaaactactaccggtgacggcatcgttgctggcttgcaggtgctggcggcgatggcacgtaaccatatgagcctgcacgacctttgcagcggcatgaaaatgttcccgcagattctggttaacgtacgttacaccgcaggtagcggcgatccacttgagcatgagtcagttaaagccgtgaccgcagaggttgaagctgcgctgggcaaccgtggacgcgtgttgctgcgtaaatccggcaccgaaccgttaattcgcgtgatggtggaaggcgaagacgaagcgcaggtgactgaatttgcacaccgcatcgccgatgcagtaaaagccgtttaa

SEQ ID NO: 4 - protein, 445 aa, E. coli
MSNRKYFGTDGIRGRVGDAPITPDFVLKLGWAAGKVLARHGSRKIIIGKDTRISGYMLESALEAGLAAAGLSALFTGPMPTPAVAYLTRTFRAEAGIVISASHNPFYDNGIKFFSIDGTKLPDAVEEAIEAEMEKEISCVDSAELGKASRIVDAAGRYIEFCKATFPNELSLSELKIVVDCANGATYHIAPNVLRELGANVIAIGCEPNGVNINAEVGATDVRALQARVLAEKADLGIAFDGDGDRVIMVDHEGNKVDGDQIMYIIAREGLRQGQLRGGAVGTLMSNMGLELALKQLGIPFARAKVGDRYVLEKMQEKGWRIGAENSGHVILLDKTTTGDGIVAGLQVLAAMARNHMSLHDLCSGMKMFPQILVNVRYTAGSGDPLEHESVKAVTAEVEAALGNRGRVLLRKSGTEPLIRVMVEGEDEAQVTEFAHRIADAVKAV

SEQ ID NO: 5 - DNA, 858 bp, E. coli
  CDS (1)..(858): E. coli essential gene murI
atggctaccaaactgcaggacgggaatacaccttgtctggcagctacaccttctgaaccacgtcccaccgtgctggtgtttgactccggcgtcggtgggttgtcggtctatgacgagatccggcatctcttaccggatctccattacatttatgctttcgataacgtcgctttcccgtatggcgaaaaaagcgaagcgtttattgttgagcgagtggtggcaattgtcaccgcggtgcaagaacgttatccccttgcgctggctgtggtcgcttgcaacactgccagtaccgtttcacttcctgcattacgcgaaaagttcgacttcccggttgttggtgtcgtgccggcgattaaacctgctgcacgtctgacggcaaatggcattgtcggattactggcaacccgcggaacagttaaacgttcttatactcatgagctgatcgcgcgtttcgctaatgaatgccagatagaaatgctgggctcggcagagatggttgagttggctgaagcgaagctacatggcgaagatgtttctctggatgcactaaaacgtatcctacgcccgtggttaagaatgaaagagccgccagataccgttgtattgggttgcacccatttccctctactacaagaagaactgttacaagtgctgccagagggaacccggctggtggattctggcgcagcgattgctcgccgaacggcctggttgttagaacatgaagccccggatgcaaaatctgccgatgcgaatattgccttttgtatggcaatgacgccaggagctgaacaattattgcccgttttacagcgttacggcttcgaaacgctcgaaaaactggcagttttaggctga

SEQ ID NO: 6 - protein, 285 aa, E. coli
MATKLQDGNTPCLAATPSEPRPTVLVFDSGVGGLSVYDEIRHLLPDLHYIYAFDNVAFPYGEKSEAFIVERVVAIVTAVQERYPLALAVVACNTASTVSLPALREKFDFPVVGVVPAIKPAARLTANGIVGLLATRGTVKRSYTHELIARFANECQIEMLGSAEMVELAEAKLHGEDVSLDALKRILRPWLRMKEPPDTVVLGCTHFPLLQEELLQVLPEGTRLVDSGAAIARRTAWLLEHEAPDAKSADANIAFCMAMTPGAEQLLPVLQRYGFETLEKLAVLG

SEQ ID NO: 7 - DNA, 1104 bp, E. coli
  CDS (1)..(1104): E. coli essential gene asd
atgaaaaatgttggttttatcggctggcgcggtatggtcggctccgttctcatgcaacgcatggttgaagagcgcgacttcgacgccattcgccctgtctacttttctacttctcagcttggtcaggctgcgccgtcttttggcggaaccactggcacacttcaggatgcctttgatctggaggcgctaaaggccctcgatatcattgtgacctgtcagggcggcgattataccaacgaaatctatccaaagcttcgtgaaagcggatggcagggttactggattgacgcagcatcgtctctgcgcatgaaagatgacgccatcatcattcttgaccccgtcaatcaggacgtcattaccgacggattaaataatggcatcaggacttttgttggcggtaactgtaccgtaagcctgatgttgatgtcgttgggtggtttattcgccaatgatcttgttgattgggtgtccgttgcaacctaccaggccgcttccggcggtggtgcgcgacatatgcgtgagttattaacccagatgggccatctgtatggccatgtagcagatgaactcgcgaccccgtcctctgctattctcgatatcgaacgcaaagtcacaaccttaacccgtagcggtgagctgccggtggataactttggcgtgccgctggcgggtagcctgattccgtggatcgacaaacagctcgataacggtcagagccgcgaagagtggaaagggcaggcggaaaccaacaagatcctcaacacatcttccgtaattccggtagatggtttatgtgtgcgtgtcggggcattgcgctgccacagccaggcattcactattaaattgaaaaaagatgtgtcgattccgaccgtggaagaactgctggctgcgcacaatccgtgggcgaaagtcgttccgaacgatcgggaaatcactatgcgtgagctaaccccagctgccgttaccggcacgctgaccacgccggtaggccgcctgcgtaagctgaatatgggaccagagttcctgtcagcctttaccgtgggcgaccagctgctgtggggggccgcggagccgctgcgtcggatgcttcgtcaactggcgtaa

SEQ ID NO: 8 - protein, 367 aa, E. coli
MKNVGFIGWRGMVGSVLMQRMVEERDFDAIRPVYFSTSQLGQAAPSFGGTTGTLQDAFDLEALKALDIIVTCQGGDYTNEIYPKLRESGWQGYWIDAASSLRMKDDAIIILDPVNQDVITDGLNNGIRTFVGGNCTVSLMLMSLGGLFANDLVDWVSVATYQAASGGGARHMRELLTQMGHLYGHVADELATPSSAILDIERKVTTLTRSGELPVDNFGVPLAGSLIPWIDKQLDNGQSREEWKGQAETNKILNTSSVIPVDGLCVRVGALRCHSQAFTIKLKKDVSIPTVEELLAAHNPWAKVVPNDREITMRELTPAAVTGTLTTPVGRLRKLNMGPEFLSAFTVGDQLLWGAAEPLRRMLRQLA

SEQ ID NO: 9 - DNA, 1104 bp, E. coli; identical to SEQ ID NO: 7
  CDS (1)..(1104): E. coli essential gene thyA

SEQ ID NO: 10 - protein, 367 aa, E. coli; identical to SEQ ID NO: 8

SEQ ID NO: 11 - DNA, 1842 bp, E. coli
  CDS (1)..(1842): E. coli essential gene rpoD
atggagcaaaacccgcagtcacagctgaaacttcttgtcacccgtggtaaggagcaaggctatctgacctatgccgaggtcaatgaccatctgccggaagatatcgtcgattcagatcagatcgaagacatcatccaaatgatcaacgacatgggcattcaggtgatggaagaagcaccggatgccgatgatctgatgctggctgaaaacaccgcggacgaagatgctgccgaagccgccgcgcaggtgctttccagcgtggaatctgaaatcgggcgcacgactgacccggtacgcatgtacatgcgtgaaatgggcaccgttgaactgttgacccgcgaaggcgaaattgacatcgctaagcgtattgaagacgggatcaaccaggttcaatgctccgttgctgaatatccggaagcgatcacctatctgctggaacagtacgatcgtgttgaagcagaagaagcgcgtctgtccgatctgatcaccggctttgttgacccgaacgcagaagaagatctggcacctaccgccactcacgtcggttctgagctttcccaggaagatctggacgatgacgaagatgaagacgaagaagatggcgatgacgacagcgccgatgatgacaacagcatcgacccggaactggctcgcgaaaaatttgcggaactacgcgctcagtacgttgtaacgcgtgacaccatcaaagcgaaaggtcgcagtcacgctaccgctcaggaagagatcctgaaactgtctgaagtattcaaacagttccgcctggtgccgaagcagtttgactacctggtcaacagcatgcgcgtcatgatggaccgcgttcgtacgcaagaacgtctgatcatgaagctctgcgttgagcagtgcaaaatgccgaagaaaaacttcattaccctgtttaccggcaacgaaaccagcgatacctggttcaacgcggcaattgcgatgaacaagccgtggtcggaaaaactgcacgatgtctctgaagaagtgcatcgcgccctgcaaaaactgcagcagattgaagaagaaaccggcctgaccatcgagcaggttaaagatatcaaccgtcgtatgtccatcggtgaagcgaaagcccgccgtgcgaagaaagagatggttgaagcgaacttacgtctggttatttctatcgctaagaaatacaccaaccgtggcttgcagttccttgacctgattcaggaaggcaacatcggtctgatgaaagcggttgataaattcgaataccgccgtggttacaagttctccacctacgcaacctggtggatccgtcaggcgatcacccgctctatcgcggatcaggcgcgcaccatccgtattccggtgcatatgattgagaccatcaacaagctcaaccgtatttctcgccagatgctgcaagagatgggccgtgaaccgacgccggaagaactggctgaacgtatgctgatgccggaagacaagatccgcaaagtgctgaagatcgccaaagagccaatctccatggaaacgccgatcggtgatgatgaagattcgcatctgggggatttcatcgaggataccaccctcgagctgccgctggattctgcgaccaccgaaagcctgcgtgcggcaacgcacgacgtgctggctggcctgaccgcgcgtgaagcaaaagttctgcgtatgcgtttcggtatcgatatgaacaccgaccacacgctggaagaagtgggtaaacagttcgacgttacccgcgaacgtatccgtcagatcgaagcgaaggcgctgcgcaaactgcgtcacccgagccgttctgaagtgctgcgtagcttcctggacgattaa

SEQ ID NO: 12 - protein, 613 aa, E. coli
MEQNPQSQLKLLVTRGKEQGYLTYAEVNDHLPEDIVDSDQIEDIIQMINDMGIQVMEEAPDADDLMLAENTADEDAAEAAAQVLSSVESEIGRTTDPVRMYMREMGTVELLTREGEIDIAKRIEDGINQVQCSVAEYPEAITYLLEQYDRVEAEEARLSDLITGFVDPNAEEDLAPTATHVGSELSQEDLDDDEDEDEEDGDDDSADDDNSIDPELAREKFAELRAQYVVTRDTIKAKGRSHATAQEEILKLSEVFKQFRLVPKQFDYLVNSMRVMMDRVRTQERLIMKLCVEQCKMPKKNFITLFTGNETSDTWFNAAIAMNKPWSEKLHDVSEEVHRALQKLQQIEEETGLTIEQVKDINRRMSIGEAKARRAKKEMVEANLRLVISIAKKYTNRGLQFLDLIQEGNIGLMKAVDKFEYRRGYKFSTYATWWIRQAITRSIADQARTIRIPVHMIETINKLNRISRQMLQEMGREPTPEELAERMLMPEDKIRKVLKIAKEPISMETPIGDDEDSHLGDFIEDTTLELPLDSATTESLRAATHDVLAGLTAREAKVLRMRFGIDMNTDHTLEEVGKQFDVTRERIRQIEAKALRKLRHPSRSEVLRSFLDD

SEQ ID NO: 13 - DNA, 546 bp, E. coli
  CDS (1)..(546): E. coli essential gene nusG
atgtctgaagctcctaaaaagcgctggtacgtcgttcaggcgttttccggttttgaaggccgcgtagcaacgtcgctgcgtgagcatatcaaattacacaacatggaagatttgtttggtgaagtcatggtaccaaccgaagaagtggttgaaatccgtggcggtcagcgtcgcaaaagcgaacgtaaattcttccctggctacgtcctcgttcagatggtgatgaacgacgcgagctggcacctggtgcgcagcgtaccgcgtgtgatgggcttcatcggcggtacttccgatcgtcctgcgccaatcagcgataaagaagtcgatgcgattatgaaccgcctgcagcaggttggtgataagccgcgtccgaaaacgctgtttgaaccgggtgaaatggtccgtgttaatgatggtccgttcgctgacttcaacggtgttgttgaagaagtggattacgagaaatctcgtctgaaagtgtctgtttctatcttcggtcgtgcgaccccggtagagctggacttcagccaggttgaaaaagcctaa

SEQ ID NO: 14 - protein, 181 aa, E. coli
MSEAPKKRWYVVQAFSGFEGRVATSLREHIKLHNMEDLFGEVMVPTEEVVEIRGGQRRKSERKFFPGYVLVQMVMNDASWHLVRSVPRVMGFIGGTSDRPAPISDKEVDAIMNRLQQVGDKPRPKTLFEPGEMVRVNDGPFADFNGVVEEVDYEKSRLKVSVSIFGRATPVELDFSQVEKA

SEQ ID NO: 15 - DNA, 216 bp, E. coli
  CDS (1)..(216): E. coli essential gene rpsU
atgccggtaattaaagtacgtgaaaacgagccgttcgacgtagctctgcgtcgcttcaagcgttcctgcgaaaaagcaggtgttctggcggaagttcgtcgtcgtgagttctatgaaaaaccgactaccgaacgtaagcgcgctaaagcttctgcagtgaaacgtcacgcgaagaaactggctcgcgaaaacgcacgccgcactcgtctgtactaa

SEQ ID NO: 16 - protein, 71 aa, E. coli
MPVIKVRENEPFDVALRRFKRSCEKAGVLAEVRRREFYEKPTTERKRAKASAVKRHAKKLARENARRTRLY

SEQ ID NO: 17 - DNA, 216 bp, E. coli; identical to SEQ ID NO: 15
  CDS (1)..(216): E. coli essential gene accD

SEQ ID NO: 18 - protein, 71 aa, E. coli; identical to SEQ ID NO: 16

SEQ ID NO: 19 - DNA, 216 bp, E. coli; identical to SEQ ID NO: 15
  CDS (1)..(216): E coli essential gene degS

SEQ ID NO: 20 - protein, 71 aa, E. coli; identical to SEQ ID NO: 16

SEQ ID NO: 21 - DNA, 531 bp, E. coli
  CDS (1)..(531): E. coli essential gene fldA
atggctatcactggcatctttttcggcagcgacaccggtaataccgaaaatatcgcaaaaatgattcaaaaacagcttggtaaagacgttgccgatgtccatgacattgcaaaaagcagcaaagaagatctggaagcttatgacattctgctgctgggcatcccaacctggtattacggcgaagcgcagtgtgactgggatgacttcttcccgactctcgaagagattgatttcaatggcaaactggttgcgctgtttggttgtggtgaccaggaagattacgccgaatatttctgcgacgcattgggcaccatccgcgacatcattgaaccgcgcggtgcaaccatcgttggtcactggccaactgcgggctatcatttcgaagcatcaaaaggtctggcagatgacgaccactttgtcggtctggctatcgacgaagaccgtcagccggaactgaccgctgaacgtgtagaaaaatgggttaaacagatttctgaagagttgcatctcgacgaaattctcaatgcctga

SEQ ID NO: 22 - protein, 176 aa, E. coli
MAITGIFFGSDTGNTENIAKMIQKQLGKDVADVHDIAKSSKEDLEAYDILLLGIPTWYYGEAQCDWDDFFPTLEEIDFNGKLVALFGCGDQEDYAEYFCDALGTIRDIIEPRGATIVGHWPTAGYHFEASKGLADDDHFVGLAIDEDRQPELTAERVEKWVKQISEELHLDEILNA

SEQ ID NO: 23 - DNA, 960 bp, E. coli
  CDS (1)..(960): E. coli essential gene ftsN
gtggcacaacgagattatgtacgccgcagccaaccggcaccttcgcggcgaaaaaagagcacctcacggaaaaagcaacgaaatctgcctgcggtttctcccgctatggtcgctattgctgccgccgttcttgtgacctttatcggtggtctgtacttcattacgcatcacaagaaagaagagtccgagacgctgcaaagccagaaagtgaccggaaacggactaccaccaaaaccagaagaacgctggcgctacattaaagagctggaaagtcgccagccgggagtgcgtgcgcccacagaaccttctgccggtggtgaagtgaaaacgccggagcaactgacaccagaacaacgtcagcttcttgaacaaatgcaggctgatatgcgccagcagccaacgcagctggttgaagttccgtggaatgaacagacgccggaacagcgtcagcaaacgctacagcgccaacgtcaggcgcagcaattagcggaacagcaacgcctggctcagcagtcgcgtacgactgaacaaagctggcagcagcagacgcgtacgtcgcaagccgcaccggtacaggcgcaaccgcgccagtctaaaccggcttcttctcagcagccgtaccaggatctgctgcaaactcctgcgcacacgactgcgcagtcgaagccgcagcaagctgcgccagttgctcgtgccgctgacgcgccaaaaccgacggcggagaaaaaagacgaacgccgctggatggtgcagtgcggttcgttcagaggcgcggaacaggcagagacggtacgtgctcagctggcgttcgaaggctttgactcgaaaatcaccaccaacaatggctggaatcgtgtggtcattggcccggtgaaaggcaaagagaacgcagacagcaccctcaatcggttgaagatggcgggccatacaaactgcattcggctcgccgccgggggttga

SEQ ID NO: 24 - protein, 319 aa, E. coli
VAQRDYVRRSQPAPSRRKKSTSRKKQRNLPAVSPAMVAIAAAVLVTFIGGLYFITHHKKEESETLQSQKVTGNGLPPKPEERWRYIKELESRQPGVRAPTEPSAGGEVKTPEQLTPEQRQLLEQMQADMRQQPTQLVEVPWNEQTPEQRQQTLQRQRQAQQLAEQQRLAQQSRTTEQSWQQQTRTSQAAPVQAQPRQSKPASSQQPYQDLLQTPAHTTAQSKPQQAAPVARAADAPKPTAEKKDERRWMVQCGSFRGAEQAETVRAQLAFEGFDSKITTNNGWNRVVIGPVKGKENADSTLNRLKMAGHTNCIRLAAGG

SEQ ID NO: 25 - DNA, 1935 bp, E. coli
  CDS (1)..(1935): E. coli essential gene hflB
atggcgaaaaacctaatactctggctggtcattgccgttgtgctgatgtcagtattccagagctttgggcccagcgagtctaatggccgtaaggtggattactctaccttcctacaagaggtcaataacgaccaggttcgtgaagcgcgtatcaacggacgtgaaatcaacgttaccaagaaagatagtaaccgttataccacttacattccggttcaggatccgaaattactggataacctgttgaccaagaacgtcaaggttgtcggtgaaccgcctgaagaaccaagcctgctggcttctatcttcatctcctggttcccgatgctgttgctgattggtgtctggatcttcttcatgcgtcaaatgcagggcggcggtggcaaaggtgccatgtcgtttggtaagagcaaagcgcgcatgctgacggaagatcagatcaaaacgacctttgctgacgttgcgggctgcgacgaagcaaaagaagaagttgctgaactggttgagtatctgcgcgagccgagccgcttccagaaactcggcggtaagatcccgaaaggcgtcttgatggtcggtcctccgggtaccggtaaaacgctgctggcgaaagcgattgcaggcgaagcgaaagttccgttctttactatctccggttctgacttcgtagaaatgttcgtcggtgtgggtgcatcccgtgttcgtgacatgttcgaacaggcgaagaaagcggcaccgtgcatcatctttatcgatgaaatcgacgccgtaggccgccagcgtggcgctggtctgggcggtggtcacgatgaacgtgaacagactctgaaccagatgctggttgagatggatggcttcgaaggtaacgaaggtatcatcgttatcgccgcgactaaccgtccggacgttctcgacccggccctgctgcgtcctggccgtttcgaccgtcaggttgtggtcggcttgccagatgttcgcggtcgtgagcagatcctgaaagttcacatgcgtcgcgtaccattggcacccgatatcgacgcggcaatcattgcccgtggtactcctggtttctccggtgctgacctggcgaacctggtgaacgaagcggcactgttcgctgctcgtggcaacaaacgcgttgtgtcgatggttgagttcgagaaagcgaaagacaaaatcatgatgggtgcggaacgtcgctccatggtgatgacggaagcgcagaaagaatcgacggcttaccacgaagcgggtcatgcgattatcggtcgcctggtgccggaacacgatccggtgcacaaagtgacgattatcccacgcggtcgtgcgctgggtgtgactttcttcttgcctgagggcgacgcaatcagcgccagccgtcagaaactggaaagccagatttctacgctgtacggtggtcgtctggcagaagagatcatctacgggccggaacatgtatctaccggtgcgtccaacgatattaaagttgcgaccaacctggcacgtaacatggtgactcagtggggcttctctgagaaattgggtccactgctgtacgcggaagaagaaggtgaagtgttcctcggccgtagcgtagcgaaagcgaaacatatgtccgatgaaactgcacgtatcatcgaccaggaagtgaaagcactgattgagcgtaactataatcgtgcgcgtcagcttctgaccgacaatatggatattctgcatgcgatgaaagatgctctcatgaaatatgagactatcgacgcaccgcagattgatgacctgatggcacgtcgcgatgtacgtccgccagcgggctgggaagaaccaggcgcttctaacaattctggcgacaatggtagtccaaaggctcctcgtccggttgatgaaccgcgtacgccgaacccgggtaacaccatgtcagagcagttaggcgacaagtaa

SEQ ID NO: 26 - protein, 644 aa, E. coli
MAKNLILWLVIAVVLMSVFQSFGPSESNGRKVDYSTFLQEVNNDQVREARINGREINVTKKDSNRYTTYIPVQDPKLLDNLLTKNVKVVGEPPEEPSLLASIFISWFPMLLLIGVWIFFMRQMQGGGGKGAMSFGKSKARMLTEDQIKTTFADVAGCDEAKEEVAELVEYLREPSRFQKLGGKIPKGVLMVGPPGTGKTLLAKAIAGEAKVPFFTISGSDFVEMFVGVGASRVRDMFEQAKKAAPCIIFIDEIDAVGRQRGAGLGGGHDEREQTLNQMLVEMDGFEGNEGIIVIAATNRPDVLDPALLRPGRFDRQVVVGLPDVRGREQILKVHMRRVPLAPDIDAAIIARGTPGFSGADLANLVNEAALFAARGNKRVVSMVEFEKAKDKIMMGAERRSMVMTEAQKESTAYHEAGHAIIGRLVPEHDPVHKVTIIPRGRALGVTFFLPEGDAISASRQKLESQISTLYGGRLAEEIIYGPEHVSTGASNDIKVATNLARNMVTQWGFSEKLGPLLYAEEEGEVFLGRSVAKAKHMSDETARIIDQEVKALIERNYNRARQLLTDNMDILHAMKDALMKYETIDAPQIDDLMARRDVRPPAGWEEPGASNNSGDNGSPKAPRPVDEPRTPNPGNTMSEQLGDK

SEQ ID NO: 27 - DNA, 612 bp, E. coli
  CDS (1)..(612): E. coli essential gene lolA
atgaaaaaaattgccatcacctgtgcattactctcaagcttagtagcaagcagcgtttgggctgatgccgcaagcgatctgaaaagccgcctggataaagtcagcagcttccacgccagcttcacacaaaaagtgactgacggtagcggcgcggcggtgcaggaaggtcagggcgatctgtgggtgaaacgtccaaacttattcaactggcatatgacacaacctgatgaaagcattctggtttctgacggtaaaacactgtggttctataacccgttcgttgagcaagctacggcaacctggctgaaagatgccaccggtaatacgccgtttatgctgattgcccgcaaccagtccagcgactggcagcagtacaatatcaaacagaatggcgatgactttgtcctgacgccgaaagccagcaatggcaatctgaagcagttcaccattaacgtgggacgtgatggcacaatccatcagtttagcgcggtggagcaggacgatcagcgcagcagttatcaactgaaatcccagcaaaatggggctgtggatgcagcgaaatttaccttcaccccgccgcaaggcgtcacggtagatgatcaacgtaagtag

SEQ ID NO: 28 - protein, 203 aa, E. coli
MKKIAITCALLSSLVASSVWADAASDLKSRLDKVSSFHASFTQKVTDGSGAAVQEGQGDLWVKRPNLFNWHMTQPDESILVSDGKTLWFYNPFVEQATATWLKDATGNTPFMLIARNQSSDWQQYNIKQNGDDFVLTPKASNGNLKQFTINVGRDGTIHQFSAVEQDDQRSSYQLKSQQNGAVDAAKFTFTPPQGVTVDDQRK

SEQ ID NO: 29 - DNA, 1083 bp, E. coli
  CDS (1)..(1083): E. coli essential gene mraY
atgttagtttggctggccgaacatttggtcaaatattattccggctttaacgtcttttcctatctgacgtttcgcgccatcgtcagcctgctgaccgcgctgttcatctcattgtggatgggcccgcgtatgattgctcatttgcaaaaactttcctttggtcaggtggtgcgtaacgacggtcctgaatcacacttcagcaagcgcggtacgccgaccatgggcgggattatgatcctgacggcgattgtgatctccgtactgctgtgggcttacccgtccaatccgtacgtctggtgcgtgttggtggtgctggtaggttacggtgttattggctttgttgatgattatcgcaaagtggtgcgtaaagacaccaaagggttgatcgctcgttggaagtatttctggatgtcggtcattgcgctgggtgtcgccttcgccctgtaccttgccggcaaagacacgcccgcaacgcagctggtggtcccattctttaaagatgtgatgccgcagctggggctgttctacattctgctggcttacttcgtcattgtgggtactggcaacgcggtaaacctgaccgatggtctcgacggcctggcaattatgccgaccgtatttgtcgccggtggttttgcgctggtggcgtgggcgaccggcaatatgaactttgccagctacttgcatataccgtatctgcgacacgccggggaactggttattgtctgtaccgcgatagtcggggcaggactgggcttcctgtggtttaacacctatccggcgcaggtctttatgggcgatgtaggttcgctggcgttaggtggtgcgttaggcattatcgccgtactgctacgtcaggaattcctgctggtgattatggggggcgtgttcgtggtagaaacgctttctgtcatcctgcaggtcggctcctttaaactgcgcggacaacgtattttccgcatggcaccgattcatcaccactatgaactgaaaggctggccggaaccgcgcgtcattgtgcgtttctggattatttcgctgatgctggttctgattggtctggcaacgctgaaggtacgttaa

SEQ ID NO: 30 - protein, 360 aa, E. coli
MLVWLAEHLVKYYSGFNVFSYLTFRAIVSLLTALFISLWMGPRMIAHLQKLSFGQVVRNDGPESHFSKRGTPTMGGIMILTAIVISVLLWAYPSNPYVWCVLVVLVGYGVIGFVDDYRKVVRKDTKGLIARWKYFWMSVIALGVAFALYLAGKDTPATQLVVPFFKDVMPQLGLFYILLAYFVIVGTGNAVNLTDGLDGLAIMPTVFVAGGFALVAWATGNMNFASYLHIPYLRHAGELVIVCTAIVGAGLGFLWFNTYPAQVFMGDVGSLALGGALGIIAVLLRQEFLLVIMGGVFVVETLSVILQVGSFKLRGQRIFRMAPIHHHYELKGWPEPRVIVRFWIISLMLVLIGLATLKVR

SEQ ID NO: 31 - DNA, 489 bp, E. coli
  CDS (1)..(489): E. coli essential gene mreD
gtggcgagctatcgtagccagggacgctgggtaatctggctctctttcctcattgcgctgttgctgcaaatcatgccctggccggataacctgattgttttccggccaaactgggtgttactcatcttgttgtattggatcctggccttgcctcatcgcgtaaatgtgggcacaggttttgtgatgggtgccatactggatctgatcagcggctcgacgcttggcgtacgcgtattggcgatgagcatcattgcttacctggtggcgctgaaataccagcttttccgcaacctcgcattatggcagcaggcgctggtcgtcatgttgctttcgctggtggtggatattattgttttctgggcagagtttttagtgattaacgtctctttcagaccggaagtgttctggagtagtgtagtcaatggggtgctctggccgtggattttcttgctgatgcgcaaagtccgtcagcagtttgcagtgcaataa

SEQ ID NO: 32 - protein, 162 aa, E. coli
VASYRSQGRWVIWLSFLIALLLQIMPWPDNLIVFRPNWVLLILLYWILALPHRVNVGTGFVMGAILDLISGSTLGVRVLAMSIIAYLVALKYQLFRNLALWQQALVVMLLSLVVDIIVFWAEFLVINVSFRPEVFWSSVVNGVLWPWIFLLMRKVRQQFAVQ

SEQ ID NO: 33 - DNA, 1260 bp, E. coli
  CDS (1)..(1260): E. coli essential gene murA
atggataaatttcgtgttcaggggccaacgaagctccagggcgaagtcacaatttccggcgctaaaaatgctgctctgcctatcctttttgccgctctactggcggaagaaccggtagagatccagaacgtcccgaaactgaaagacgtcgatacatcaatgaagctgctaagccagctgggtgcgaaagtagaacgtaatggttctgtgcatattgatgcccgcgacgttaatgtattctgcgcaccttacgatctggttaaaaccatgcgtgcttctatctgggcactggggccgctggtagcgcgctttggtcaggggcaagtttcactacctggcggttgtacgatcggtgcgcgtccggttgatctacacatttctggcctcgaacaattaggcgcgaccatcaaactggaagaaggttacgttaaagcttccgtcgatggtcgtctgaaaggcgcacatatcgtgatggataaagtcagcgttggcgcaacggtgaccatcatgtgtgctgcaaccctggcggaaggcaccacgattattgaaaacgcagcgcgtgaaccggaaatcgtcgataccgcgaacttcctgattacgctgggtgcgaaaattagcggtcagggcaccgatcgtatcgtcatcgaaggtgtggaacgtttaggcggcggtgtctatcgcgtgctgccggatcgtatcgaaaccggtacattcctggtggcggcggcgatttctcgcggcaaaattatctgccgtaacgcgcagccagatactctcgacgccgtgctggcgaaactgcgtgacgctggagcggacatcgaagtcggcgaagactggattagcctggatatgcatggcaaacgtccgaaggctgttaacgtacgtaccgcgccgcatccggcattcccgaccgatatgcaggcccagttcacgctgttgaacctggtggcagaagggactggattcatcaccgaaacggtctttgaaaaccgctttatgcatgtgccagagctgagccgtatgggcgcgcacgccgaaatcgaaagcaataccgttatttgtcacggtgttgaaaaactttctggcgcacaggttatggcaaccgatctgcgtgcatcagcaagcctggtgctggctggctgtattgcggaagggacgacggtggttgatcgtatttatcacatcgatcgtggctacgaacgcattgaagacaaactgcgcgctttaggtgcaaatattgagcgtgtgaaaggcgagtaa

SEQ ID NO: 34 - protein, 419 aa, E. coli
MDKFRVQGPTKLQGEVTISGAKNAALPILFAALLAEEPVEIQNVPKLKDVDTSMKLLSQLGAKVERNGSVHIDARDVNVFCAPYDLVKTMRASIWALGPLVARFGQGQVSLPGGCTIGARPVDLHISGLEQLGATIKLEEGYVKASVDGRLKGAHIVMDKVSVGATVTIMCAATLAEGTTIIENAAREPEIVDTANFLITLGAKISGQGTDRIVIEGVERLGGGVYRVLPDRIETGTFLVAAAISRGKIICRNAQPDTLDAVLAKLRDAGADIEVGEDWISLDMHGKRPKAVNVRTAPHPAFPTDMQAQFTLLNLVAEGTGFITETVFENRFMHVPELSRMGAHAEIESNTVICHGVEKLSGAQVMATDLRASASLVLAGCIAEGTTVVDRIYHIDRGYERIEDKLRALGANIERVKGE

SEQ ID NO: 35 - DNA, 1029 bp, E. coli
  CDS (1)..(1029): E. coli essential gene murB
atgaaccactccttaaaaccctggaacacatttggcattgatcataatgctcagcacattgtatgtgccgaagacgaacaacaattactcaatgcctggcagcatgcaaccgcagaaggacaacccgttcttattctgggtgaaggaagtaatgtactttttctggaagactatcgcggcacggtgatcatcaaccggatcaaaggtatcgaaattcatgatgaacctgatgcgtggtatttacatgtaggagccggagaaaactggcatcgcctggtaaaatacactttgcaggaaggtatgcctggtctggaaaatctggcattaattcctggttgtgtcggctcatcacctatccagaatattggtgcttatggcgtagaattacagcgagtttgcgcttatgttgattgtgttgaactggcgacaggcaagcaagtgcgcttaactgccaaagagtgccgttttggctatcgcgacagtatttttaaacatgaataccaggatcgcttcgccattgtagccgtaggtctgcgtctgccaaaagagtggcaacctgtactaacgtatggtgacttaactcgtctggatcctacaacagtaacgccacagcaagtatttaatgcggtgtgtcatatgcgcaccaccaaactccctgatccaaaagtgaatggcaatgccggtagtttcttcaaaaaccctgttgtatctgccgaaacggctgaagcattactgtcacaatttccaacagcaccaaattacccccaggcggatggttcagtaaaactggcagcaggttggcttattgatcagtgccagctaaaagggatgcaaatgggtggggctgcggtgcaccgtcaacaggcgttagttctcattaatgaagacaatgcaaaaagcgaagatgtggtgcaactggcacaccatgtaagacaaaaagtgggtgaaaaatttaatgtctggcttgagcctgaagtccgctttattggtgcatcaggtgaagtgagcgcagtggagacaatttcatga

SEQ ID NO: 36 - protein, 342 aa, E. coli
MNHSLKPWNTFGIDHNAQHIVCAEDEQQLLNAWQHATAEGQPVLILGEGSNVLFLEDYRGTVIINRIKGIEIHDEPDAWYLHVGAGENWHRLVKYTLQEGMPGLENLALIPGCVGSSPIQNIGAYGVELQRVCAYVDCVELATGKQVRLTAKECRFGYRDSIFKHEYQDRFAIVAVGLRLPKEWQPVLTYGDLTRLDPTTVTPQQVFNAVCHMRTTKLPDPKVNGNAGSFFKNPVVSAETAEALLSQFPTAPNYPQADGSVKLAAGWLIDQCQLKGMQMGGAAVHRQQALVLINEDNAKSEDVVQLAHHVRQKVGEKFNVWLEPEVRFIGASGEVSAVETIS

SEQ ID NO: 37 - DNA, 1359 bp, E. coli
  CDS (1)..(1359): E. coli essential gene murF
atgattagcgtaacccttagccaacttaccgacattctcaacggtgaactgcaaggtgcagatatcacccttgatgctgtaaccactgatacccgaaaactgacgccgggctgcctgtttgttgccctgaaaggcgaacgttttgatgcccacgattttgccgaccaggcgaaagctggcggcgcaggcgcactactggttagccgtccgctggacatcgacctgccgcagttaatcgtcaaggatacgcgtctggcgtttggtgaactggctgcatgggttcgccagcaagttccggcgcgcgtggttgctctgacggggtcctccggcaaaacctccgttaaagagatgacggcggcgattttaagccagtgcggcaacacgctttatacggcaggcaatctcaacaacgacatcggtgtaccgatgacgctgttgcgcttaacgccggaatacgattacgcagttattgaacttggcgcgaaccatcagggcgaaatagcctggactgtgagtctgactcgcccggaagctgcgctggtcaacaacctggcagcggcgcatctggaaggttttggctcgcttgcgggtgtcgcgaaagcgaaaggtgaaatctttagcggcctgccggaaaacggtatcgccattatgaacgccgacaacaacgactggctgaactggcagagcgtaattggctcacgcaaagtgtggcgtttctcacccaatgccgccaacagcgatttcaccgccaccaatatccatgtgacctcgcacggtacggaatttaccctacaaaccccaaccggtagcgtcgatgttctgctgccgttgccggggcgtcacaatattgcgaatgcgctggcagccgctgcgctctccatgtccgtgggcgcaacgcttgatgctatcaaagcggggctggcaaatctgaaagctgttccaggccgtctgttccccatccaactggcagaaaaccagttgctgctcgacgactcctacaacgccaatgtcggttcaatgactgcagcagtccaggtactggctgaaatgccgggctaccgcgtgctggtggtgggcgatatggcggaactgggcgctgaaagcgaagcctgccatgtacaggtgggcgaggcggcaaaagctgctggtattgaccgcgtgttaagcgtgggtaaacaaagccatgctatcagcaccgccagcggcgttggcgaacattttgctgataaaactgcgttaattacgcgtcttaaatcactgattgctgagcaacaggtaattacgattttagttaagggttcacgtagtgccgccatggaagaggtagtacgcgctttacaggagaatgggacatgttag

SEQ ID NO: 38 - protein, 452 aa, E. coli
MISVTLSQLTDILNGELQGADITLDAVTTDTRKLTPGCLFVALKGERFDAHDFADQAKAGGAGALLVSRPLDIDLPQLIVKDTRLAFGELAAWVRQQVPARVVALTGSSGKTSVKEMTAAILSQCGNTLYTAGNLNNDIGVPMTLLRLTPEYDYAVIELGANHQGEIAWTVSLTRPEAALVNNLAAAHLEGFGSLAGVAKAKGEIFSGLPENGIAIMNADNNDWLNWQSVIGSRKVWRFSPNAANSDFTATNIHVTSHGTEFTLQTPTGSVDVLLPLPGRHNIANALAAAALSMSVGATLDAIKAGLANLKAVPGRLFPIQLAENQLLLDDSYNANVGSMTAAVQVLAEMPGYRVLVVGDMAELGAESEACHVQVGEAAKAAGIDRVLSVGKQSHAISTASGVGEHFADKTALITRLKSLIAEQQVITILVKGSRSAAMEEVVRALQENGTC

SEQ ID NO: 39 - DNA, 642 bp, E. coli
  CDS (1)..(642): E. coli essential gene nadD
atgaaatctttacaggctctgtttggcggcacctttgatccggtgcactatggtcatctaaaacccgtggaaacgctggcgaatttgattggtctgacgcgggtcacaatcatccctaataatgttcctccgcatcgtccccagccggaagcgaacagcgtgcagcgtaaacacatgcttgaactggcgattgccgacaagccattatttactcttgatgaacgcgagctaaagcgcaatgccccctcttacactgcgcaaacactgaaagagtggcggcaggaacaaggaccggacgtgccgctggcgtttattattggtcaggattcattgctgacctttccgacctggtacgaatacgaaacgatactcgacaatgcacatttgatcgtctgtcggcgtccaggttacccacttgaaatggcgcaaccgcaataccagcaatggctggaagatcatttgacacataacccggaagatcttcaccttcagcctgccggtaaaatttatctggctgaaacgccgtggtttaacatctcggcgaccatcatccgcgaacgtttgcaaaacggtgaatcgtgtgaggatttattgccggaaccggtattgacttacattaaccaacaaggcttgtatcgctga

SEQ ID NO: 40 - protein, 213 aa, E. coli
MKSLQALFGGTFDPVHYGHLKPVETLANLIGLTRVTIIPNNVPPHRPQPEANSVQRKHMLELAIADKPLFTLDERELKRNAPSYTAQTLKEWRQEQGPDVPLAFIIGQDSLLTFPTWYEYETILDNAHLIVCRRPGYPLEMAQPQYQQWLEDHLTHNPEDLHLQPAGKIYLAETPWFNISATIIRERLQNGESCEDLLPEPVLTYINQQGLYR

SEQ ID NO: 41 - DNA, 333 bp, E. coli
  CDS (1)..(333): E. coli essential gene rplV
atggaaactatcgctaaacatcgccatgctcgttcttctgctcagaaggttcgccttgttgctgacctgattcgcggtaagaaagtgtcgcaggctctggatattttgacctacaccaacaagaaagcggctgtactggtcaagaaagttctggaatctgccattgctaacgctgaacacaacgatggcgctgacattgacgatctgaaagttacgaaaattttcgtagacgaaggcccgagcatgaagcgcattatgccgcgtgcaaaaggtcgtgcagatcgcatcctgaagcgcaccagccacatcactgtggttgtgtccgatcgctga

SEQ ID NO: 42 - protein, 110 aa, E. coli [sequence omitted]

SEQ ID NO: 43 - DNA, 471 bp, E. coli
  CDS (1)..(471): E. coli essential gene rpsG
atgccacgtcgtcgcgtcattggtcagcgtaaaattctgccggatccgaagttcggatcagaactgctggctaaatttgtaaatatcctgatggtagatggtaaaaaatctactgctgaatctatcgtatacagcgcgctggagaccctggctcagcgctctggtaaatctgaactggaagcattcgaagtagctctcgaaaacgtgcgcccgactgtagaagttaagtctcgccgcgttggtggttctacttatcaggtaccagttgaagtccgtccggttcgtcgtaatgctctggcaatgcgttggatcgttgaagctgctcgtaaacgcggtgataaatccatggctctgcgcctggcgaacgaactttctgatgctgcagaaaacaaaggtactgcagttaagaaacgtgaagacgttcaccgtatggccgaagccaacaaggcgttcgcacactaccgttggtaa

SEQ ID NO: 44 - protein, 156 aa, E. coli
MPRRRVIGQRKILPDPKFGSELLAKFVNILMVDGKKSTAESIVYSALETLAQRSGKSELEAFEVALENVRPTVEVKSRRVGGSTYQVPVEVRPVRRNALAMRWIVEAARKRGDKSMALRLANELSDAAENKGTAVKKREDVHRMAEANKAFAHYRW

SEQ ID NO: 45 - DNA, 2475 bp, S. cerevisiae
  CDS (1)..(2475): S. cerevisiae essential gene FOL1 YNL256W SGDID:S000005200
atgtcaaagctattttctactgtcaattctgcaagacatagtgtaccactaggcggcatgagagattatgtgcacattaagaaactagagatgaatacagttcttgggcctgattcctggaatcaattaatgcctcagaaatgtctactaagcttagatatgggtacagattttagtaaatctgcggctacggatgatttgaaatattctctaaattatgcagttatttctcgtgatttgacgaatttcgtcagcaaaaaaaagaattggggttctgtttctaatttggctaaatctgtgtctcaatttgttatggacaaatattctggtgtcgagtgtctgaatttagaagtgcaggcggatacaacgcatattagaagtgaccacatatcttgtattattcaacaagaaagagggaatccagaatcacaggaatttgacgttgttaggatatctgagttaaaaatgttgactttgattggtgttttcacctttgagagacttaagaaacagtatgtaactttggatataaagttgccttggccaaagaaagccgaattgccaccgccagtgcaaagcataattgataacgttgtcaagtttgtggaggaatcaaatttcaagactgtggaagctcttgtagaatctgtgtcagctgttattgcccataacgagtattttcaaaagtttccagattcgcctttggtggtgaaggttttgaaattaaacgcaatcacagccacagaaggtgttggtgtaagctgtattagagagcccagggagattgcgatggtaaatattccatatctttcctccatacatgaatcgtctgatattaagttccaattgtcttcatcacaaaacactcctattgagggtaaaaatacatggaaaagagcgtttttagcgtttggttcaaacattggggaccgtttcaaacacattcaaatggcgttgcaattattatcaagggaaaaaacggttaaattacggaatatttcgtctatttttgaaagtgaaccaatgtatttcaaagatcaaacccctttcatgaatgggtgtgttgaggtggagacattactgaccccaagcgaattattaaaattgtgtaaaaaaattgaatatgaagagttgcaaagagtcaagcattttgataatggtccgagaacaatagatctggatattgttatgtttttgaatagcgccggagaagatattatagtaaatgaaccggatttgaatataccgcatcctagaatgctggagaggactttcgttcttgagccgttatgtgaattaatatcccccgttcaccttcatcctgtgacagcggaacccattgtagaccatttaaaacagttatacgacaaacagcatgatgaagataccttatggaaattagttccattgccttatcgtagtggtgtggagcctagatttttgaaattcaagaccgctacaaaacttgacgaatttactggagaaacaaacagaattactgtttcacctacatatatcatggctatcttcaacgctacaccagattcattttccgatggaggtgagcattttgcggacattgaaagtcaattgaatgatatcattaaattgtgtaaagacgcattatatttgcatgagagcgtcatcatcgacgttggagggtgttctaccaggcctaactctattcaggcgtctgaggaagaagaaatacgcaggtctatcccattaattaaggccattagagaaagcactgagttaccgcaagataaagtcatactatccattgatacttatcgttccaatgtcgctaaagaagcgattaaagttggagtggatattattaatgatatttcgggaggtttatttgacagcaacatgtttgccgtaattgcagagaacccagaaatttgttatattttatcacacacacgtggtgatatttcaacgatgaataggctggcgcattacgaaaattttgcattgggtgattctattcagcaagaatttgttcataataccgacattcagcagctagacgacttgaaagacaaaacagtgttaatcaggaatgttggtcaagaaattggcgaaaggtatatcaaagcgattgataatggagtaaagcgctggcaaattctaatcgaccctggacttggttttgctaagacctggaagcaaaacttacaaattattagacatatccccattttaaagaactactcattcaccatgaactcaaacaattcgcaagtgtatgttaacctcagaaatatgcccgttttattgggtccatcgcgcaaaaaattcattggacatatcacaaaagatgtggatgcgaagcaaagagactttgctactggagcggtggtagcgtcgtgtattggtttcggcagcgacatggttagggtccatgacgttaaaaattgttcgaagagcattaaattagcagatgctatttataaaggtttggaataa

SEQ ID NO: 46 - protein, 824 aa, S. cerevisiae
MSKLFSTVNSARHSVPLGGMRDYVHIKKLEMNTVLGPDSWNQLMPQKCLLSLDMGTDFSKSAATDDLKYSLNYAVISRDLTNFVSKKKNWGSVSNLAKSVSQFVMDKYSGVECLNLEVQADTTHIRSDHISCIIQQERGNPESQEFDVVRISELKMLTLIGVFTFERLKKQYVTLDIKLPWPKKAELPPPVQSIIDNVVKFVEESNFKTVEALVESVSAVIAHNEYFQKFPDSPLVVKVLKLNAITATEGVGVSCIREPREIAMVNIPYLSSIHESSDIKFQLSSSQNTPIEGKNTWKRAFLAFGSNIGDRFKHIQMALQLLSREKTVKLRNISSIFESEPMYFKDQTPFMNGCVEVETLLTPSELLKLCKKIEYEELQRVKHFDNGPRTIDLDIVMFLNSAGEDIIVNEPDLNIPHPRMLERTFVLEPLCELISPVHLHPVTAEPIVDHLKQLYDKQHDEDTLWKLVPLPYRSGVEPRFLKFKTATKLDEFTGETNRITVSPTYIMAIFNATPDSFSDGGEHFADIESQLNDIIKLCKDALYLHESVIIDVGGCSTRPNSIQASEEEEIRRSIPLIKAIRESTELPQDKVILSIDTYRSNVAKEAIKVGVDIINDISGGLFDSNMFAVIAENPEICYILSHTRGDISTMNRLAHYENFALGDSIQQEFVHNTDIQQLDDLKDKTVLIRNVGQEIGERYIKAIDNGVKRWQILIDPGLGFAKTWKQNLQIIRHIPILKNYSFTMNSNNSQVYVNLRNMPVLLGPSRKKFIGHITKDVDAKQRDFATGAVVASCIGFGSDMVRVHDVKNCSKSIKLADAIYKGLE

SEQ ID NO: 47 - DNA, 669 bp, S. cerevisiae
  CDS (1)..(669): S. cerevisiae essential gene MED7 YOL135C SGDID:S000005495
atgtccaatgatcctggtaatgaggttagctccttgtacccacctccacccccatacgtgaagtttttcacacagtccaatctggaaaaattaccaaaatacaaagaaaagaaggccgcaagtgcgaagcagacggctccaaataacagtaacggcggcagtgaagaggagattacatgtgcgctagattacctaatcccaccccccatgcccaaaaatcagcagtaccgagcgtttgggagtatatggcaggtgaaggaccaactgcccgatttagagagcatgggactcacccaactttataagaaatccacagaaaacgaaagcacaaattatcaatacaaaatccaagagctacgcaaactattgaaatccctcctgctaaattacttggaactcatcggcgtattgagcataaatccggatatgtatgagcgcaaagtggagaacataaggaccattcttgtcaatattcaccacctacttaatgagtacagaccccatcagtcccgagagtcccttattatgctattggaagaacaattagaatacaagcgcggggaaattcgcgagatcgagcaagtatgcaaacaggtacacgacaaactcaccagcatacaggacaccttaagaaccggatcacaatctcctccatcgtcgtcccaatga

SEQ ID NO: 48 - protein, 222 aa, S. cerevisiae
MSNDPGNEVSSLYPPPPPYVKFFTQSNLEKLPKYKEKKAASAKQTAPNNSNGGSEEEITCALDYLIPPPMPKNQQYRAFGSIWQVKDQLPDLESMGLTQLYKKSTENESTNYQYKIQELRKLLKSLLLNYLELIGVLSINPDMYERKVENIRTILVNIHHLLNEYRPHQSRESLIMLLEEQLEYKRGEIREIEQVCKQVHDKLTSIQDTLRTGSQSPPSSSQ

SEQ ID NO: 49 - DNA, 723 bp, S. cerevisiae
  CDS (1)..(723): S. cerevisiae essential gene RRP40 YOL142W SGDID:S000005502
atgtctacgttcatattccctggtgatagctttcctgtagaccctactacacctgttaaactgggccctggcatatattgtgaccccaatactcaagaaatacgacctgttaatacaggtgttttgcatgtttccgctaagggtaagagtggtgttcagaccgcatatatagactattctagtaagagatacattccatctgtaaacgattttgtaatcggtgtcattatagggacattttcagatagctataaggtttcgttgcaaaatttctcctccagtgtttcactatcgtatatggcttttcccaatgcttcaaagaaaaacaggccaactttgcaagtgggagatctagtgtatgcgagagtttgtaccgcagaaaaggaactagaagccgaaatagaatgttttgactcaactacaggacgcgatgctggtttcgggatattggaagatggtatgatcattgacgtgaatttgaatttcgcacgccagttgcttttcaataatgacttcccgttattaaaagtgttggctgcacataccaagtttgaagtcgccattggtctcaatgggaagatctgggttaagtgcgaggaattatctaacactttagcttgttatagaaccataatggagtgttgtcaaaaaaacgacacggcagcgttcaaggatatagcaaaaagacagtttaaagaaatacttacggtcaaggaggagtag

SEQ ID NO: 50 - protein, 240 aa, S. cerevisiae
MSTFIFPGDSFPVDPTTPVKLGPGIYCDPNTQEIRPVNTGVLHVSAKGKSGVQTAYIDYSSKRYIPSVNDFVIGVIIGTFSDSYKVSLQNFSSSVSLSYMAFPNASKKNRPTLQVGDLVYARVCTAEKELEAEIECFDSTTGRDAGFGILEDGMIIDVNLNFARQLLFNNDFPLLKVLAAHTKFEVAIGLNGKIWVKCEELSNTLACYRTIMECCQKNDTAAFKDIAKRQFKEILTVKEE

SEQ ID NO: 51 - DNA, 1455 bp, S. cerevisiea
  CDS (1)..(1455): S. cerevisiae essential gene NOP8 YOL144W SGDID:S000005504
atggatagtgtaattcaaaaaagaatttttgtcggaaatattttccataatgcagatgattgttattcagaactactagatcgatttggaaaatttggtgattgccaagattttcagtttgaaaaacacaaccactttgcatttatcgatataaggtttaatgatgaggcagattttaacaagctaagaaagagctttaataatgttaagtttaaagggaacattttgaaggttgatgaagcaaagccgaattgggaaagcacctgggcggtacaacatgcaaaggaccttaaagaagatattatactaaatgctaaaatgaaaaaaaagaattggcaacattataagaaaatggaaaatgtagcgaaaagttggaaagatcataaggaagttattgctggcagaatgagggaggcgccgagaaaaaggagtcaattgaggaacattacattcaggatcaatgtcaatggttcattgaaagtttacaaatgctataagactaaattatggggttatgaaaggaacaaagaattgaatgaccttgtgtacaagtttacaaataatttctggaaaaacggatacaaccacattgtcgatagattggattacagtcgtgctgttaaaactgttcgattcaaaaatgggctgaaacagttaacagtgtcaaaagatgaaaacgtttgcagtggagagatggacagcgatgagaatatgtcagaagaggagaaggagaaaaataatgttattcttaatgacctattaaaggactttgacttcgataagccaatgacgttgaatgattcggacgaggaacttctgacagagcaacgtaaaggagaggaagaagaagaagaagaagaagaaaaagaagtaaacgctcccgaatacgagaatgttaataagacgaaggaccagagcaccctaccacaagaaaaaccagaggaaaggaaagaacaggacgagggcgacgggcaggaggataatgaatttattccgactttcaccaaggaaattggtcaaggtacaataagcaacactgagacgttaagaaacctattcaaccccaacgaggcagaacctgtatcacaattcaaattgattgaagattctgataatgatattgatcatgcgaaagatgttgatgtgaaccaactggaggaagaagtaagtaaatcatctgacaccctaggtttgacatcggctcccgtaccacatgtatctagagataaagataacaaaaatttcttgtttttccctcatttgcaatcgccatttttagtaggacaaacacagttgagtaaagtaagggctcctggaagagaaacaatgctatcgaactgggatgaggagttctgggctaacagaggtaattggacccgtgatatgaggcgcaaaatgaaagatgcattgaagcaccgtaagaggaaacaatcaaagagcgggcttcttctatag

SEQ ID NO: 52 - protein, 484 aa, S. cerevisiea
MDSVIQKRIFVGNIFHNADDCYSELLDRFGKFGDCQDFQFEKHNHFAFIDIRFNDEADFNKLRKSFNNVKFKGNILKVDEAKPNWESTWAVQHAKDLKEDIILNAKMKKKNWQHYKKMENVAKSWKDHKEVIAGRMREAPRKRSQLRNITFRINVNGSLKVYKCYKTKLWGYERNKELNDLVYKFTNNFWKNGYNHIVDRLDYSRAVKTVRFKNGLKQLTVSKDENVCSGEMDSDENMSEEEKEKNNVILNDLLKDFDFDKPMTLNDSDEELLTEQRKGEEEEEEEEEKEVNAPEYENVNKTKDQSTLPQEKPEERKEQDEGDGQEDNEFIPTFTKEIGQGTISNTETLRNLFNPNEAEPVSQFKLIEDSDNDIDHAKDVDVNQLEEEVSKSSDTLGLTSAPVPHVSRDKDNKNFLFFPHLQSPFLVGQTQLSKVRAPGRETMLSNWDEEFWANRGNWTRDMRRKMKDALKHRKRKQSKSGLLL

SEQ ID NO: 53 - DNA, 1665 bp, S. cerevisiae
  CDS (1)..(1665): S. cerevisiae essential gene PGI1 YBR196C SGDID:S000000400
atgtccaataactcattcactaacttcaaactggccactgaattgccagcctggtctaagttgcaaaaaatttatgaatctcaaggtaagactttgtctgtcaagcaagaattccaaaaagatgccaagcgttttgaaaaattgaacaagactttcaccaactatgatggttccaaaatcttgttcgactactcaaagaacttggtcaacgatgaaatcattgctgcattgattgaactggccaaggaggctaacgtcaccggtttgagagatgctatgttcaaaggtgaacacatcaactccactgaagatcgtgctgtctaccacgtcgcattgagaaacagagctaacaagccaatgtacgttgatggtgtcaacgttgctccagaagtcgactctgtcttgaagcacatgaaggagttctctgaacaagttcgttctggtgaatggaagggttataccggtaagaagatcaccgatgttgttaacatcggtattggtggttccgatttgggtccagtcatggtcactgaggctttgaagcactacgctggtgtcttggatgtccacttcgtttccaacattgacggtactcacattgctgaaaccttgaaggttgttgacccagaaactactttgtttttgattgcttccaagactttcactaccgctgaaactatcactaacgctaacactgccaagaactggttcttgtcgaagacaggtaatgatccatctcacattgctaagcatttcgctgctttgtccactaacgaaaccgaagttgccaagttcggtattgacaccaaaaacatgtttggtttcgaaagttgggtcggtggtcgttactctgtctggtcggctattggtttgtctgttgccttgtacattggctatgacaactttgaggctttcttgaagggtgctgaagccgtcgacaaccacttcacccaaaccccattggaagacaacattccattgttgggtggtttgttgtctgtctggtacaacaacttctttggtgctcaaacccatttggttgctccattcgaccaatacttgcacagattcccagcctacttgcaacaattgtcaatggaatctaacggtaagtctgttaccagaggtaacgtgtttactgactactctactggttctatcttgtttggtgaaccagctaccaacgctcaacactctttcttccaattggttcaccaaggtaccaagttgattccatctgatttcatcttagctgctcaatctcataacccaattgagaacaaattacatcaaaagatgttggcttcaaacttctttgctcaagctgaagctttaatggttggtaaggatgaagaacaagttaaggctgaaggtgccactggtggtttggtcccacacaaggtcttctcaggtaacagaccaactacctctatcttggctcaaaagattactccagctactttgggtgctttgattgcctactacgaacatgttactttcactgaaggtgccatttggaatatcaactctttcgaccaatggggtgttgaattgggtaaagtcttggctaaagtcatcggcaaggaattggacaactcctccaccatttctacccacgatgcttctaccaacggtttaatcaatcaattcaaggaatggatgtga

SEQ ID NO: 54 - protein, 554 aa, S. cerevisiae
MSNNSFTNFKLATELPAWSKLQKIYESQGKTLSVKQEFQKDAKRFEKLNKTFTNYDGSKILFDYSKNLVNDEIIAALIELAKEANVTGLRDAMFKGEHINSTEDRAVYHVALRNRANKPMYVDGVNVAPEVDSVLKHMKEFSEQVRSGEWKGYTGKKITDVVNIGIGGSDLGPVMVTEALKHYAGVLDVHFVSNIDGTHIAETLKVVDPETTLFLIASKTFTTAETITNANTAKNWFLSKTGNDPSHIAKHFAALSTNETEVAKFGIDTKNMFGFESWVGGRYSVWSAIGLSVALYIGYDNFEAFLKGAEAVDNHFTQTPLEDNIPLLGGLLSVWYNNFFGAQTHLVAPFDQYLHRFPAYLQQLSMESNGKSVTRGNVFTDYSTGSILFGEPATNAQHSFFQLVHQGTKLIPSDFILAAQSHNPIENKLHQKMLASNFFAQAEALMVGKDEEQVKAEGATGGLVPHKVFSGNRPTTSILAQKITPATLGALIAYYEHVTFTEGAIWNINSFDQWGVELGKVLAKVIGKELDNSSTISTHDASTNGLINQFKEWM

SEQ ID NO: 55 - DNA, 759 bp, S. cerevisiae
  CDS (1)..(759): S. cerevisiae essential gene NEP1 EMG1 YLR186W SGDID:S000004176
atggtcgaagattccagagttagagacgccctcaaaggtggtgatcagaaggcattaccggcctctttggttcctcaagcacctcctgtcttgacatcaaaggataagattactaagcggatgattgtggtattagcgatggcatccctcgagacacacaagatatcgtccaacgggcctggtggtgacaaatatgtccttttgaactgtgacgaccatcaaggtttattaaaaaaaatgggtagagacattagtgaagcaagacctgatattacccaccaatgtcttttgacgttgctagattctccaatcaacaaagccggaaagctgcaggtctatattcaaacaagtcgaggaattctgatcgaggttaaccccactgttcgtataccaagaactttcaaaagattttcaggtttaatggttcagttactacataagctttctatcagatcggtaaattctgaagaaaagttacttaaagtcattaagaacccaattaccgatcacctacctactaagtgccgtaaggtgacattatcctttgacgcaccagttatccgcgttcaagattacatcgaaaaactagacgatgatgaaagtatatgtgtctttgttggtgccatggcaagaggtaaagataactttgcggatgaatacgtcgacgaaaaagtcggcttgtccaattacccattgtctgcctcagttgcatgttctaaattttgccatggcgctgaagatgcttggaatattttatag

SEQ ID NO: 56 - protein, 252 aa, S. cerevisiae
MVEDSRVRDALKGGDQKALPASLVPQAPPVLTSKDKITKRMIVVLAMASLETHKISSNGPGGDKYVLLNCDDHQGLLKKMGRDISEARPDITHQCLLTLLDSPINKAGKLQVYIQTSRGILIEVNPTVRIPRTFKRFSGLMVQLLHKLSIRSVNSEEKLLKVIKNPITDHLPTKCRKVTLSFDAPVIRVQDYIEKLDDDESICVFVGAMARGKDNFADEYVDEKVGLSNYPLSASVACSKFCHGAEDAWNIL

SEQ ID NO: 57 - DNA, 804 bp, S. cerevisiea
  CDS (1)..(804): S. cerevisea essential gene URA3
atgtcgaaagctacatataaggaacgtgctgctactcatcctagtcctgttgctgccaagctatttaatatcatgcacgaaaagcaaacaaacttgtgtgcttcattggatgttcgtaccaccaaggaattactggagttagttgaagcattaggtcccaaaatttgtttactaaaaacacatgtggatatcttgactgatttttccatggagggcacagttaagccgctaaaggcattatccgccaagtacaattttttactcttcgaagacagaaaatttgctgacattggtaatacagtcaaattgcagtactctgcgggtgtatacagaatagcagaatgggcagacattacgaatgcacacggtgtggtgggcccaggtattgttagcggtttgaagcaggcggcagaagaagtaacaaaggaacctagaggccttttgatgttagcagaattgtcatgcaagggctccctatctactggagaatatactaagggtactgttgacattgcgaagagcgacaaagattttgttatcggctttattgctcaaagagacatgggtggaagagatgaaggttacgattggttgattatgacacccggtgtgggtttagatgacaagggagacgcattgggtcaacagtatagaaccgtggatgatgtggtctctacaggatctgacattattattgttggaagaggactatttgcaaagggaagggatgctaaggtagagggtgaacgttacagaaaagcaggctgggaagcatatttgagaagatgcggccagcaaaactaa

SEQ ID NO: 58 - protein, 267 aa, S. cerevisiea
MSKATYKERAATHPSPVAAKLFNIMHEKQTNLCASLDVRTTKELLELVEALGPKICLLKTHVDILTDFSMEGTVKPLKALSAKYNFLLFEDRKFADIGNTVKLQYSAGVYRIAEWADITNAHGVVGPGIVSGLKQAAEEVTKEPRGLLMLAELSCKGSLSTGEYTKGTVDIAKSDKDFVIGFIAQRDMGGRDEGYDWLIMTPGVGLDDKGDALGQQYRTVDDVVSTGSDIIIVGRGLFAKGRDAKVEGERYRKAGWEAYLRRCGQQN

SEQ ID NO: 59 - DNA, 1095 bp, S. cerevisiae
  CDS (1)..(1095): S. ceverisiae essential gene LEU2
atgtctgcccctaagaagatcgtcgttttgccaggtgaccacgttggtcaagaaatcacagccgaagccattaaggttcttaaagctatttctgatgttcgttccaatgtcaagttcgatttcgaaaatcatttaattggtggtgctgctatcgatgctacaggtgtcccacttccagatgaggcgctggaagcctccaagaaggttgatgccgttttgttaggtgctgtggctggtcctaaatggggtaccggtagtgttagacctgaacaaggtttactaaaaatccgtaaagaacttcaattgtacgccaacttaagaccatgtaactttgcatccgactctcttttagacttatctccaatcaagccacaatttgctaaaggtactgacttcgttgttgtcagagaattagtgggaggtatttactttggtaagagaaaggaagacgatggtgatggtgtcgcttgggatagtgaacaatacaccgttccagaagtgcaaagaatcacaagaatggccgctttcatggccctacaacatgagccaccattgcctatttggtccttggataaagctaatcttttggcctcttcaagattatggagaaaaactgtggaggaaaccatcaagaacgaattccctacattgaaggttcaacatcaattgattgattctgccgccatgatcctagttaagaacccaacccacctaaatggtattataatcaccagcaacatgtttggtgatatcatctccgatgaagcctccgttatcccaggttccttgggtttgttgccatctgcgtccttggcctctttgccagacaagaacaccgcatttggtttgtacgaaccatgccacggttctgctccagatttgccaaagaataaggttgaccctatcgccactatcttgtctgctgcaatgatgttgaaattgtcattgaacttgcctgaagaaggtaaggccattgaagatgcagttaaaaaggttttggatgcaggtatcagaactggtgatttaggtggttccaacagtaccaccgaagtcggtgatgctgtcgccgaagaagttaagaaaatccttgcttaa

SEQ ID NO: 60 - protein, 364 aa, S. cerevisiae
MSAPKKIVVLPGDHVGQEITAEAIKVLKAISDVRSNVKFDFENHLIGGAAIDATGVPLPDEALEASKKVDAVLLGAVAGPKWGTGSVRPEQGLLKIRKELQLYANLRPCNFASDSLLDLSPIKPQFAKGTDFVVVRELVGGIYFGKRKEDDGDGVAWDSEQYTVPEVQRITRMAAFMALQHEPPLPIWSLDKANLLASSRLWRKTVEETIKNEFPTLKVQHQLIDSAAMILVKNPTHLNGIIITSNMFGDIISDEASVIPGSLGLLPSASLASLPDKNTAFGLYEPCHGSAPDLPKNKVDPIATILSAAMMLKLSLNLPEEGKAIEDAVKKVLDAGIRTGDLGGSNSTTEVGDAVAEEVKKILA

SEQ ID NO: 61 - DNA, 675 bp, S. cerevisiae
  CDS (1)..(675): S. cerevisiae essential gene TRP1
atgtctgttattaatttcacaggtagttctggtccattggtgaaagtttgcggcttgcagagcacagaggccgcagaatgtgctctagattccgatgctgacttgctgggtattatatgtgtgcccaatagaaagagaacaattgacccggttattgcaaggaaaatttcaagtcttgtaaaagcatataaaaatagttcaggcactccgaaatacttggttggcgtgtttcgtaatcaacctaaggaggatgttttggctctggtcaatgattacggcattgatatcgtccaactgcatggagatgagtcgtggcaagaataccaagagttcctcggtttgccagttattaaaagactcgtatttccaaaagactgcaacatactactcagtgcagcttcacagaaacctcattcgtttattcccttgtttgattcagaagcaggtgggacaggtgaacttttggattggaactcgatttctgactgggttggaaggcaagagagccccgaaagcttacattttatgttagctggtggactgacgccagaaaatgttggtgatgcgcttagattaaatggcgttattggtgttgatgtaagcggaggtgtggagacaaatggtgtaaaagactctaacaaaatagcaaatttcgtcaaaaatgctaagaaatag

SEQ ID NO: 62 - protein, 224 aa, S. cerevisiae
MSVINFTGSSGPLVKVCGLQSTEAAECALDSDADLLGIICVPNRKRTIDPVIARKISSLVKAYKNSSGTPKYLVGVFRNQPKEDVLALVNDYGIDIVQLHGDESWQEYQEFLGLPVIKRLVFPKDCNILLSAASQKPHSFIPLFDSEAGGTGELLDWNSISDWVGRQESPESLHFMLAGGLTPENVGDALRLNGVIGVDVSGGVETNGVKDSNKIANFVKNAKK

SEQ ID NO: 63 - DNA, 657 bp, S. cerevisiae
  CDS (1)..(657): S. cerevisiae essential gene HIS3
atgacagagcagaaagccctagtaaagcgtattacaaatgaaaccaagattcagattgcgatctctttaaagggtggtcccctagcgatagagcactcgatcttcccagaaaaagaggcagaagcagtagcagaacaggccacacaatcgcaagtgattaacgtccacacaggtatagggtttctggaccatatgatacatgctctggccaagcattccggctggtcgctaatcgttgagtgcattggtgacttacacatagacgaccatcacaccactgaagactgcgggattgctctcggtcaagcttttaaagaggccctactggcgcgtggagtaaaaaggtttggatcaggatttgcgcctttggatgaggcactttccagagcggtggtagatctttcgaacaggccgtacgcagttgtcgaacttggtttgcaaagggagaaagtaggagatctctcttgcgagatgatcccgcattttcttgaaagctttgcagaggctagcagaattaccctccacgttgattgtctgcgaggcaagaatgatcatcaccgtagtgagagtgcgttcaaggctcttgcggttgccataagagaagccacctcgcccaatggtaccaacgatgttccctccaccaaaggtgttcttatg

SEQ ID NO: 64 - protein, 219 aa, S. cerevisiae
MTEQKALVKRITNETKIQIAISLKGGPLAIEHSIFPEKEAEAVAEQATQSQVINVHTGIGFLDHMIHALAKHSGWSLIVECIGDLHIDDHHTTEDCGIALGQAFKEALLARGVKRFGSGFAPLDEALSRAVVDLSNRPYAVVELGLQREKVGDLSCEMIPHFLESFAEASRITLHVDCLRGKNDHHRSESAFKALAVAIREATSPNGTNDVPSTKGVLM

SEQ ID NO: 65 - DNA, 290 bp, E. coli
  promoter (1)..(290): burden sensing promoter p(htpG)
gccaccaaccccacggttgaaggtgaagctaccgctaactacattgccgagctttgcgcgcaatatgacgtggaagccagccgaatcgctcatggcgtaccggttggcggcgaactggaaatggtcgatggcaccacgctgtcacactcccttgccgggcgtcataagattcgtttttaagcaaacgagagcaggatcacctgctctcgcttgaaattattctcccttgtccccatctctccctcatcctgtttttaaccttaaaatggcattattgaggtagacctaca

SEQ ID NO: 66 - DNA, 257 bp, E. coli
  promoter (1)..(257): burden sensing promoter p(ibpA)
atcccttgctgaaaataacatcatcattacgtcgcactgtggcggctatcgcactttaacgtttcgtgctgccccctcagtctatgcaatagaccataaactgcaaaaaaaagtccgctgataaggcttgaaaagttcatttccagacccatttttacatcgtagccgatgaggacgcgcctgatgggtgttctggctacctgacctgtccattgtggaaggtcttacattctcgctgatttcaggagctattgatt

SEQ ID NO: 67 - DNA, 298 bp, E.coli
  promoter (1)..(298): burden sensing promoter p(clpB)
gataagtatctggcggatatttatctgcttgcccggcagcgtctggcgagcgttggtgttgaacaaattttcggcggcgaccgttgtacatatacggaaaatgagactttcttctcttatcgtcgcgacaagaccaccgggcgtatggcaagtttcatttggctgatataacctaaagaatcaagacgatccggtacgcgtgattttcttttcacattaatctggtcaataaccttgaataattgagggatgacctcatttaatctccagtagcaactttgatccgttatgggaggag

SEQ ID NO: 68 - DNA, 300 bp, E. coli
  promoter (1)..(300): burden sensing promoter p(yccV)
ggttataaagacatcaacatgctggcgattcagctgctgaatgaaggcggtattctcctgactttctcctgttccggtctgatgaccagcgatttatttcagaaaatcatcgcggatgccgcaattgatgccggtcgtgatgtacaatttatagagcagttccgtcaggcagccgatcatccggtgatcgctacctatccggaagggctatatctgaaagggtttgcctgtcgcgtcatgtaacttgaaatgtggaattttacccttatatcaaaggtaaagatttcccgggaggtgact

SEQ ID NO: 69 - DNA, 300 bp, E. coli
  promoter (1)..(300): burden sensing promoter p(grpE)
tctccgcgagcgtgccagttttcacattcttcagttgcagttcgtgagcgatttgttgctcaacgatgacctcgtaaccttttgtgcacagccagcggtagagcatttcatgtgttgtcagtgcagtggggtgccgtgggtgtcccacaatgccaatacacttgaaatgattattcatttttccgaggtccttgttgcgaagattgatgacaatgtgagtgcttcccttgaaaccctgaaactgatccccataataagcgaagttagcgagatgaatgcgaaaaaaacgcggagaaattc

SEQ ID NO: 70 - DNA, 300 bp, E. coli
  promoter (1)..(300): burden sensing promoter p(ycjX)
ttggctgatactgtaattcttcaatggcccgtaacactttttcgcgcgcttccggggagatattagtttgcttattcagcacgcgtgatacggtggattttgatacgcctgcaaccctggcaatatcataaatagtaggggacataggtcaggaactccgtccgaacgtgaatgctgcacatcttatggagttcgccggtcgatgacaacacgggcagttgataatcaatggcctggcccccacattcatatccttacgaatgattttttttctggtcttcagagcagcacaggacagca

SEQ ID NO: 71 - DNA, 300 bp, E. coli
  promoter (1)..(300): burden sensing promoter p(ldhA)
gggaacccacagcccgagcgtcatcagcagcgtcaacggcacaagaataatcagtaataacagcgcgagaacggctttatatttacccagcatgggtagttaatatcctgatttagcgaaaaattaagcattcaatacgggtattgtggcatgtttaaccgttcagttgaaggttgcgcctacactaagcatagttgttgatgaatttttcaatatcgccatagctttcaattatatttgaaattttgtaaaatatttttagtagcttaaatgtgattcaacatcactggagaaagtctt

SEQ ID NO: 72 - DNA, 300 bp, E. coli
  promoter (1)..(300): burden sensing promoter p(mutM)
ggcgaaaagtactaagtacttagaggaaataaatcatggctaaaggtattcgtgagaaaatcaagctggtttcttctgctggtactggtcacttctataccactacgaagaacaaacgtactaagccggaaaaactggaactgaaaaaattcgatccagttgttcgccagcacgtgatctacaaagaagcgaaaatcaaataattctcgctttgatgtaacaaaaaacctcgctccggcggggttttttgttatctgcttgcccccatattgactgcatctgttcattcctggagatgct

SEQ ID NO: 73 - DNA, 300 bp, E. coli
  promoter (1)..(300): burden sensing promoter p(ybbN)
cccattcgtactcgcttcaccgacaacgtcaaccagacgcaaagtgataaaccagtcgaaaatcccggcatcgccgcccgctttacgttgggaccggaagcggtggtggacaaagtacgccatgcttttattagcgagaagccgaagatgcgctatccggtaacgctggtgacctgggcagtaatggtgcttaagcgcctgctgccggggcgcgtgatggacaaaatattgcaggggtgagttgaagcgcgcgcttaagcccccatgtcaaagaaaatatcgacaacagagagcgactcc

SEQ ID NO: 74 - DNA, 298 bp, E. coli
  promoter (1)..(298): burden sensing promoter p(prlC)
agttcttgtttgagtccactcatgggttgatgtccgattgcgcccaaattttgggcaactgcgtagattttcgatggtagcacaatcagattcgcttatgacggtgatgaagaaattgcgatgaaatgtgaggtgaatcagggttttcacccgattttgtgctgatcagaattttttttctttttcccccttgaaggggcgaagcctcatccccatttctctggtcaccagccgggaaaccacgtaagctccggcgtcacccataacagatacggactttctcaaaggagagttatca

SEQ ID NO: 75 - DNA, 298 bp, E. coli; identical to SEQ ID NO: 74
  promoter (1)..(298): burden sensing promoter p(groES)

SEQ ID NO: 76 - DNA, 392 bp, E. coli
  promoter (1)..(392): burden sensing promoter p(fxsA)
  misc_feature (328)..(328): N is A, T, C or G
gatccccggaatattcatatgttaaacacacagaatatatgtggtttcgaatgtttttcgaccgacgattatcccctgcatcgaccgaatacccgagatcatatgctgcttgaggatttctaccgtaatctggatcactttaagtgtcggtttttaccccttaattattaatttgtgaaatagatcaccgctttgggattactaccaaaaatagttgcgcaaacatcttgaaattttgctaatgaccacaatataagctgaacgcgattcgcaacccattcaggtagccgggttttaccggctgctattacaggagaaacctacttgnaaggtatgaaactctttgcccagggtacttcactggaccttagccatcctcacgtaatggggat

SEQ ID NO: 77 - DNA, 300 bp, E. coli
  promoter (1)..(300): burden sensing promoter p(htpX)
agattaccaggagccggatccttatctggatgagacggtgaatatcgcactcgatctggcgaagcttgaaaaagccagacccgcggaacaacccgctcccgtcaagtaatatcaatcaggcacaagaaattgtgcctgattttttaacagcggcaagatgccgtaaatcagatgctacaaaatgtaaagttgtgtctttctggtgacttacgcactatccagacttgaaaatagtcgcgtaacccatacgatgtgggtatcgcatattgcgttttgttaaactgaggtaaaaagaaaatt

SEQ ID NO: 78 - DNA, 275 bp, E. coli
  promoter (1)..(275): burden sensing promoter p(rrnB)
gcaaacacgccgccgggtcagcggggttctcctgagaattccggcagagaaagcaaaaataaatgcttgactctgtagcgggaaagcgtattatgcacaccccgcgccgctgagaaaaagcgaagcggcactgctctttaacaatttatcagacaatctgtgtgggcactcgaagatacggattcttaacgtcgcaagacgaaaaatgaataccaagtctcaagagtgaacacgtaattcattacgaagtttaattctttgagcgtcaaactttt

SEQ ID NO: 79 - DNA, 296 bp, E. coli
  promoter (1)..(296): burden sensing promoter p(rrnE)
aatgcgcctccgttgagacgacaacgtgaaacacttcacaggatggtcggaacaacgaagagaaaaaaatcctgaaattcagggttgactctgaaagaggaaagcgtaatatacgccacctcgcgacagtgagctgaaagccgcgtcgcaactgctctttaacaatttatcagacaatctgtgtgggcactcgaagatacggattcttaacgtcgcaagacgaaaaatgaataccaagtctcaagagtgaacacgtaattcattacgaagtttaattctttgagcatcaaactttt

SEQ ID NO: 80 - DNA, 300 bp, E. coli
  promoter (1)..(300): burden sensing promoter p(cspD)
cggttatcggcagaacgccctgccgctgacaagagcttatttgcctgaccaatctactccacatgatagataactatcatctatcgttggcatcagcgacatctgtcacattcctgtcaatagcgttaactgcttcaaatttttgattcatacctgccccctgtcccctgtcaaatgcttgacggctcgccctaattctctaaattgtatttctagagttggcgaggttttgaacagccccctctctgaccccggtttattccatcttacttgtataagatttgcgaaggatgtcgaagc

SEQ ID NO: 81 - DNA, 299 bp, E. coli
  promoter (1)..(299): burden sensing promoter p(katE)
taaatccatctttatcgcatgttctggcggcgcgggttccgtgcgtgggacatagctaataatctggcggttttgctggcggagcggtttcttcattactggcttcactaaacgcatattaaaaatcagaaaaactgtagtttagccgatttagcccctgtacgtcccgctttgcgtgtatttcataacaccgtttccagaatagtctccgaagcgggatctggctggtggtctatagttagagagttttttgaccaaaacagcggccctttcagtaataaattaaggagacgagttca

SEQ ID NO: 82 - DNA, 300 bp, E. coli
  promoter (1)..(300): burden sensing promoter p(xthA)
caaaccatatgcatttaaagtgcatataaagtgaatacgtttgcgatgtgggtgaataaaaagaataaaaaacgcaatgttatgcagaagtaaaatataattctggaattgtgatcattgacgaaatttactggaaattactgcgccattctgacgcagcgcgcaccaaaagcgggcattttttgcgccatcgttgacatcattaacaatcatcgatcaaatcacttaacaacaggcggtaagcaacgcgaaattctgctaccatccacgcactctttatctgaataaatggcagcgact

SEQ ID NO: 83 - DNA, 301 bp, E. coli
  promoter (1)..(301): burden sensing promoter p(uspE)
taatatctgggcctgacggtagaaaccatcagccgtctgctgggtcgcttccagaaaagcggtatgctggcagtcaaaggtaaatacatcaccatcgaaaataacgatgcgctggcccagcttgctggtcatacgcgtaacgttgcctgatttttccgcataactcactatccttctgtcatatcattaaatttttctgatttattgatctggcagaaggttcatcactgtttcattcaccagatatgggttaatcttttaattacaaactgcgttgacagttgttgtaaggagaccctgt

SEQ ID NO: 84 - DNA, 300 bp, E. coli
  promoter (1)..(300): burden sensing promoter p(gadB)
taattttataaatgcgttcaaaataataatcaagtactaatagtgatattttaaggtctgatttttacgtgataattcaggaggcacagaatgcgcataaaaataacagcataaaacaccttaccaccacccaagaatttcatattgtattgtttttcaatgaaaaaatattattcgcgtaatatctcacgataaataacattaggattttgttatttaaacacgagtcctttgcacttgcttactttatcgataaatcctacttttttaatgcgatccaatcattttaaggagtttaaa

SEQ ID NO: 85 - DNA, 300 bp, E. coli
  promoter (1)..(300): burden sensing promoter p(ahpC)
tagatcaggtgattgccctttgtttatgagggtgttgtaatccatgtcgttgttgcatttgtaagggcaacacctcagcctgcaggcaggcactgaagataccaaagggtagttcagattacacggtcacctggaaagggggccattttactttttatcgccgctggcggtgcaaagttcacaaagttgtcttacgaaggttgtaaggtaaaacttatcgatttgataatggaaacgcattagccgaatcggcaaaaattggttaccttacatctcatcgaaaacacggaggaagtatag

SEQ ID NO: 86 - DNA, 300 bp, E. coli
  promoter (1)..(300): burden sensing promoter p(katG)
gtgatcacaaattttaaacagagcacaaaatgctgcctcgaaatgagggcgggaaaataaggttatcagccttgttttctccctcattacttgaaggatatgaagctaaaacccttttttataaagcatttgtccgaattcggacataatcaaaaaagcttaattaagatcaatttgatctacatctctttaaccaacaatatgtaagatctcaactatcgcatccgtggattaattcaattataacttctctctaacgctgtgtatcgtaacggtaacactgtagaggggagcacattg

SEQ ID NO: 87 - DNA, 300 bp, E. coli
  promoter (1)..(300): burden sensing promoter p(grxA)
tagaatctgcacttctggccgagaaaatggctcaggcagcgacagggagtcgcttaccgacagcagcgccaccgccagtagcatcattccgataaattccagtatcaacacgcctttaggcaatttaccgatcgcgcgcatacgcttccctctgcaaagtgagccttcagtctaaaacttttcactgtattgtgtttaacagttatagcttttagcaattaatgcaacaggttaaacctactttcagcgaatacattttagcgtgatcattacaggcataaatctatgaggagagaaata

SEQ ID NO: 88 - DNA, 299 bp, E. coli
  promoter (1)..(299): burden sensing promoter p(oxyS)
taactgatccaccagcagcattcccgcctgggtgaacaacactttacggctggtccgctccagcaacatcacgcccagctcatcttccagcttacgaatttgcccgctaagcgtcggctggctaacgtggcaggaatctgccgcacgccgaaaatggcggtgttcagccaatgccaccaggtactcaagatcacgaatattcattatccatcctccatcgccacgatagttcatggcgataggtagaatagcaatgaacgattatccctatcaagcattctgactgataattgctcaca

SEQ ID NO: 89 - DNA, 300 bp, E. coli
  promoter (1)..(300): burden sensing promoter p(poxB)
taggttgtcgctgcctgccgtgcgggtgtttgcggctgctgtaagacaaaagtggtttccggtgaatatacggtgagcagcacaatgacgctgaccgacgccgaaatcgctgaaggttacgtactggcctgctcctgccatccgcagggggatttggttctcgcataatcgccttatgcccgatgatattcctttcatcgggctatttaaccgttagtgcctcctttctctcccatcccttccccctccgtcagatgaactaaacttgttaccgttatcacattcaggagatggagaacc

SEQ ID NO: 90 - DNA, 299 bp, E. coli
  promoter (1)..(299): burden sensing promoter p(trxC)
tagcgggttgtgggtacgtttatcagaatcatcatcactgcggacatacatcactttgaccttgccgcttttacctttcatttcatcgttcatgcttttctccaccagcgctgcgcgaagcgcgcagattacccgaagtccgcgcggttcgccatgatttcgtaccaaagcctgcgactatcatacctattgaataaaacagattgttgtctggaacaatgtccccgataatatgtaacatattagaaacataccggcgtcgttgccgataagtctccttactcatcccgaggttagtt

SEQ ID NO: 91 - DNA, 1000 bp, S. cerevisiae
  promoter (1)..(1000): burden sensing promoter pKAR2
gtgggagtcaatcaaatcccaatcgacgctattactggacaagtcaactttattcgcaaaacaagtcctgtaatcatcaccaaaagtctcaatgaatgcttcttcattaagatactttgaccattccataggcggaaacgtgtttttatccaacactctgtcactcttggaccgtggctttggcgccctttcattttgtcttacataaaagtatctcagcagcattattgcttctttcctcaagatccccggtatactctcgtaccctgccgcactattgttcttgggcactaatgtacacgtatcatgatttactgacaagacagtaccgttgcctccaaatctctcgttgccacaaccgaacaccacctttccaatgtctaattgcttgagagcagatgcacacattatacacggttctacagtaacatatagagtaatgtctttgaacacgtcaacaactcctcgggagcccaacatcgccttgatctgatcgatccccatgaactcagcatgtgctactccagttaatgacttgttcgtatcgttcatgccataagccatcacctggccagttggcgtatgtacaaagatgcaagctaccggtgtctcatcgtggtcaagagcgtatctagccaaacggacagctgtcctcatatgtttaatatgctgcatagtgtgagtcctctagtttttaccgcagccaccagccgcttctcgagcaaagtgtagatcccattaggactcatcattcatctaattttgctatgttagctgcaactttctattttaatagaaccttctggaaatttcacccggcgcggcacccgaggaactggacagcgtgtcgaaaaagttgcttttttatataaaggacacgaaaagggttctctggaagatataaatatggctatgtaattctaaagattaacgtgttactgttttacttttttaaagtccccaagagtagtctcaagggaaaaagcgtatcaaacatacc

SEQ ID NO: 92 - DNA, 1000 bp, S. cerevisiea
  promoter (1)..(1000): burden sensing promoter pPDI1
caggtcgtcagatgtgacgttctcatcgtctagcaaatcatcgggaatcttggacttcatttgctccatggagaaagtatgatctccatgcaagttaacagaacatatacggaaattggtaccacccaggtcggcggctagtaaaacaccgcgctccgtcccgttgggtgacccggtgacgaacgccggaatcataggaagacctttgtccgaggccaatgtgtggccttcctttggtggagctagacctttttccatttgttcgatgaagtaagcagttaattcgtccagcttctcgggggtaacctcgaaatcgtcgcagatctggtccacggcctggatgaccgctctctcagtggctttgtgtaagtcgtcgaatgacatcttgtgtatgatagagttgtattagtggtggtgttgtggtttacggaagctgagttgggcactgatgggggggttgggggttctgttgatagcggatatttatatgggcgcgttttcattagtgcccaccgtttgagcgtggtgtgacaccacgcccaagatagggggccccctgaaaggggttgaccgtccgtcggcacaccacttataatgcggggtgcaagcgccgcgtctaaaattttttttttttccatttttgtcgttattgttatttcccgttttttgttttttttgattttttcggagcgacaaacctttcgaaacacgtgtcctgaaaattatcctgggctgcacgtgataatatgttaccctgtcgggcggcgcctctttttcccttttctctcactagtctctttttccaatttgccaccgtgtagcattttgttgtgctgttacaaccacaacaaaacgaaaaacccgtatggacatacatatatatatatatatatatatatattttgttacgcgtgcattttcttgttgcaagcagcatgtctaattggtaattttaaagctgccaagctctacataaagaaaaacatacatctatcccgtt

SEQ ID NO: 93 - DNA, 1000 bp, S. cerevisiae
  promoter (1)..(1000): burden sensing promoter pSSA1
cactcatatcgggggtcttacttcccatcataaacacggaccaaagaattaaattcatcattcacataagcgaaaaaaagtaatcattattagttaacttccctttacatgtaaccataggaaaaaaaaaaaagaaagaaaaacaacgatctataaagtaaactaaatcggaacatacccttcaatgtatgacttgtcagccaaagaagcgtttaattgtttcaaagtttcaatcttggagaaatcggtggatgccattatgtgtgtatatattcggttggactcttcagtgctgaaaggtagaaagcatgaggtaaaaagataaagagtagaaggaaaaaaaaaagaaccaactaaatatagtgggtagataaccttaaactatttatttagaggcgacaatgtgaaaaattttttcttcaaaggctcggttgtcgacaaattgttacgttgtgctttgatttctaaagcgcttcttcacctgcaggttctgagccctaagaaaaaaaatttccttggttgaaaatggcggaaaaaaaaaattcagaaaaagaaataaagcacgtgtgcgcggtgtgtggatgatggtttcatcattgtcaacggcattttcgttcttgtggattgttgtaaactttccagaacattctagaaagaaagcacacggaacgtttagaagctgtcatttgcgttttttctccagattttagttgagaaagtaattaaattattcttctttttccagaacgttccatcggcggcaaaagggagagaaagaacccaaaaagaaggggggccatttagattagctgatcgtttcgaggacttcaaggttatataaggggtggattgatgtatcttcgagaagggattgagttgtagtttcgtttcccaattcttacttaagttgttttattttctctatttgtaagataagcacatcaaaagaaaagtaatcaagtattacaagaaacaaaaattcaagtaaataacagataat

SEQ ID NO: 94 - DNA, 1000 bp, S. cerevisiea
  promoter (1)..(1000): burden sensing promoter pFPR2
ctgatcttttcacgcagttaggtaaggaaaatcgtggccaaataaatttcattgcattaaactctacaatgttcccacaccacgttagattcctaaatatgagagaacagttcccattatttgctatccataatatgatcaataatctgaaatatggtttaccacaactaccagaagaagagtacgcgaaattagaaaaaccacaaccactagacagagatatgatcgttcagttggtaaaagattaccgtgaaggtactgccaagccaattgttaagtcagaagagattccaaaagaacaaaagtccaatgtttataaaatagttgggaagacacatgacgacattgttcatgatgatgacaaggatgtccttgtcaaatattacgcgacatggtgtattcatagtaaaaggtttgcgcctatttacgaagaaattgcaaatgtcttagcatctgatgaatctgttcgcgataaaatcttgatcgccgaagtagattcaggggcaaatgatatcttaagttttcctgtgacaggatatccaaccattgctttgtatcctgccggaaataactctaagcctattatcttcaataaaattagaaatttggaagatgttttcgaatttatcaaggaatcaggtacacatcacattgacggccaggcaatttatgataaattgcaccaggccaaggattctgaagtgtctactgaagataccgtacatgatgaattataatcaataaataaagcatatataatgcacatttttaacatctgattactcgcatcgtttctggaagaaaatagctaatattcgttatttatggcatcacgattattctcaccagttacccgtttatgctcttgaagagatttagcattactgccagcgcatcttcaaatacaggtttatatgagacccattactataaccctaagaagagaaaaaggagtgctttcgttttcaatcacattctagtttacagtaattgagtctcg

SEQ ID NO: 95 - DNA, 1000 bp, S. cerevisiae
  promoter (1)..(1000): burden sensing promoter pRPL3
cctttcctgcgggatagcttttgcttcaggttcttctgaggttctgaaaatcaatatatttttccgacaatttctcactatgcctctatcccccttaaaaagaaacactttctaccctcttttctaaactctgcacactagaccgagacagcaaatcggagcccgagagaaaatccggaggacggaaaaactagaagtaatcttatgcggggagcatgcaccagaacgcccagaaaacgtgaatgacactacatactttgatacggatgttggtatttttccggctttttctattttatcgatgccgtgtctgctgccattacgtacaggtaggcaaaggcaaacaagaatagcactttttcacttgctgcttttttttgtgaatgaagtttatcgtatattctgttagtgccgctcgtatcagccacttacgttatcattctaaagtaagtatacgaaatgtgcaaaccttagtagacgttcaagaattgctcgataattgcgaacaaaccagctgctaagccgggaagttaagtcctcaacacagaaatgatgcaaacaatttattaaattcagtggtaatgcaacagcaagaggaaaggtggagggattaacgcatttcagacagctttatagggggaaagaaagcactcgcaaacttgctgcctgttcgcagtcattggttgcaaaaactaaactctactcacgcacactggaatgaatggcaatattcttttttaggttaaccggccggacagtaatatagtaatcgttttgtacgtttttcaagaagcgacgcacaactgttttccattttttttttttttttttcagtgatcatcgtccatgaaaaaaatttttcatttgtctctttcgtgcttcctggatatataaaatacgatttatttagttgtctttgtcaatcctcatctttctttactcattatttcatttcggttttgtcatctctagaacaacacagttactacaacaatcaatc

SEQ ID NO: 96 - DNA, 1000 bp, S. cerevisiae
  promoter (1)..(1000): burden sensing promoter pRPL6A
attctcgtgcaagcagttttgcgcgtactttagctcctcatggcacttacaatggttttattaccgtggttgctgcggaaaacgttgccaagcatgttcaaattaagatctctttaactcaaggtggtagactaaaacacatatacaaaacgaaaagccaaaaagccaataatgatggtgttgccgtatttgatgaagagtgctcgttcaaggcttctcccgaagccaatttggtactgggtgcaatttcccatcaaagactatcgagggacaaagatcttggtattgctcaaatcaacttgggtgaccctcaaattcaacaagatggccaaatttctgtaaaattaggagacggtcatctgattgtaaagattaattacggtaaagacaagaatggtcaggtacctcccgtgccagaagttcctcaagaatacacgcagtaataaacagtgaaaactattcttttatacgctcaataagggcacatttggtgtgttaacaggtgtcttttctgtgtttgttataattttgcgctattattatataacgttatatttactataatatattacaacatatattacaacatatttcaacgctctcctgttactgcttagggagaagaaagaaatgtgaagactgctattaaatccgtacattattaaaatgtatggatttgttatatttttcttcagttttttccttaaccagattcgaaaagcggcccgcctagaccattgcggttgcggctaaagcgttctggagagggcttctccgctgggcggacaacagaagcgagagacacgtttcccgtctgggaggactcaccggatttgtccagtttcccactggagtgtgctttgttccttttgcaaaatttcgttggtatggaggttatcgaatggaagggttacatgaatagattaaatgtactactcattaaagattgaatatcagttttacattaggcgaaacaacaaagtaatagccatccaacgaa

SEQ ID NO: 97 - DNA, 1000 bp, S. cerevisiae
  promoter (1)..(1000): pRPL28
  promoter (1)..(1000): burden sensing promoter pRPL28
gggatagccctccatgggaatgtcaaattctgagcacgaaagcacctgctgaggtgcatttaattccgacaagtggtaaccaaattgtattgaaccgattgaggctactataattgcataacataacgcctttgtaattttatgcttgttttgccttggcatgctaacattggatagcaacgatgcactagatagaatcctattcatactatgctacgtacctgtttaactcttctcattttatccgttttctttcttcaccgttcctcttaagttctttatttttttcataacagaatgatcacccctttcactttgccgccaatataatattaacacacaagaaataagtatgaggtagtttgctctcgaaaaaaccaagtaatagttcaaaaaatgaaaaaaagaaaacaaataccaaattatgccaccgttaccttacgtttcatggttaatcatcgtttactgccgcctatgagcgtaagctaatgttataaagaaacaagctataatattgttaaatatagttgatcaacagcattgtaatgattacaagagacgaggtggaatgaaccttatgaaatgcgtattatatataaactgtaataagagctaagttgaattgaaatctacgatacttgatgttgacattatagcactagttcccaggaaaccctttcgaaaaacacagcaaaaacaagagtactgtaaccaatgtaacatctgtacaccagggacccacacattaccaaaatcaaaattatttttctaatgcctgttatttttcctatttttcctctggcgcgtgaatagcccgcagagacgcaaacaattttcctcgcagtttttcgcttgtttaatgcgtattttcccagataggttcaaacctttcatctgtatcccgtatatttaagatggcgtttgctttctccgttgatttttttccttcttagtgatttttttgcattaaatcccagaacaatcatccaactaatcaaga

SEQ ID NO: 98 - DNA, 580 bp, S. cerevisiae
  promoter (1)..(580): burden sensing promoter pOGG1
tgcaatcaggttcttcccaatcatccgaatcagagagcaaatctaggtcttcttttgaaagtatggaaggatgcttcaattgtgcttgaataaagttattagacctgaaaccacgactactcatagaaaacgatagtttggcgtgcgatacgtttttgagtaaaagaaaactgttgaaactacagataaatggccttcttggtataatatgattcaatgttgatcttatccactttggcatgtaaaattgattgatacaagtaagctaatcgctcaatggataatattacaaataaaaatatcgaggcaataccagtatttcaatgtctggccaaataaatagtttagtacagcaatttgattaacgttaaagttactctcctctttgaataatgtcgtggttaaaaagtaaagtatttgtttatacattaagtgaagaaaattaagacgcgcctttctttaatgtaacgccaaaaattttcaagagatgagctgaacagcatcacaaaactactatttccagcggaagaaggcatttgaagcgtcctgattcataattgcgattttatttatcaaccag

SEQ ID NO: 99 - DNA, 1000 bp, S. cerevisiae
  promoter (1)..(1000): burden sensing promoter pRAD51
ccgcaataaagggcttcccggacttggaattaatacctgctaccaccggccccacaaagtatggaccgaatcttctttcataaagtgaacttgacactaattgggtaaacgtttcaggctcaatggccctttcttccttcaacttatataggttcgtcttgtagcggaacatctcgttcagagtagtcacgtcggtagccagaccggtaatccctaagaacacatgcccatagtggaagattttttcaaacttgttcgacacacctagtgactggcttccgagacgcaaatcacaggcaatggccacacagtctttacctgtcatcgcaacgacgataccaccgttaatagaacttggatccgacattttttttttatgctttattcactgttcaatattttcaccacaattcgcaagaaacgcactctacttcgaaactacggttcaaacttacttagcagcttcccgatttaattggcctttctactatgccataaactctttcttcctctcttttcatcgcccctgcatttgcacttttttgccaccggcagtgccatccggtcacatgactacaccacgttaatagcgatctggcttatcattgtcacagagtaaattaaaatggacggtaaatgttggaaatgcaccactaccgttcttcaaccaatctagtttagctatcctgcaacaggtggccttcttgagcattccctgagcattccaaccggttgtatcagtgttttatcaccgtctcaccatatcccacgactaggccacacttcgttaccctatgctacgcgtcatttccgctatttctgtcctggtttgtttacagtacgcgtggtgggaccataaaggggaatagtggggactggagaaaaaattttctcagttacttcttctatcttccgtagtttccatatactagtagttgagtgtagcgacaaagagcagacgtagttatttgttaaaggcctactaatttgttatcgtcat

SEQ ID NO: 100 - DNA, 1000 bp, S. cerevisiae
  promoter (1)..(1000): burden sensing promoter pRAD54
tgcgctacggttcctgccgctcgtgggaaccccacgcaaaacatattattcgcttctctctgctgacaactccggtttacgttataccgtattaggatcactataagggttccttcgggaggaggggggaggggaagaatgtacatcgtcataaggcctttatggtgtgaagtgggttttgcgtggaaaattcgttttcaatgatatagagcccacgcatatacgtacatactagtggccaaaagcgtggggtgggcggacaaagctacactggtaaaatacaggattctatgaacaataacaacaaccagctcacgttgctgaacagccgaggtcagccgatgcaaccgaggtttccaaagtagcatttctgtgctagctatgtctgtaggtttacatttaatggtgcgtggttccagcttcatgtgcttgcatgtgatgtcctgcagatggtaagaagattctgaaagccgcgctaggagaaaaatattctgctcgaagatctgtcctcttaagtagaaagcgtgaaattgttgcgttcttgcattactactcaacgcgtacgcaaatgcgtctactgcacctgcatgataaagcttatgtatcaaaaatttaacatcttgaaaatacacaagtggtgcaaagatgtgtcacgttctggacctgagtggtgccatgtatgctatttaacatgcaaaggggaagacccttccgccttactgcaataataaaaagtattttacgcgttacccaatatagcaaagtttcgcgcaaaaaaaaaaataaaaaacaattacaaacaaaaagaaaaaaaaggaaataatagaagatctaactgaagcgaaggccaaaactcttctcacttgacgtaatagccgatacaaaatctagagcagcaacttttctctttcttcactaaagctgctacgaaagtatagaaaaatcaaacgctcagaacttagctctatttcaaggtaccatatatatttccttataactg

SEQ ID NO: 101 - DNA, 5776 bp, synthetic
  plasmid (1)..(5776): pEG34
  CDS (463)..(1758): hGH-glycine linker-GFP
atcgatgcatgcgcccaatacgcaaaccgcctctccccgcgcgttggccgattcattaatgcagctggcacgacaggtttcccgactggaaagcgggcagtgagcgcaacgcaattaatgtgagttagctcactcattaggcaccccaggctttacactttatgcttccggctcgtatgttgtgtggaattgtgagcggataacaatttcacacaggaaacagctatgaccatgattacgccaagcgcgcaattaaccctcactaaagggaacaaaagctgggtaccgggccccccctcgaggtcgacggtatcgataagcttgatatcagctgaattcattaaagaggagaaaggtaccatgggtctgggcaagaaaaagaaactgctgctgctgttactgagcagcgcagttgcagcaagctttatgagcctgaccattagcctgcctggtgttcaggcatttccgaccattccgctgagccgtctgtttgataatgcaatgctgcgtgcacatcgtctgcatcagctggcatttgatacctatcaagaatttgaagaagcgtatatcccgaaagagcagaaatatagcttcctgcagaatccgcagaccagcctgtgttttagcgaaagcattccgacaccgagcaatcgtgaagaaacccagcagaaaagcaatctggaactgctgcgtattagtctgctgctgattcagagctggctggaaccggtgcagtttctgcgtagcgtttttgcaaatagcctggtttatggtgcaagcgatagcaatgtttatgatctgctgaaagatctggaagaaggtattcagaccctgatgggtcgtctggaagatggttcaccgcgtaccggtcagatctttaaacagacctatagcaaattcgataccaacagccataatgatgatgccctgctgaaaaactatggtctgctgtattgtttccgcaaagatatggataaagtggaaacctttctgcgcattgttcagtgtcgtagcgttgaaggtagctgtggttttggtggcatgcgtaaaggcgaagagctgttcactggtttcgtcactattctggtggaactggatggtgatgtcaacggtcataagttttccgtgcgtggcgagggtgaaggtgacgcaactaatggtaaactgacgctgaagttcatctgtactactggtaaactgccggtaccttggccgactctggtaacgacgctgacttatggtgttcagtgctttgctcgttatccggaccacatgaagcagcatgacttcttcaagtccgccatgccggaaggctatgtgcaggaacgcacgatttcctttaaggatgacggcacgtacaaaacgcgtgcggaagtgaaatttgaaggcgataccctggtaaaccgcattgagctgaaaggcattgactttaaagaagacggcaatatcctgggccataagctggaatacaattttaacagccacaatgtttacatcaccgccgataaacaaaaaaatggcattaaagcgaattttaaaattcgccacaacgtggaggatggcagcgtgcagctggctgatcactaccagcaaaacactccaatcggtgatggtcctgttctgctgccagacaatcactatctgagcacgcaaagcgttctgtctaaagatccgaacgagaaacgcgatcacatggttctgctggagttcgtaaccgcagcgggcatcacgcatggtatggatgaactgtacaaataagtcgacctgcaggcatgcaagcttggctgttttggcggatgagagaagattttcagcctgatacagattaaatcagaacgcagaagcggtctgataaaacagaatttgcctggcggcagtagcgcggtggtcccacctgaccccatgccgaactcagaagtgaaacgccgtagcgccgatggtagtgtggggtctccccatgcgagagtagggaactgccaggcatcaaataaaacgaaaggctcagtcgaaagactgggcctttcgttttatctgttgtttgtcggtgaacgctctcctgagtaggacaaatccgccgggagcggatttgaacgttgcgaagcaacggcccggagggtggcgggcaggacgcccgccataaactgccaggcatcaaattaagcagaaggccatcctgacggatggcctttttgcgtttctacaaactcttttgtttatttttctaaatacattcaaatatgtatccgctcatgagacaataaccctgataaatgcttcaataatattgaaaaaggaagagtatgagtattcaacatttccgtgtcgcccttattcccttttttgcggcattttgccttcctgtttttgctcacccagaaacgctggtgaaagtaaaagatgctgaagatcagttgggtgcagcaaactattaactggcgaactacttactctagcttcccggcaacaattaatagactggatggaggcggataaagttgcaggaccacttctgcgctcggcccttccggctggctggtttattgctgataaatctggagccggtgagcgtgggtctcgcggtatcattgcagcactggggccagatggtaagccctcccgtatcgtagttatctacacgacggggagtcaggcaactatggatgaacgaaatagacagatcgctgagataggtgcctcactgattaagcattggtaactgtcagaccaagtttactcatatatactttagattgatttacgcgccctgtagcggcgcattaagcgcggcgggtgtggtggttacgcgcagcgtgaccgctacacttgccagcgccctagcgcccgctcctttcgctttcttcccttcctttctcgccacgttcgccggctttccccgtcaagctctaaatcgggggctccctttagggttccgatttagtgctttacggcacctcgaccccaaaaaacttgatttgggtgatggttcacgtagtgggccatcgccctgatagacggtttttcgccctttgacgttggagtccacgttctttaatagtggactcttgttccaaacttgaacaacactcaaccctatctcgggctattcttttgatttataagggattttgccgatttcggcctattggttaaaaaatgagctgatttaacaaaaatttaacgcgaattttaacaaaatattaacgtttacaatttaaaaggatctaggtgaagatcctttttgataatctcatgaccaaaatcccttaacgtgagttttcgttccactgagcgtcagaccccgtagaaaagatcaaaggatcttcttgagatcctttttttctgcgcgtaatctgctgcttgcaaacaaaaaaaccaccgctaccagcggtggtttgtttgccggatcaagagctaccaactctttttccgaaggtaactggcttcagcagagcgcagataccaaatactgtccttctagtgtagccgtagttaggccaccacttcaagaactctgtagcaccgcctacatacctcgctctgctaatcctgttaccagtggggcatttgagaagcacacggtcacactgcttccggtagtcaataaaccggtaaaccagcaatagacataagcggctatttaacgaccctgccctgaaccgacgaccgggtcgaatttgctttcgaatttctgccattcatccgcttattatcacttattcaggcgtagcaccaggcgtttaagggcaccaataactgccttaaaaaaattacgccccgccctgccactcatcgcagtactgttgtaattcattaagcattctgccgacatggaagccatcacagacggcatgatgaacctgaatcgccagcggcatcagcaccttgtcgccttgcgtataatatttgcccatggtgaaaacgggggcgaagaagttgtccatattggccacgtttaaatcaaaactggtgaaactcacccagggattggctgagacgaaaaacatattctcaataaaccctttagggaaataggccaggttttcaccgtaacacgccacatcttgcgaatatatgtgtagaaactgccggaaatcgtcgtggtattcactccagagcgatgaaaacgtttcagtttgctcatggaaaacggtgtaacaagggtgaacactatcccatatcaccagctcaccgtctttcattgccatacggaattccggatgagcattcatcaggcgggcaagaatgtgaataaaggccggataaaacttgtgcttatttttctttacggtctttaaaaaggccgtaatatccagctgaacggtctggttataggtacattgagcaactgactgaaatgcctcaaaatgttctttacgatgccattgggatatatcaacggtggtatatccagtgatttttttctccattttagcttccttagctcctgaaaatctcgataactcaaaaaatacgcccggtagtgatcttatttcattatggtgaaagttggaacctcttacgtgccgatcaacgtctcattttcgccaaaagttggcccagggcttcccggtatcaacagggacaccaggatttatttattctgcgaagtgatcttccgtcacaggtatttattcggcgcaaagtgcgtcgggtgatgctgccaacttactgatttagtgtatgatggtgtttttgaggtgctccagtggcttctgtttctatcagctgtccctcctgttcagctactgacggggtggtgcgtaacggcaaaagcaccgccggacatcagcgctagcggagtgtatactggcttactatgttggcactgatgagggtgtcagtgaagtgcttcatgtggcaggagaaaaaaggctgcaccggtgcgtcagcagaatatgtgatacaggatatattccgcttcctcgctcactgactcgctacgctcggtcgttcgactgcggcgagcggaaatggcttacgaacggggcggagatttcctggaagatgccaggaagatacttaacagggaagtgagagggccgcggcaaagccgtttttccataggctccgcccccctgacaagcatcacgaaatctgacgctcaaatcagtggtggcgaaacccgacaggactataaagataccaggcgtttccccctggcggctccctcgtgcgctctcctgttcctgcctttcggtttaccggtgtcattccgctgttatggccgcgtttgtctcattccacgcctgacactcagttccgggtaggcagttcgctccaagctggactgtatgcacgaaccccccgttcagtccgaccgctgcgccttatccggtaactatcgtcttgagtccaacccggaaagacatgcaaaagcaccactggcagcagccactggtaattgatttagaggagttagtcttgaagtcatgcgccggttaaggctaaactgaaaggacaagttttggtgactgcgctcctccaagccagttacctcggttcaaagagttggtagctcagagaaccttcgaaaaaccgccctgcaaggcggttttttcgttttcagagcaagagattacgcgcagaccaaaacgatctcaagaagatcatcttattaatcagataaaatatttgctcatgagcccgaagtggcgagcccgatcttccccatcggtgatgtcggcgatataggcgccagcaaccgcacctgtggcgccggtgatgccggccacgatgcgtccggcgtagaggatctgctcatgtttgacagcttatc

SEQ ID NO: 102 - protein, 431 aa, synthetic
FPTIPLSRLFDNAMLRAHRLHQLAFDTYQEFEEAYIPKEQKYSFLQNPQTSLCFSESIPTPSNREETQQKSNLELLRISLLLIQSWLEPVQFLRSVFANSLVYGASDSNVYDLLKDLEEGIQTLMGRLEDGSPRTGQIFKQTYSKFDTNSHNDDALLKNYGLLYCFRKDMDKVETFLRIVQCRSVEGSCGFGGMRKGEELFTGFVTILVELDGDVNGHKFSVRGEGEGDATNGKLTLKFICTTGKLPVPWPTLVTTLTYGVQCFARYPDHMKQHDFFKSAMPEGYVQERTISFKDDGTYKTRAEVKFEGDTLVNRIELKGIDFKEDGNILGHKLEYNFNSHNVYITADKQKNGIKANFKIRHNVEDGSVQLADHYQQNTPIGDGPVLLPDNHYLSTQSVLSKDPNEKRDHMVLLEFVTAAGITHGMDELYK

SEQ ID NO: 103 - DNA, 660 bp, synthetic
  CDS (1)..(660): Chloramphenicol_acetyltransferase
atggagaaaaaaatcactggatataccaccgttgatatatcccaatggcatcgtaaagaacattttgaggcatttcagtcagttgctcaatgtacctataaccagaccgttcagctggatattacggcctttttaaagaccgtaaagaaaaataagcacaagttttatccggcctttattcacattcttgcccgcctgatgaatgctcatccggaattccgtatggcaatgaaagacggtgagctggtgatatgggatagtgttcacccttgttacaccgttttccatgagcaaactgaaacgttttcatcgctctggagtgaataccacgacgatttccggcagtttctacacatatattcgcaagatgtggcgtgttacggtgaaaacctggcctatttccctaaagggtttattgagaatatgtttttcgtctcagccaatccctgggtgagtttcaccagttttgatttaaacgtggccaatatggacaacttcttcgcccccgttttcaccatgggcaaatattatacgcaaggcgacaaggtgctgatgccgctggcgattcaggttcatcatgccgtctgtgatggcttccatgtcggcagaatgcttaatgaattacaacagtactgcgatgagtggcagggcggggcgtaa

SEQ ID NO: 104 - protein, 219 aa, synthetic
MEKKITGYTTVDISQWHRKEHFEAFQSVAQCTYNQTVQLDITAFLKTVKKNKHKFYPAFIHILARLMNAHPEFRMAMKDGELVIWDSVHPCYTVFHEQTETFSSLWSEYHDDFRQFLHIYSQDVACYGENLAYFPKGFIENMFFVSANPWVSFTSFDLNVANMDNFFAPVFTMGKYYTQGDKVLMPLAIQVHHAVCDGFHVGRMLNELQQYCDEWQGGA

SEQ ID NO: 105 - DNA, 4347 bp, synthetic
  plasmid (1)..(4347): pEG0
atcgatgcatgcgcccaatacgcaaaccgcctctccccgcgcgttggccgattcattaatgcagctggcacgacaggtttcccgactggaaagcgggcagtgagcgcaacgcaattaatgtgagttagctcactcattaggcaccccaggctttacactttatgcttccggctcgtatgttgtgtggaattgtgagcggataacaatttcacacaggaaacagctatgaccatgattacgccaagcgcgcaattaaccctcactaaagggaacaaaagctgggtaccgggccccccctcgaggtcgacggtatcgataagcttgatatcgaattcctgcaggcatgcaagcttggctgttttggcggatgagagaagattttcagcctgatacagattaaatcagaacgcagaagcggtctgataaaacagaatttgcctggcggcagtagcgcggtggtcccacctgaccccatgccgaactcagaagtgaaacgccgtagcgccgatggtagtgtggggtctccccatgcgagagtagggaactgccaggcatcaaataaaacgaaaggctcagtcgaaagactgggcctttcgttttatctgttgtttgtcggtgaacgctctcctgagtaggacaaatccgccgggagcggatttgaacgttgcgaagcaacggcccggagggtggcgggcaggacgcccgccataaactgccaggcatcaaattaagcagaaggccatcctgacggatggcctttttgcgtttctacaaactcttttgtttatttttctaaatacattcaaatatgtatccgctcatgagacaataaccctgataaatgcttcaataatattgaaaaaggaagagtatgagtattcaacatttccgtgtcgcccttattcccttttttgcggcattttgccttcctgtttttgctcacccagaaacgctggtgaaagtaaaagatgctgaagatcagttgggtgcagcaaactattaactggcgaactacttactctagcttcccggcaacaattaatagactggatggaggcggataaagttgcaggaccacttctgcgctcggcccttccggctggctggtttattgctgataaatctggagccggtgagcgtgggtctcgcggtatcattgcagcactggggccagatggtaagccctcccgtatcgtagttatctacacgacggggagtcaggcaactatggatgaacgaaatagacagatcgctgagataggtgcctcactgattaagcattggtaactgtcagaccaagtttactcatatatactttagattgatttacgcgccctgtagcggcgcattaagcgcggcgggtgtggtggttacgcgcagcgtgaccgctacacttgccagcgccctagcgcccgctcctttcgctttcttcccttcctttctcgccacgttcgccggctttccccgtcaagctctaaatcgggggctccctttagggttccgatttagtgctttacggcacctcgaccccaaaaaacttgatttgggtgatggttcacgtagtgggccatcgccctgatagacggtttttcgccctttgacgttggagtccacgttctttaatagtggactcttgttccaaacttgaacaacactcaaccctatctcgggctattcttttgatttataagggattttgccgatttcggcctattggttaaaaaatgagctgatttaacaaaaatttaacgcgaattttaacaaaatattaacgtttacaatttaaaaggatctaggtgaagatcctttttgataatctcatgaccaaaatcccttaacgtgagttttcgttccactgagcgtcagaccccgtagaaaagatcaaaggatcttcttgagatcctttttttctgcgcgtaatctgctgcttgcaaacaaaaaaaccaccgctaccagcggtggtttgtttgccggatcaagagctaccaactctttttccgaaggtaactggcttcagcagagcgcagataccaaatactgtccttctagtgtagccgtagttaggccaccacttcaagaactctgtagcaccgcctacatacctcgctctgctaatcctgttaccagtggggcatttgagaagcacacggtcacactgcttccggtagtcaataaaccggtaaaccagcaatagacataagcggctatttaacgaccctgccctgaaccgacgaccgggtcgaatttgctttcgaatttctgccattcatccgcttattatcacttattcaggcgtagcaccaggcgtttaagggcaccaataactgccttaaaaaaattacgccccgccctgccactcatcgcagtactgttgtaattcattaagcattctgccgacatggaagccatcacagacggcatgatgaacctgaatcgccagcggcatcagcaccttgtcgccttgcgtataatatttgcccatggtgaaaacgggggcgaagaagttgtccatattggccacgtttaaatcaaaactggtgaaactcacccagggattggctgagacgaaaaacatattctcaataaaccctttagggaaataggccaggttttcaccgtaacacgccacatcttgcgaatatatgtgtagaaactgccggaaatcgtcgtggtattcactccagagcgatgaaaacgtttcagtttgctcatggaaaacggtgtaacaagggtgaacactatcccatatcaccagctcaccgtctttcattgccatacggaattccggatgagcattcatcaggcgggcaagaatgtgaataaaggccggataaaacttgtgcttatttttctttacggtctttaaaaaggccgtaatatccagctgaacggtctggttataggtacattgagcaactgactgaaatgcctcaaaatgttctttacgatgccattgggatatatcaacggtggtatatccagtgatttttttctccattttagcttccttagctcctgaaaatctcgataactcaaaaaatacgcccggtagtgatcttatttcattatggtgaaagttggaacctcttacgtgccgatcaacgtctcattttcgccaaaagttggcccagggcttcccggtatcaacagggacaccaggatttatttattctgcgaagtgatcttccgtcacaggtatttattcggcgcaaagtgcgtcgggtgatgctgccaacttactgatttagtgtatgatggtgtttttgaggtgctccagtggcttctgtttctatcagctgtccctcctgttcagctactgacggggtggtgcgtaacggcaaaagcaccgccggacatcagcgctagcggagtgtatactggcttactatgttggcactgatgagggtgtcagtgaagtgcttcatgtggcaggagaaaaaaggctgcaccggtgcgtcagcagaatatgtgatacaggatatattccgcttcctcgctcactgactcgctacgctcggtcgttcgactgcggcgagcggaaatggcttacgaacggggcggagatttcctggaagatgccaggaagatacttaacagggaagtgagagggccgcggcaaagccgtttttccataggctccgcccccctgacaagcatcacgaaatctgacgctcaaatcagtggtggcgaaacccgacaggactataaagataccaggcgtttccccctggcggctccctcgtgcgctctcctgttcctgcctttcggtttaccggtgtcattccgctgttatggccgcgtttgtctcattccacgcctgacactcagttccgggtaggcagttcgctccaagctggactgtatgcacgaaccccccgttcagtccgaccgctgcgccttatccggtaactatcgtcttgagtccaacccggaaagacatgcaaaagcaccactggcagcagccactggtaattgatttagaggagttagtcttgaagtcatgcgccggttaaggctaaactgaaaggacaagttttggtgactgcgctcctccaagccagttacctcggttcaaagagttggtagctcagagaaccttcgaaaaaccgccctgcaaggcggttttttcgttttcagagcaagagattacgcgcagaccaaaacgatctcaagaagatcatcttattaatcagataaaatatttgctcatgagcccgaagtggcgagcccgatcttccccatcggtgatgtcggcgatataggcgccagcaaccgcacctgtggcgccggtgatgccggccacgatgcgtccggcgtagaggatctgctcatgtttgacagcttatc

SEQ ID NO: 106 - DNA, 6076 bp, synthetic
  plasmid (1)..(6076): pENDU5CAM
  CDS (108)..(911): ompA-lysostaphin
gatctcgatcccgcgaaattaatacgactcactataggggaattgtgagcggataacaattcccctctagaaataattttgtttaactttaagaaggagatatacatatgaaaaagacagctatcgcgattgcagtggcactggctggtttcgctaccgtagcgcaggctgcagcaacccatgaacatagcgcacagtggctgaataattacaaaaaaggttatggctatggtccgtatccgctgggtattaatggtggtatgcattatggtgtggatttctttatgaatattggcacaccggttaaagcaattagcagcggtaaaattgttgaagcaggttggagcaattatggtggtggtaatcagattggcctgattgaaaatgatggtgttcatcgtcagtggtatatgcatctgagcaaatacaatgtgaaagtgggcgattatgttaaagccggtcagattattggttggagcggtagcaccggttatagtaccgcaccgcatctgcattttcagcgtatggttaatagctttagcaatagcaccgcacaggatccgatgccgtttctgaaaagcgcaggttatggtaaagcaggcggtacagttaccccgacaccgaataccggttggaaaaccaacaaatatggcaccctgtataaaagcgaaagcgcaagctttaccccgaatacagatattatcacccgtaccaccggtccgtttcgtagcatgccgcagagcggtgttctgaaagcaggtcagaccattcattatgatgaagtgatgaaacaggatggtcatgtttgggttggttataccggtaatagcggtcagcgtatttatctgccggttcgtacctggaataaaagcaccaatacactgggtgttctgtggggcaccatcaaataatgagatccggctgctaacaaagcccgaaaggaagctgagttggctgctgccaccgctgagcaataactagcataaccccttggggcctctaaacgggtcttgaggggttttttgctgaaaggaggaactatatccggattggcgaatgggacgcgccctgtagcggcgcattaagcgcggcgggtgtggtggttacgcgcagcgtgaccgctacacttgccagcgccctagcgcccgctcctttcgctttcttcccttcctttctcgccacgttcgccggctttccccgtcaagctctaaatcgggggctccctttagggttccgatttagtgctttacggcacctcgaccccaaaaaacttgattagggtgatggttcacgtagtgggccatcgccctgatagacggtttttcgccctttgacgttggagtccacgttctttaatagtggactcttgttccaaactggaacaacactcaaccctatctcggtctattcttttgatttataagggattttgccgatttcggcctattggttaaaaaatgagctgatttaacaaaaatttaacgcgaattttaacaaaatattaacgtttacaatttcaggtggcacttttcggggaaatgtgcgcggaacccctatttgtttatttttctaaatacattcaaatatgtatccgctcaataactgccttaaaaaaattacgccccgccctgccactcatcgcagtactgttgtaattcattaagcattctgccgacatggaagccatcacagacggcatgatgaacctgaatcgccagcggcatcagcaccttgtcgccttgcgtataatatttgcccatggtgaaaacgggggcgaagaagttgtccatattggccacgtttaaatcaaaactggtgaaactcacccagggattggctgagacgaaaaacatattctcaataaaccctttagggaaataggccaggttttcaccgtaacacgccacatcttgcgaatatatgtgtagaaactgccggaaatcgtcgtggtattcactccagagcgatgaaaacgtttcagtttgctcatggaaaacggtgtaacaagggtgaacactatcccatatcaccagctcaccgtctttcattgccatacggaattccggatgagcattcatcaggcgggcaagaatgtgaataaaggccggataaaacttgtgcttatttttctttacggtctttaaaaaggccgtaatatccagctgaacggtctggttataggtacattgagcaactgactgaaatgcctcaaaatgttctttacgatgccattgggatatatcaacggtggtatatccagtgatttttttctccattttagcttccttagctcctgaaaatctcgataactcaaaaaatacgcccggtagtgatcttatttcattatggtgaaagttggaacctcttacgtgccgatcaacgtctcattttcgccaaaagttggcccagggcttcccggtatcaacagggacaccaggatttatttattctgcgaagtgatcttccgtcacaggtatttattcggcgcaaagtgcgtcattgttcatgaccaaaatcccttaacgtgagttttcgttccactgagcgtcagaccccgtagaaaagattgttcatgaccaaaatcccttaacgtgatcaaaggatcttcttgagatcctttttttctgcgcgtaatctgctgcttgcaaacaaaaaaaccaccgctaccagcggtggtttgtttgccggatcaagagctaccaactctttttccgaaggtaactggcttcagcagagcgcagataccaaatactgtccttctagtgtagccgtagttaggccaccacttcaagaactctgtagcaccgcctacatacctcgctctgctaatcctgttaccagtggctgctgccagtggcgataagtcgtgtcttaccgggttggactcaagacgatagttaccggataaggcgcagcggtcgggctgaacggggggttcgtgcacacagcccagcttggagcgaacgacctacaccgaactgagatacctacagcgtgagctatgagaaagcgccacgcttcccgaagggagaaaggcggacaggtatccggtaagcggcagggtcggaacaggagagcgcacgagggagcttccagggggaaacgcctggtatctttatagtcctgtcgggtttcgccacctctgacttgagcgtcgatttttgtgatgctcgtcaggggggcggagcctatggaaaaacgccagcaacgcggcctttttacggttcctggccttttgctggccttttgctcacatgttctttcctgcgttatcccctgattctgtggataaccgtattaccgcctttgagtgagctgataccgctcgccgcagccgaacgaccgagcgcagcgagtcagtgagcgaggaagcggaagagcgcctgatgcggtattttctccttacgcatctgtgcggtatttcacaccgcatatatggtgcactctcagtacaatctgctctgatgccgcatagttaagccagtatacactccgctatcgctacgtgactgggtcatggctgcgccccgacacccgccaacacccgctgacgcgccctgacgggcttgtctgctcccggcatccgcttacagacaagctgtgaccgtctccgggagctgcatgtgtcagaggttttcaccgtcatcaccgaaacgcgcgaggcagctgcggtaaagctcatcagcgtggtcgtgaagcgattcacagatgtctgcctgttcatccgcgtccagctcgttgagtttctccagaagcgttaatgtctggcttctgataaagcgggccatgttaagggcggttttttcctgtttggtcactgatgcctccgtgtaagggggatttctgttcatgggggtaatgataccgatgaaacgagagaggatgctcacgatacgggttactgatgatgaacatgcccggttactggaacgttgtgagggtaaacaactggcggtatggatgcggcgggaccagagaaaaatcactcagggtcaatgccagcgcttcgttaatacagatgtaggtgttccacagggtagccagcagcatcctgcgatgcagatccggaacataatggtgcagggcgctgacttccgcgtttccagactttacgaaacacggaaaccgaagaccattcatgttgttgctcaggtcgcagacgttttgcagcagcagtcgcttcacgttcgctcgcgtatcggtgattcattctgctaaccagtaaggcaaccccgccagcctagccgggtcctcaacgacaggagcacgatcatgcgcacccgtggggccgccatgccggcgataatggcctgcttctcgccgaaacgtttggtggcgggaccagtgacgaaggcttgagcgagggcgtgcaagattccgaataccgcaagcgacaggccgatcatcgtcgcgctccagcgaaagcggtcctcgccgaaaatgacccagagcgctgccggcacctgtcctacgagttgcatgataaagaagacagtcataagtgcggcgacgatagtcatgccccgcgcccaccggaaggagctgactgggttgaaggctctcaagggcatcggtcgagatcccggtgcctaatgagtgagctaacttacattaattgcgttgcgctcactgcccgctttccagtcgggaaacctgtcgtgccagctgcattaatgaatcggccaacgcgcggggagaggcggtttgcgtattgggcgccagggtggtttttcttttcaccagtgagacgggcaacagctgattgcccttcaccgcctggccctgagagagttgcagcaagcggtccacgctggtttgccccagcaggcgaaaatcctgtttgatggtggttaacggcgggatataacatgagctgtcttcggtatcgtcgtatcccactaccgagatatccgcaccaacgcgcagcccggactcggtaatggcgcgcattgcgcccagcgccatctgatcgttggcaaccagcatcgcagtgggaacgatgccctcattcagcatttgcatggtttgttgaaaaccggacatggcactccagtcgccttcccgttccgctatcggctgaatttgattgcgagtgagatatttatgccagccagccagacgcagacgcgccgagacagaacttaatgggcccgctaacagcgcgatttgctggtgacccaatgcgaccagatgctccacgcccagtcgcgtaccgtcttcatgggagaaaataatactgttgatgggtgtctggtcagagacatcaagaaataacgccggaacattagtgcaggcagcttccacagcaatggcatcctggtcatccagcggatagttaatgatcagcccactgacgcgttgcgcgagaagattgtgcaccgccgctttacaggcttcgacgccgcttcgttctaccatcgacaccaccacgctggcacccagttgatcggcgcgagatttaatcgccgcgacaatttgcgacggcgcgtgcagggccagactggaggtggcaacgccaatcagcaacgactgtttgcccgccagttgttgtgccacgcggttgggaatgtaattcagctccgccatcgccgcttccactttttcccgcgttttcgcagaaacgtggctggcctggttcaccacgcgggaaacggtctgataagagacaccggcatactctgcgacatcgtataacgttactggtttcacattcaccaccctgaattgactctcttccgggcgctatcatgccataccgcgaaaggttttgcgccattcgatggtgtccgggatctcgacgctctcccttatgcgactcctgcattaggaagcagcccagtagtaggttgaggccgttgagcaccgccgccgcaaggaatggtgcatgcaaggagatggcgcccaacagtcccccggccacggggcctgccaccatacccacgccgaaacaagcgctcatgagcccgaagtggcgagcccgatcttccccatcggtgatgtcggcgatataggcgccagcaaccgcacctgtggcgccggtgatgccggccacgatgcgtccggcgtagaggatcga

SEQ ID NO: 107 - protein, 267 aa, synthetic
MKKTAIAIAVALAGFATVAQAAATHEHSAQWLNNYKKGYGYGPYPLGINGGMHYGVDFFMNIGTPVKAISSGKIVEAGWSNYGGGNQIGLIENDGVHRQWYMHLSKYNVKVGDYVKAGQIIGWSGSTGYSTAPHLHFQRMVNSFSNSTAQDPMPFLKSAGYGKAGGTVTPTPNTGWKTNKYGTLYKSESASFTPNTDIITRTTGPFRSMPQSGVLKAGQTIHYDEVMKQDGHVWVGYTGNSGQRIYLPVRTWNKSTNTLGVLWGTIK

SEQ ID NO: 108 - DNA, 8593 bp, synthetic
  plasmid (1)..(8593): pMevT
  CDS (380)..(1564): Acetyl-CoA_acetyltransferase
  CDS (1578)..(3053): 3-hydroxy-3-methylglutaryl-coenzyme_A_synthase
  CDS (3067)..(4575): N-Terminally_Truncated_3-Hydroxy-3-Methylglutaryl_Coenzyme_A_Redu ctase
atcgatgcatgcgcccaatacgcaaaccgcctctccccgcgcgttggccgattcattaatgcagctggcacgacaggtttcccgactggaaagcgggcagtgagcgcaacgcaattaatgtgagttagctcactcattaggcaccccaggctttacactttatgcttccggctcgtatgttgtgtggaattgtgagcggataacaatttcacacaggaaacagctatgaccatgattacgccaagcgcgcaattaaccctcactaaagggaacaaaagctgggtaccgggccccccctcgaggtcgacggtatcgataagcttgatatcgaattcctgcagcccggggatcctctagagtcgactaggaggaatataaaatgaaaaattgtgtcatcgtcagtgcggtacgtactgctatcggtagttttaacggttcactcgcttccaccagcgccatcgacctgggggcgacagtaattaaagccgccattgaacgtgcaaaaatcgattcacaacacgttgatgaagtgattatgggtaacgtgttacaagccgggctggggcaaaatccggcgcgtcaggcactgttaaaaagcgggctggcagaaacggtgtgcggattcacggtcaataaagtatgtggttcgggtcttaaaagtgtggcgcttgccgcccaggccattcaggcaggtcaggcgcagagcattgtggcggggggtatggaaaatatgagtttagccccctacttactcgatgcaaaagcacgctctggttatcgtcttggagacggacaggtttatgacgtaatcctgcgcgatggcctgatgtgcgccacccatggttatcatatggggattaccgccgaaaacgtggctaaagagtacggaattacccgtgaaatgcaggatgaactggcgctacattcacagcgtaaagcggcagccgcaattgagtccggtgcttttacagccgaaatcgtcccggtaaatgttgtcactcgaaagaaaaccttcgtcttcagtcaagacgaattcccgaaagcgaattcaacggctgaagcgttaggtgcattgcgcccggccttcgataaagcaggaacagtcaccgctgggaacgcgtctggtattaacgacggtgctgccgctctggtgattatggaagaatctgcggcgctggcagcaggccttacccccctggctcgcattaaaagttatgccagcggtggcgtgccccccgcattgatgggtatggggccagtacctgccacgcaaaaagcgttacaactggcggggctgcaactggcggatattgatctcattgaggctaatgaagcatttgctgcacagttccttgccgttgggaaaaacctgggctttgattctgagaaagtgaatgtcaacggcggggccatcgcgctcgggcatcctatcggtgccagtggtgctcgtattctggtcacactattacatgccatgcaggcacgcgataaaacgctggggctggcaacactgtgcattggcggcggtcagggaattgcgatggtgattgaacggttgaattaaggaggacagctaaatgaaactctcaactaaactttgttggtgtggtattaaaggaagacttaggccgcaaaagcaacaacaattacacaatacaaacttgcaaatgactgaactaaaaaaacaaaagaccgctgaacaaaaaaccagacctcaaaatgtcggtattaaaggtatccaaatttacatcccaactcaatgtgtcaaccaatctgagctagagaaatttgatggcgtttctcaaggtaaatacacaattggtctgggccaaaccaacatgtcttttgtcaatgacagagaagatatctactcgatgtccctaactgttttgtctaagttgatcaagagttacaacatcgacaccaacaaaattggtagattagaagtcggtactgaaactctgattgacaagtccaagtctgtcaagtctgtcttgatgcaattgtttggtgaaaacactgacgtcgaaggtattgacacgcttaatgcctgttacggtggtaccaacgcgttgttcaactctttgaactggattgaatctaacgcatgggatggtagagacgccattgtagtttgcggtgatattgccatctacgataagggtgccgcaagaccaaccggtggtgccggtactgttgctatgtggatcggtcctgatgctccaattgtatttgactctgtaagagcttcttacatggaacacgcctacgatttttacaagccagatttcaccagcgaatatccttacgtcgatggtcatttttcattaacttgttacgtcaaggctcttgatcaagtttacaagagttattccaagaaggctatttctaaagggttggttagcgatcccgctggttcggatgctttgaacgttttgaaatatttcgactacaacgttttccatgttccaacctgtaaattggtcacaaaatcatacggtagattactatataacgatttcagagccaatcctcaattgttcccagaagttgacgccgaattagctactcgcgattatgacgaatctttaaccgataagaacattgaaaaaacttttgttaatgttgctaagccattccacaaagagagagttgcccaatctttgattgttccaacaaacacaggtaacatgtacaccgcatctgtttatgccgcctttgcatctctattaaactatgttggatctgacgacttacaaggcaagcgtgttggtttattttcttacggttccggtttagctgcatctctatattcttgcaaaattgttggtgacgtccaacatattatcaaggaattagatattactaacaaattagccaagagaatcaccgaaactccaaaggattacgaagctgccatcgaattgagagaaaatgcccatttgaagaagaacttcaaacctcaaggttccattgagcatttgcaaagtggtgtttactacttgaccaacatcgatgacaaatttagaagatcttacgatgttaaaaaataaggaggattacactatggttttaaccaataaaacagtcatttctggatcgaaagtcaaaagtttatcatctgcgcaatcgagctcatcaggaccttcatcatctagtgaggaagatgattcccgcgatattgaaagcttggataagaaaatacgtcctttagaagaattagaagcattattaagtagtggaaatacaaaacaattgaagaacaaagaggtcgctgccttggttattcacggtaagttacctttgtacgctttggagaaaaaattaggtgatactacgagagcggttgcggtacgtaggaaggctctttcaattttggcagaagctcctgtattagcatctgatcgtttaccatataaaaattatgactacgaccgcgtatttggcgcttgttgtgaaaatgttataggttacatgcctttgcccgttggtgttataggccccttggttatcgatggtacatcttatcatataccaatggcaactacagagggttgtttggtagcttctgccatgcgtggctgtaaggcaatcaatgctggcggtggtgcaacaactgttttaactaaggatggtatgacaagaggcccagtagtccgtttcccaactttgaaaagatctggtgcctgtaagatatggttagactcagaagagggacaaaacgcaattaaaaaagcttttaactctacatcaagatttgcacgtctgcaacatattcaaacttgtctagcaggagatttactcttcatgagatttagaacaactactggtgacgcaatgggtatgaatatgatttctaaaggtgtcgaatactcattaaagcaaatggtagaagagtatggctgggaagatatggaggttgtctccgtttctggtaactactgtaccgacaaaaaaccagctgccatcaactggatcgaaggtcgtggtaagagtgtcgtcgcagaagctactattcctggtgatgttgtcagaaaagtgttaaaaagtgatgtttccgcattggttgagttgaacattgctaagaatttggttggatctgcaatggctgggtctgttggtggatttaacgcacatgcagctaatttagtgacagctgttttcttggcattaggacaagatcctgcacaaaatgttgaaagttccaactgtataacattgatgaaagaagtggacggtgatttgagaatttccgtatccatgccatccatcgaagtaggtaccatcggtggtggtactgttctagaaccacaaggtgccatgttggacttattaggtgtaagaggcccgcatgctaccgctcctggtaccaacgcacgtcaattagcaagaatagttgcctgtgccgtcttggcaggtgaattatccttatgtgctgccctagcagccggccatttggttcaaagtcatatgacccacaacaggaaacctgctgaaccaacaaaacctaacaatttggacgccactgatataaatcgtttgaaagatgggtccgtcacctgcattaaatcctaagtcgacctgcaggcatgcaagcttggctgttttggcggatgagagaagattttcagcctgatacagattaaatcagaacgcagaagcggtctgataaaacagaatttgcctggcggcagtagcgcggtggtcccacctgaccccatgccgaactcagaagtgaaacgccgtagcgccgatggtagtgtggggtctccccatgcgagagtagggaactgccaggcatcaaataaaacgaaaggctcagtcgaaagactgggcctttcgttttatctgttgtttgtcggtgaacgctctcctgagtaggacaaatccgccgggagcggatttgaacgttgcgaagcaacggcccggagggtggcgggcaggacgcccgccataaactgccaggcatcaaattaagcagaaggccatcctgacggatggcctttttgcgtttctacaaactcttttgtttatttttctaaatacattcaaatatgtatccgctcatgagacaataaccctgataaatgcttcaataatattgaaaaaggaagagtatgagtattcaacatttccgtgtcgcccttattcccttttttgcggcattttgccttcctgtttttgctcacccagaaacgctggtgaaagtaaaagatgctgaagatcagttgggtgcagcaaactattaactggcgaactacttactctagcttcccggcaacaattaatagactggatggaggcggataaagttgcaggaccacttctgcgctcggcccttccggctggctggtttattgctgataaatctggagccggtgagcgtgggtctcgcggtatcattgcagcactggggccagatggtaagccctcccgtatcgtagttatctacacgacggggagtcaggcaactatggatgaacgaaatagacagatcgctgagataggtgcctcactgattaagcattggtaactgtcagaccaagtttactcatatatactttagattgatttacgcgccctgtagcggcgcattaagcgcggcgggtgtggtggttacgcgcagcgtgaccgctacacttgccagcgccctagcgcccgctcctttcgctttcttcccttcctttctcgccacgttcgccggctttccccgtcaagctctaaatcgggggctccctttagggttccgatttagtgctttacggcacctcgaccccaaaaaacttgatttgggtgatggttcacgtagtgggccatcgccctgatagacggtttttcgccctttgacgttggagtccacgttctttaatagtggactcttgttccaaacttgaacaacactcaaccctatctcgggctattcttttgatttataagggattttgccgatttcggcctattggttaaaaaatgagctgatttaacaaaaatttaacgcgaattttaacaaaatattaacgtttacaatttaaaaggatctaggtgaagatcctttttgataatctcatgaccaaaatcccttaacgtgagttttcgttccactgagcgtcagaccccgtagaaaagatcaaaggatcttcttgagatcctttttttctgcgcgtaatctgctgcttgcaaacaaaaaaaccaccgctaccagcggtggtttgtttgccggatcaagagctaccaactctttttccgaaggtaactggcttcagcagagcgcagataccaaatactgtccttctagtgtagccgtagttaggccaccacttcaagaactctgtagcaccgcctacatacctcgctctgctaatcctgttaccagtggggcatttgagaagcacacggtcacactgcttccggtagtcaataaaccggtaaaccagcaatagacataagcggctatttaacgaccctgccctgaaccgacgaccgggtcgaatttgctttcgaatttctgccattcatccgcttattatcacttattcaggcgtagcaccaggcgtttaagggcaccaataactgccttaaaaaaattacgccccgccctgccactcatcgcagtactgttgtaattcattaagcattctgccgacatggaagccatcacagacggcatgatgaacctgaatcgccagcggcatcagcaccttgtcgccttgcgtataatatttgcccatggtgaaaacgggggcgaagaagttgtccatattggccacgtttaaatcaaaactggtgaaactcacccagggattggctgagacgaaaaacatattctcaataaaccctttagggaaataggccaggttttcaccgtaacacgccacatcttgcgaatatatgtgtagaaactgccggaaatcgtcgtggtattcactccagagcgatgaaaacgtttcagtttgctcatggaaaacggtgtaacaagggtgaacactatcccatatcaccagctcaccgtctttcattgccatacggaattccggatgagcattcatcaggcgggcaagaatgtgaataaaggccggataaaacttgtgcttatttttctttacggtctttaaaaaggccgtaatatccagctgaacggtctggttataggtacattgagcaactgactgaaatgcctcaaaatgttctttacgatgccattgggatatatcaacggtggtatatccagtgatttttttctccattttagcttccttagctcctgaaaatctcgataactcaaaaaatacgcccggtagtgatcttatttcattatggtgaaagttggaacctcttacgtgccgatcaacgtctcattttcgccaaaagttggcccagggcttcccggtatcaacagggacaccaggatttatttattctgcgaagtgatcttccgtcacaggtatttattcggcgcaaagtgcgtcgggtgatgctgccaacttactgatttagtgtatgatggtgtttttgaggtgctccagtggcttctgtttctatcagctgtccctcctgttcagctactgacggggtggtgcgtaacggcaaaagcaccgccggacatcagcgctagcggagtgtatactggcttactatgttggcactgatgagggtgtcagtgaagtgcttcatgtggcaggagaaaaaaggctgcaccggtgcgtcagcagaatatgtgatacaggatatattccgcttcctcgctcactgactcgctacgctcggtcgttcgactgcggcgagcggaaatggcttacgaacggggcggagatttcctggaagatgccaggaagatacttaacagggaagtgagagggccgcggcaaagccgtttttccataggctccgcccccctgacaagcatcacgaaatctgacgctcaaatcagtggtggcgaaacccgacaggactataaagataccaggcgtttccccctggcggctccctcgtgcgctctcctgttcctgcctttcggtttaccggtgtcattccgctgttatggccgcgtttgtctcattccacgcctgacactcagttccgggtaggcagttcgctccaagctggactgtatgcacgaaccccccgttcagtccgaccgctgcgccttatccggtaactatcgtcttgagtccaacccggaaagacatgcaaaagcaccactggcagcagccactggtaattgatttagaggagttagtcttgaagtcatgcgccggttaaggctaaactgaaaggacaagttttggtgactgcgctcctccaagccagttacctcggttcaaagagttggtagctcagagaaccttcgaaaaaccgccctgcaaggcggttttttcgttttcagagcaagagattacgcgcagaccaaaacgatctcaagaagatcatcttattaatcagataaaatatttgctcatgagcccgaagtggcgagcccgatcttccccatcggtgatgtcggcgatataggcgccagcaaccgcacctgtggcgccggtgatgccggccacgatgcgtccggcgtagaggatctgctcatgtttgacagcttatc

SEQ ID NO: 109 - protein, 394 aa, synthetic
MKNCVIVSAVRTAIGSFNGSLASTSAIDLGATVIKAAIERAKIDSQHVDEVIMGNVLQAGLGQNPARQALLKSGLAETVCGFTVNKVCGSGLKSVALAAQAIQAGQAQSIVAGGMENMSLAPYLLDAKARSGYRLGDGQVYDVILRDGLMCATHGYHMGITAENVAKEYGITREMQDELALHSQRKAAAAIESGAFTAEIVPVNVVTRKKTFVFSQDEFPKANSTAEALGALRPAFDKAGTVTAGNASGINDGAAALVIMEESAALAAGLTPLARIKSYASGGVPPALMGMGPVPATQKALQLAGLQLADIDLIEANEAFAAQFLAVGKNLGFDSEKVNVNGGAIALGHPIGASGARILVTLLHAMQARDKTLGLATLCIGGGQGIAMVIERLN

SEQ ID NO: 110 - protein, 491 aa, synthetic
MKLSTKLCWCGIKGRLRPQKQQQLHNTNLQMTELKKQKTAEQKTRPQNVGIKGIQIYIPTQCVNQSELEKFDGVSQGKYTIGLGQTNMSFVNDREDIYSMSLTVLSKLIKSYNIDTNKIGRLEVGTETLIDKSKSVKSVLMQLFGENTDVEGIDTLNACYGGTNALFNSLNWIESNAWDGRDAIVVCGDIAIYDKGAARPTGGAGTVAMWIGPDAPIVFDSVRASYMEHAYDFYKPDFTSEYPYVDGHFSLTCYVKALDQVYKSYSKKAISKGLVSDPAGSDALNVLKYFDYNVFHVPTCKLVTKSYGRLLYNDFRANPQLFPEVDAELATRDYDESLTDKNIEKTFVNVAKPFHKERVAQSLIVPTNTGNMYTASVYAAFASLLNYVGSDDLQGKRVGLFSYGSGLAASLYSCKIVGDVQHIIKELDITNKLAKRITETPKDYEAAIELRENAHLKKNFKPQGSIEHLQSGVYYLTNIDDKFRRSYDVKK

SEQ ID NO: 111 - protein, 502 aa, synthetic
MVLTNKTVISGSKVKSLSSAQSSSSGPSSSSEEDDSRDIESLDKKIRPLEELEALLSSGNTKQLKNKEVAALVIHGKLPLYALEKKLGDTTRAVAVRRKALSILAEAPVLASDRLPYKNYDYDRVFGACCENVIGYMPLPVGVIGPLVIDGTSYHIPMATTEGCLVASAMRGCKAINAGGGATTVLTKDGMTRGPVVRFPTLKRSGACKIWLDSEEGQNAIKKAFNSTSRFARLQHIQTCLAGDLLFMRFRTTTGDAMGMNMISKGVEYSLKQMVEEYGWEDMEVVSVSGNYCTDKKPAAINWIEGRGKSVVAEATIPGDVVRKVLKSDVSALVELNIAKNLVGSAMAGSVGGFNAHAANLVTAVFLALGQDPAQNVESSNCITLMKEVDGDLRISVSMPSIEVGTIGGGTVLEPQGAMLDLLGVRGPHATAPGTNARQLARIVACAVLAGELSLCAALAAGHLVQSHMTHNRKPAEPTKPNNLDATDINRLKDGSVTCIKS

SEQ ID NO: 112 - DNA, 32 bp, synthetic
  primer (1)..(32): yccV forward primer
attcatatguggttataaagacatcaacatgc

SEQ ID NO: 113 - DNA, 90 bp, synthetic
  primer (1)..(90): yccV reverse primer
  misc_feature (65)..(65): N is A, T, C or G
atccccattacgtgaggatggctaaggtccagtgaagtaccctgggcaaagagtttcataccttncaagtagtcacctcccgggaaatct

SEQ ID NO: 114 - DNA, 32 bp, synthetic
  primer (1)..(32): ycjX forward primer
attcatatguttggctgatactgtaattcttc

SEQ ID NO: 115 - DNA, 90 bp, synthetic
  primer (1)..(90): ycjX reverse primer
  misc_feature (65)..(65): N is A, T, C or G
atccccattacgtgaggatggctaaggtccagtgaagtaccctgggcaaagagtttcataccttncaagttgctgtcctgtgctgctctg

SEQ ID NO: 116 - DNA, 32 bp, synthetic
  primer (1)..(32): mutM forward primer
attcatatguggcgaaaagtactaagtactta

SEQ ID NO: 117 - DNA, 90 bp, synthetic
  primer (1)..(90): mutM reverse primer
  misc_feature (65)..(65): N is A, T, C or G
atccccattacgtgaggatggctaaggtccagtgaagtaccctgggcaaagagtttcataccttncaagtagcatctccaggaatgaaca

SEQ ID NO: 118 - DNA, 19 bp, synthetic
  primer (1)..(19): primer P492
tgcaactcttcttcaacgc

SEQ ID NO: 119 - DNA, 19 bp, synthetic
  primer (1)..(19): primer P493
aagaaccaggcgcttctaa

SEQ ID NO: 120 - DNA, 19 bp, synthetic
  primer (1)..(19): primer P525
attgatgacctgatggcac

SEQ ID NO: 121 - DNA, 18 bp, synthetic
  primer (1)..(18): primer P526
gatccagacttcgaagcg

SEQ ID NO: 122 - DNA, 90 bp, synthetic
  primer (1)..(90): ibpA forward primer
  misc_feature (65)..(65): N is A, T, C or G
atccccattacgtgaggatggctaaggtccagtgaagtaccctgggcaaagagtttcataccttncaagtaatcaatagctcctgaaatc

SEQ ID NO: 123 - DNA, 31 bp, synthetic
  primer (1)..(31): ibpA reverse primer
  misc_feature (65)..(65): N is A, T, C or G
attcatatgtttggcctgatgagttatagcg

SEQ ID NO: 124 - DNA, 32 bp, synthetic
  primer (1)..(32): grpE forward primer
attcatatgutctccgcgagcgtgccagtttt

SEQ ID NO: 125 - DNA, 90 bp, synthetic
  primer (1)..(90): grpE reverse primer
  misc_feature (65)..(65): N is A, T, C or G
atccccattacgtgaggatggctaaggtccagtgaagtaccctgggcaaagagtttcataccttncaagtgaatttctccgcgttttttt

SEQ ID NO: 126 - DNA, 32 bp, synthetic
  primer (1)..(32): ldhA forward primer
attcatatgugggaacccacagcccgagcgtc

SEQ ID NO: 127 - DNA, 90 bp, synthetic
  primer (1)..(90): ldhA reverse primer
  misc_feature (65)..(65): N is A, T, C or G
atccccattacgtgaggatggctaaggtccagtgaagtaccctgggcaaagagtttcataccttncaagtaagactttctccagtgatgt

SEQ ID NO: 128 - DNA, 122 bp, synthetic
  primer (1)..(122): ybbN forward primer
  misc_feature (97)..(97): N is A, T, C or G
attcatatgucccattcgtactcgcttcaccgatccccattacgtgaggatggctaaggtccagtgaagtaccctgggcaaagagtttcataccttncaagtggagtcgctctctgttgtcg

SEQ ID NO: 129 - DNA, 90 bp, synthetic
  primer (1)..(90): ybbN reverse primer
  misc_feature (65)..(65): N is A, T, C or G
atccccattacgtgaggatggctaaggtccagtgaagtaccctgggcaaagagtttcataccttncaagtggagtcgctctctgttgtcg

SEQ ID NO: 130 - DNA, 32 bp, synthetic
  primer (1)..(32): fxsA forward primer
attcatatgutaaacacacagaatatatgtgg

SEQ ID NO: 131 - DNA, 90 bp, synthetic
  primer (1)..(90): fxsA reverse primer
  misc_feature (65)..(65): N is A, T, C or G
atccccattacgtgaggatggctaaggtccagtgaagtaccctgggcaaagagtttcataccttncaagtaggtttctcctgtaatagca

SEQ ID NO: 132 - DNA, 31 bp, synthetic
  primer (1)..(31): rrnB forward primer
attcatatgugcaaacacgccgccgggtcag

SEQ ID NO: 133 - DNA, 90 bp, synthetic
  primer (1)..(90): rrnB reverse primer
  misc_feature (65)..(65): N is A, T, C or G
atccccattacgtgaggatggctaaggtccagtgaagtaccctgggcaaagagtttcataccttncaagtaaaagtttgacgctcaaaga

SEQ ID NO: 134 - DNA, 35 bp, synthetic
  primer (1)..(35): rrnE forward primer
attcatatguaatgcgcctccgttgagacgacaac

SEQ ID NO: 135 - DNA, 90 bp, synthetic
  primer (1)..(90): rrnE reverse primer
  misc_feature (65)..(65): N is A, T, C or G
atccccattacgtgaggatggctaaggtccagtgaagtaccctgggcaaagagtttcataccttncaagtaaaagtttgatgctcaaaga

SEQ ID NO: 136 - DNA, 32 bp, synthetic
  primer (1)..(32): poxB forwrad primer
attcatatgutaggttgtcgctgcctgccgtg

SEQ ID NO: 137 - DNA, 90 bp, synthetic
  primer (1)..(90): poxB reverse primer
  misc_feature (65)..(65): N is A, T, C or G
atccccattacgtgaggatggctaaggtccagtgaagtaccctgggcaaagagtttcataccttncaagtggttctccatctcctgaatg

SEQ ID NO: 138 - DNA, 32 bp, synthetic
  primer (1)..(32): cspD forward primer
attcatatgucggttatcggcagaacgccctg

SEQ ID NO: 139 - DNA, 90 bp, synthetic
  primer (1)..(90): cspD reverse primer
  misc_feature (65)..(65): N is A, T, C or G
atccccattacgtgaggatggctaaggtccagtgaagtaccctgggcaaagagtttcataccttncaagtgcttcgacatccttcgcaaa

SEQ ID NO: 140 - DNA, 1902 bp, synthetic
  integration sequence s9_pmutM_folP (1)..(1902)
  CDS (299)..(1093): kanR
  promoter (1533)..(1832): burden sensing promoter p(mutM)
  RBS (1833)..(1838): rbs catalog
  misc_feature (1838)..(1838): N is A, T, C or G
  gene (1844)..(1902): beginning of folP gene
aagaaccaggcgcttctaacaattctggcgacaatggtagtccaaaggctcctcgtccggttgatgaaccgcgtacgccgaacccgggtaacaccatgtcagagcagttaggcgacaagtaagttcccgcatcagatgactgtatttgtaccgaaaaccccggggcgtgctccggggttttttcttatcaattcataccagggataacatcagcgattgtgtaggctggagctgcttcgaagttcctatactttctagagaataggaacttcggaataggaacttcaagatccccttattagaagaactcgtcaagaaggcgatagaaggcgatgcgctgcgaatcgggagcggcgataccgtaaagcacgaggaagcggtcagcccattcgccgccaagctcttcagcaatatcacgggtagccaacgctatgtcctgatagcggtccgccacacccagccggccacagtcgatgaatccagaaaagcggccattttccaccatgatattcggcaagcaggcatcgccatgggtcacgacgagatcctcgccgtcgggcatgcgcgccttgagcctggcgaacagttcggctggcgcgagcccctgatgctcttcgtccagatcatcctgatcgacaagaccggcttccatccgagtacgtgctcgctcgatgcgatgtttcgcttggtggtcgaatgggcaggtagccggatcaagcgtatgcagccgccgcattgcatcagccatgatggatactttctcggcaggagcaaggtgagatgacaggagatcctgccccggcacttcgcccaatagcagccagtcccttcccgcttcagtgacaacgtcgagcacagctgcgcaaggaacgcccgtcgtggccagccacgatagccgcgctgcctcgtcctgcagttcattcagggcaccggacaggtcggtcttgacaaaaagaaccgggcgcccctgcgctgacagccggaacacggcggcatcagagcagccgattgtctgttgtgcccagtcatagccgaatagcctctccacccaagcggccggagaacctgcgtgcaatccatcttgttcaatcatgcgaaacgatcctcatcctgtctcttgatcagatcttgatcccctgcgccatcagatccttggcggcaagaaagccatccagtttactttgcagggcttcccaaccttaccagagggcgccccagctggcaattccggttcgcttgctgtccataaaaccgcccagtctagctatcgccatgtaagcccactgcaagctacctgctttctctttgcgcttgcgttttcccttgtccagatagcccagtagctgacattcatccggggtcagcaccgtttctgcggactggctttctacgtgttccgcttcctttagcagcccttgcgccctgagtgcttgcggcagcgtgagcttcaaaagcgctctgaagttcctatactttctagagaataggaacttcgaactgcaggtcgacggatccccggaatattcatatgtggcgaaaagtactaagtacttagaggaaataaatcatggctaaaggtattcgtgagaaaatcaagctggtttcttctgctggtactggtcacttctataccactacgaagaacaaacgtactaagccggaaaaactggaactgaaaaaattcgatccagttgttcgccagcacgtgatctacaaagaagcgaaaatcaaataattctcgctttgatgtaacaaaaaacctcgctccggcggggttttttgttatctgcttgcccccatattgactgcatctgttcattcctggagatgctacttgnaaggtatgaaactctttgcccagggtacttcactggaccttagccatcctcacgtaatggggat

SEQ ID NO: 141 - protein, 161 aa, synthetic
LEELVKKAIEGDALRIGSGDTVKHEEAVSPFAAKLFSNITGSQRYVLIAVRHTQPATVDESRKAAIFHHDIRQAGIAMGHDEILAVGHARLEPGEQFGWREPLMLFVQIILIDKTGFHPSTCSLDAMFRLVVEWAGSRIKRMQPPHCISHDGYFLGRSKVR

SEQ ID NO: 142 - protein, 10 aa, synthetic
QEILPRHFAQ

SEQ ID NO: 143 - protein, 25 aa, synthetic
QPVPSRFSDNVEHSCARNARRGQPR

SEQ ID NO: 144 - protein, 26 aa, synthetic
PRCLVLQFIQGTGQVGLDKKNRAPLR

SEQ ID NO: 145 - protein, 20 aa, synthetic
QPEHGGIRAADCLLCPVIAE

SEQ ID NO: 146 - protein, 18 aa, synthetic
PLHPSGRRTCVQSILFNH

SEQ ID NO: 147 - DNA, 1347 bp, Bacillus licheniformis
  CDS (1)..(1347): Bacillus licheniformis essential gene glmM
atgggcaagtattttggtacagacggtgtaagaggcgtggcaaacagtgaacttacacctgagctggcctttaaagtcggacgctttggcggatatgtcctaacaaaagataaggagcgtcccaaggttctgatcggccgtgacacgcgcatttcagggcatatgctggaaggggcccttgtagcaggccttctttcgataggagcagaagtcatgcgtctcggcgtgatttcgacgcccggagtcgcatatttgacgaaggctatggacgcggaggcgggtgtgatgatttccgcttcccacaaccctgtccaggacaacggaattaagtttttcggcggcgacggctttaagctttccgatgaacaggagcttgaaatcgagcgtctgatggatcagccggaagatcacctgccaaggcctgtaggcgctgatctgggcatggtgaacgactactttgaaggcggacagaaatatttgcagtttcttaagcagtctgctgatgaagacttcacaggcattcatgtcgcgcttgactgtgcgcacggggcgacatcttcgctggcgacccacctgtttgccgatcttgacgcagatgtatcgacgatggggacttctccgaacggattaaacatcaatgacggagtcggatcaacccaccctgaagccctggcagaatttgtgaaggaaaagggagctgacgtcggcatggcgtttgacggggatggcgaccgcttaatcgctgtcgacgaaaaagggaatatcgtagacggcgatcaaatcatgtacatatgcgcgaagtacttgaagagcgaggggcgcctgacggacaataccgttgtctccacggtgatgagcaacctcggtttctacaaagcgcttgaagcggaaggcattaaaagcgttcagacagcggtcggcgaccgctatgtagtggaggcgatgaaaaagggcggatttaccctcggcggagaacagtcgggacacctgattttccttgattacaatacgacaggcgacggactgctttctgcgatcatgctgatgaacacgattaaaatgacaggcaagccgctgtctgagcttgcggcagagatgcagaagtttccgcagctcctcttgaatgtgaaagtaaccgataaacataaagtaacggaaaacgaaaaggtaaaagcggtcatcgaagaagttgagaaggaaatgaacggtgacggccgcatccttgtgcgcccatccggcaccgagccgcttgtccgtgtcatggctgaagcgaaaacgaaggagctttgcgagaagtacgtaggccgcattgcagatgtcgtgaaagctgaaatgggagcagagtaa

SEQ ID NO: 148 - protein, 448 aa, Bacillus licheniformis
MGKYFGTDGVRGVANSELTPELAFKVGRFGGYVLTKDKERPKVLIGRDTRISGHMLEGALVAGLLSIGAEVMRLGVISTPGVAYLTKAMDAEAGVMISASHNPVQDNGIKFFGGDGFKLSDEQELEIERLMDQPEDHLPRPVGADLGMVNDYFEGGQKYLQFLKQSADEDFTGIHVALDCAHGATSSLATHLFADLDADVSTMGTSPNGLNINDGVGSTHPEALAEFVKEKGADVGMAFDGDGDRLIAVDEKGNIVDGDQIMYICAKYLKSEGRLTDNTVVSTVMSNLGFYKALEAEGIKSVQTAVGDRYVVEAMKKGGFTLGGEQSGHLIFLDYNTTGDGLLSAIMLMNTIKMTGKPLSELAAEMQKFPQLLLNVKVTDKHKVTENEKVKAVIEEVEKEMNGDGRILVRPSGTEPLVRVMAEAKTKELCEKYVGRIADVVKAEMGAE

SEQ ID NO: 149 - DNA, 282 bp, Bacillus licheniformis
  CDS (1)..(282): Bacillus licheniformis essential gene ylaN
ttggcgtctgagattgtagtcgaccatcgtgaaaaagcacttgctctgttaaaacgtgatgctgataaaatcttaaagctgattcaagtgcaaatggacaacttaacgatgcctcaatgtcctctttatgaagaggttttagatacacaaatgttcggactctctagagaaattgattttgctgtccgccttggattagtggatgaagaagagggtaaagaactgctttacaggctggagcgtgaattgtctgcattacatgatgcatttacaaaaaaataa

SEQ ID NO: 150 - protein, 93 aa, Bacillus licheniformis
LASEIVVDHREKALALLKRDADKILKLIQVQMDNLTMPQCPLYEEVLDTQMFGLSREIDFAVRLGLVDEEEGKELLYRLERELSALHDAFTKK

SEQ ID NO: 151 - DNA, 219 bp, Bacillus licheniformis
  CDS (1)..(219): Bacillus licheniformis essential gene infA
atggcgaaagacgatgtaattgaagtggaaggtactgtagtcgaaacgctgccaaacgcaatgttcaaagttgaacttgagaatggccacacggttttggctcacgtatctggtaaaatccgcatgcacttcattcgcattttacctggagacaaagttacggtagaattatctccatatgacttaactcgtggtagaattacgtaccgttacaaataa

SEQ ID NO: 152 - protein, 72 aa, Bacillus licheniformis
MAKDDVIEVEGTVVETLPNAMFKVELENGHTVLAHVSGKIRMHFIRILPGDKVTVELSPYDLTRGRITYRYK

SEQ ID NO: 153 - DNA, 870 bp, Bacillus licheniformis
  CDS (1)..(870): Bacillus licheniformis essential gene dapA
atgaacttcggaaatatcgcaaccgcgatggttacgccctttgacaaaaatgaaaatatcgattttcaaaaactgtcaaagctgatcgattatttactaaacaatgggacggattccctggtcgttgccggaacaaccggagaatcgccgacgctttccgaagaagaaaaggtagcgctcattcaatactctgtcaaggaagcggcaggccgtgccccaatcatcgccggcacgggaagcaacaacacgaaggcgtcgatcaagctgacgaaaaaagctgaagaagccggcgctgacgctgtcatgctcgtcactccgtactacaacaagccttctcaggaaggcatgtaccgccatttcagagcgattgcggaggaaacatcgctgcctgtcatgctttataatgtgccgggaagaacggctgcttcgctcgcaccagagacgacaatccgccttgcggagatcccgaatattatcgccattaaagaagcgagcggcgacctagatgcgataacaaaaatcgtagccgaaacccctgaggactttgcagtttattcaggagatgacagcctgacactgccggcgctgtccgtgggagcgagaggaatcgtttccgttgcatcacacatcatcggaccggaaatgcaggaaatgatcaaacattataccgaggggaacacggctcaggctgctttgatccatcaaaagctgcttccgctgatgaaagggctttttgccgcaccgaacccgtctccattaaagacggctcttcagctgaagggtcttgacgtcgggtccgtccggctccctttgattccgctaaatgaagatgaacgactccgtttaagcagcctgatgaacggcctgtaa

SEQ ID NO: 154 - protein, 289 aa, Bacillus licheniformis
MNFGNIATAMVTPFDKNENIDFQKLSKLIDYLLNNGTDSLVVAGTTGESPTLSEEEKVALIQYSVKEAAGRAPIIAGTGSNNTKASIKLTKKAEEAGADAVMLVTPYYNKPSQEGMYRHFRAIAEETSLPVMLYNVPGRTAASLAPETTIRLAEIPNIIAIKEASGDLDAITKIVAETPEDFAVYSGDDSLTLPALSVGARGIVSVASHIIGPEMQEMIKHYTEGNTAQAALIHQKLLPLMKGLFAAPNPSPLKTALQLKGLDVGSVRLPLIPLNEDERLRLSSLMNGL

SEQ ID NO: 155 - DNA, 2830 bp, synthetic
  promoter (1)..(1000): pAOX1 promoter
  misc_feature (1)..(2830): pAOX1-ALB construct
  CDS (1001)..(2830): cds encoding Human_serum_albumin (hAS) protein
atgttggtattgtgaaatagacgcagatcgggaacactgaaaaataacagttattattcgagatctaacatccaaagacgaaaggttgaatgaaacctttttgccatccgacatccacaggtccattctcacacataagtgccaaacgcaacaggaggggatacactagcagcagaccgttgcaaacgcaggacctccactcctcttctcctcaacacccacttttgccatcgaaaaaccagcccagttattgggcttgattggagctcgctcattccaattccttctattaggctactaacaccatgactttattagcctgtctatcctggcccccctggcgaggttcatgtttgtttatttccgaatgcaacaagctccgcattacacccgaacatcactccagatgagggctttctgagtgtggggtcaaatagtttcatgttccccaaatggcccaaaactgacagtttaaacgctgtcttggaacctaatatgacaaaagcgtgatctcatccaagatgaactaagtttggttcgttgaaatgctaacggccagttggtcaaaaagaaacttccaaaagtcggcataccgtttgtcttgtttggtattgattgacgaatgctcaaaaataatctcattaatgcttagcgcagtctctctatcgcttctgaaccccggtgcacctgtgccgaaacgcaaatggggaaacacccgctttttggatgattatgcattgtctccacattgtatgcttccaagattctggtgggaatactgctgatagcctaacgttcatgatcaaaatttaactgttctaacccctacttgacagcaatatataaacagaaggaagctgccctgtcttaaacctttttttttatcatcattattagcttactttcataattgcgactggttccaattgacaagcttttgattttaacgacttttaacgacaacttgagaagatcaaaaaacaactaattattcgaaacgatgaagtgggtaacctttatttcccttctttttctctttagctcggcttattccaggggtgtgtttcgtcgagatgcacacaagagtgaggttgctcatcggtttaaagatttgggagaagaaaatttcaaagccttggtgttgattgcctttgctcagtatcttcagcagtgtccatttgaagatcatgtaaaattagtgaatgaagtaactgaatttgcaaaaacatgtgttgctgatgagtcagctgaaaattgtgacaaatcacttcataccctttttggagacaaattatgcacagttgcaactcttcgtgaaacctatggtgaaatggctgactgctgtgcaaaacaagaacctgagagaaatgaatgcttcttgcaacacaaagatgacaacccaaacctcccccgattggtgagaccagaggttgatgtgatgtgcactgcttttcatgacaatgaagagacatttttgaaaaaatacttatatgaaattgccagaagacatccttacttttatgccccggaactccttttctttgctaaaaggtataaagctgcttttacagaatgttgccaagctgctgataaagctgcctgcctgttgccaaagctcgatgaacttcgggatgaagggaaggcttcgtctgccaaacagagactcaagtgtgccagtctccaaaaatttggagaaagagctttcaaagcatgggcagtagctcgcctgagccagagatttcccaaagctgagtttgcagaagtttccaagttagtgacagatcttaccaaagtccacacggaatgctgccatggagatctgcttgaatgtgctgatgacagggcggaccttgccaagtatatctgtgaaaatcaagattcgatctccagtaaactgaaggaatgctgtgaaaaacctctgttggaaaaatcccactgcattgccgaagtggaaaatgatgagatgcctgctgacttgccttcattagctgctgattttgttgaaagtaaggatgtttgcaaaaactatgctgaggcaaaggatgtcttcctgggcatgtttttgtatgaatatgcaagaaggcatcctgattactctgtcgtgctgctgctgagacttgccaagacatatgaaaccactctagagaagtgctgtgccgctgcagatcctcatgaatgctatgccaaagtgttcgatgaatttaaacctcttgtggaagagcctcagaatttaatcaaacaaaattgtgagctttttgagcagcttggagagtacaaattccagaatgcgctattagttcgttacaccaagaaagtaccccaagtgtcaactccaactcttgtagaggtctcaagaaacctaggaaaagtgggcagcaaatgttgtaaacatcctgaagcaaaaagaatgccctgtgcagaagactatctatccgtggtcctgaaccagttatgtgtgttgcatgagaaaacgccagtaagtgacagagtcaccaaatgctgcacagaatccttggtgaacaggcgaccatgcttttcagctctggaagtcgatgaaacatacgttcccaaagagtttaatgctgaaacattcaccttccatgcagatatatgcacactttctgagaaggagagacaaatcaagaaacaaactgcacttgttgagctcgtgaaacacaagcccaaggcaacaaaagagcaactgaaagctgttatggatgatttcgcagcttttgtagagaagtgctgcaaggctgacgataaggagacctgctttgccgaggagggtaaaaaacttgttgctgcaagtcaagctgccttaggcttataa

SEQ ID NO: 156 - protein, 609 aa, synthetic [sequence omitted]

SEQ ID NO: 157 - DNA, 3505 bp, synthetic
  misc_feature (1)..(3505): construct KU70(up)-pPDI1-kanMX-terminator-KU70
  misc_feature (1)..(1002): upstream region
  promoter (1002)..(1542): promoter pPDI1
  CDS (1543)..(2352): kanMX
  terminator (2353)..(2555): terminator
  misc_feature (2556)..(3505): downstream region
gctcttcagaagcctaactttaatggggtaaaatatcagcagtaggctgaatatagagcatggcaacgtttacgtcaacagagtttaatagtgaaaactacgataggttcaggcctgtatacccagacgagttgtatcagcaattagtggattatcatgttggtgctaaaggattgtgtgtcgatgttggatgtggctctggccaggcaacgttcaccctgaaaaagtactttgacaaggtcataggatctgatatctcagaaaatcagttggcagtggctaggaaaagacagcctgctggaattgaatttaggttaggaacgggcgaggatttttcttggctaacggagacgccagatgtaatcaccgccgctgaatgcctgcactgggtagacccacagaaattcgttgcaaatgtcgccaattctctaagggatcatggcaccttgagttactggctttatacagaaccaatttttcagaacgaaagggccaatcaggtttacaacaaattcacctacgggtctgactacctgggcccatattgggatcctggccgtacacatttcagaaatcatttaaaggagttgaatcacatcttactggatagcgagctttttgacgaagtgaaaatttctaattttaaacaagaggaaggggtcaaaaacggagatatcttatacttggaaaaagagatgacaatcagtgatttcatcaattttgtatctagttggccttctgtgttttcgtggaagcagcaacgaggaaaggagggtatcctagatgatttttacaacgaactgaacgactgctttgaggggggtaacatgaaagtaatatggaactccgtcctagtatttgccaggaggaagcaaagggttgtataggctttagtacttatagaggaaacggggttacgtgcaagcgcgcatgcctgagctttgaggggggggactttcacatctcttcttctcacacttagccctaacacagagatcaactactcaaggcagcaccaaaagacgccagaaattatatggtccaggaaaaaacaactctctttactacaaaatttgaacaggtgtcctgcctgcggaaactacaaacgatcacacaccctctgcatgcattgcgtaggacaaatcaggagacattggaacgactctgttcctcaacaggaggcatttcgtgaagagtttgttaatcctttggatgagaagattctttatccaggaaagaaagaactgcccgatgaacgaactttacgtaagaaggagtggctgaagagaagaccccgaacactccctgttgaatagaacacgaacactgtaaatagaataaaagaaaacttggatagtagaacttcaatgtagtgtttctattgtcttacgcggctctttagattgcaatccccagaatggaatcgtccatctttctcaacccactcaaagataatctaccagacatacctacgccctccatcccagcaccacgtcgcgatcacccctaaaacttcaataattgaacacgtactgatttccaatgggtaaggaaaagactcacgtttcgaggccgcgattaaattccaacatggatgctgatttatatgggtataaatgggctcgcgataatgtcgggcaatcaggtgcgacaatctatcgattgtatgggaagcccgatgcgccagagttgtttctgaaacatggcaaaggtagcgttgccaatgatgttacagatgagatggtcagactaaactggctgacggaatttatgcctcttccgaccatcaagcattttatccgtactcctgatgatgcatggttactcaccactgcgatccccggcaaaacagcattccaggtattagaagaatatcctgattcaggtgaaaatattgttgatgcgctggcagtgttcctgcgccggttgcattcgattcctgtttgtaattgtccttttaacagcgatcgcgtatttcgtctcgctcaggcgcaatcacgaatgaataacggtttggttgatgcgagtgattttgatgacgagcgtaatggctggcctgttgaacaagtctggaaagaaatgcataagcttttgccattctcaccggattcagtcgtcactcatggtgatttctcacttgataaccttatttttgacgaggggaaattaataggttgtattgatgttggacgagtcggaatcgcagaccgataccaggatcttgccatcctatggaactgcctcggtgagttttctccttcattacagaaacggctttttcaaaaatatggtattgataatcctgatatgaataaattgcagtttcatttgatgctcgatgagtttttctaatcagtactgacaataaaaagattcttgttttcaagaacttgtcatttgtatagtttttttatattgtagttgttctattttaatcaaatgttagcgtgatttatattttttttcgcctcgacatcatctgcccagatgcgaagttaagtgcgcagaaagtaatatcatgcgtcaatcgtatgtgaatgctggtcgctatactgttcatcttagagaatgtcagtgaggttatttctgagctaatcattaccttgcccggtacaggaatagggtgttaccttattaattacgacggtggtcaaaacgacgaaatttaccccatttttgagttacaagacctgaatttggaaatgatgaaacaattgtaccaagtcttggaggaccatgtaagtgggcttaatcctctcgagaagcaattcccaattgaacacagtaaaccgttatcagccactctgttctttcacttaaggtctcttttttacatggcgaagactcataagcgtactggaagacattacaacttgaaaaagattttcttgttcactaataacgataaaccttacaatggaaactctcagctgagagttcccttgaagaaaaccctggctgattacaatgacgtagacattactttgattccgtttcttctgaacaagccttcaggtgtcaagtttgacaagacggaatactcagaaattttgttctatgataaagatgcttgttcgatgtcaattgaggagatccgccaacgaatttctagacataaggagatcaagcgggtttacttcacctgtcctttgaaaatcgcaaataacttgtgcatttctgtgaaaggttattctatgttttatcatgaaactccaaggaagatcaaatttgtcgtcaatgagggttcaactttcaaagatgtggagacaaaatctcagtttgtcgatccaacatccggaaaagagttttccagtgaacagctgatcaaagcatatcctctaggtgccgatgcttacattcctttaaactcagagcaagtcaaaacaataaatcgatttaatgatatcatcaatatcccctctttggaaattctaggtttcagggatatatctaattggttgccacagtatcagtttggcaaagcatcgtttttatcccctaataa

SEQ ID NO: 158 - protein, 269 aa, synthetic
MGKEKTHVSRPRLNSNMDADLYGYKWARDNVGQSGATIYRLYGKPDAPELFLKHGKGSVANDVTDEMVRLNWLTEFMPLPTIKHFIRTPDDAWLLTTAIPGKTAFQVLEEYPDSGENIVDALAVFLRRLHSIPVCNCPFNSDRVFRLAQAQSRMNNGLVDASDFDDERNGWPVEQVWKEMHKLLPFSPDSVVTHGDFSLDNLIFDEGKLIGCIDVGRVGIADRYQDLAILWNCLGEFSPSLQKRLFQKYGIDNPDMNKLQFHLMLDEFF

SEQ ID NO: 159 - DNA, 3533 bp, synthetic
  misc_feature (1)..(3533): KU70(up)-pFPR2-kanMX-terminator-KU70 construct
  misc_feature (1)..(1002): KU70 upstream region
  promoter (1003)..(1570): promoter pFPR2
  CDS (1571)..(2380): kanMX
  terminator (2381)..(2583): terminator
  misc_feature (2584)..(3533): KU70 downstream region
gctcttcagaagcctaactttaatggggtaaaatatcagcagtaggctgaatatagagcatggcaacgtttacgtcaacagagtttaatagtgaaaactacgataggttcaggcctgtatacccagacgagttgtatcagcaattagtggattatcatgttggtgctaaaggattgtgtgtcgatgttggatgtggctctggccaggcaacgttcaccctgaaaaagtactttgacaaggtcataggatctgatatctcagaaaatcagttggcagtggctaggaaaagacagcctgctggaattgaatttaggttaggaacgggcgaggatttttcttggctaacggagacgccagatgtaatcaccgccgctgaatgcctgcactgggtagacccacagaaattcgttgcaaatgtcgccaattctctaagggatcatggcaccttgagttactggctttatacagaaccaatttttcagaacgaaagggccaatcaggtttacaacaaattcacctacgggtctgactacctgggcccatattgggatcctggccgtacacatttcagaaatcatttaaaggagttgaatcacatcttactggatagcgagctttttgacgaagtgaaaatttctaattttaaacaagaggaaggggtcaaaaacggagatatcttatacttggaaaaagagatgacaatcagtgatttcatcaattttgtatctagttggccttctgtgttttcgtggaagcagcaacgaggaaaggagggtatcctagatgatttttacaacgaactgaacgactgctttgaggggggtaacatgaaagtaatatggaactccgtcctagtatttgccaggaggaagcaaagggttgtataggctttagtacttatagaggaaacggggttacgtgcaagcgcgcatgcctgagctttgaggggggggactttcacatctcttcttctcacacttagccctaacacagagatcaactacaagcggcaattcctacagaaagtgtttgcaaagttcctaatctcggtttgtcaccaagtcacttttctacgaaccctgagtttcctcacgaggaatcaagttttgaaatgcccgatttgtcgcagtttgatagttttgatgaattttttaatggaatctttccagaatttaaaagagtcaagaatatttaacttgtgagcgaacgaacatgaaaaccgaaagaatagttgatgatgatgttgaagcaatgcaagtaccatataaattaggagaagtcctttgtgtattggcgattccttttgatgcaagtgagcgtaaatggttaacaggctgatacatttactcaagctagtagtgaaagccattgcgaaatcagtttatcatagtagtggacgtcacaatggaactcatctctgcgaatcgttgtagaataactgtaggtaaatatgcaattctaacttctggtctaaaatgttcagtgacaatgcttatttctgtagtcgcgaagaattgcttctgaggagacggagcgagccatgtattctcgccaacttgacaagaacgccatgggtaaggaaaagactcacgtttcgaggccgcgattaaattccaacatggatgctgatttatatgggtataaatgggctcgcgataatgtcgggcaatcaggtgcgacaatctatcgattgtatgggaagcccgatgcgccagagttgtttctgaaacatggcaaaggtagcgttgccaatgatgttacagatgagatggtcagactaaactggctgacggaatttatgcctcttccgaccatcaagcattttatccgtactcctgatgatgcatggttactcaccactgcgatccccggcaaaacagcattccaggtattagaagaatatcctgattcaggtgaaaatattgttgatgcgctggcagtgttcctgcgccggttgcattcgattcctgtttgtaattgtccttttaacagcgatcgcgtatttcgtctcgctcaggcgcaatcacgaatgaataacggtttggttgatgcgagtgattttgatgacgagcgtaatggctggcctgttgaacaagtctggaaagaaatgcataagcttttgccattctcaccggattcagtcgtcactcatggtgatttctcacttgataaccttatttttgacgaggggaaattaataggttgtattgatgttggacgagtcggaatcgcagaccgataccaggatcttgccatcctatggaactgcctcggtgagttttctccttcattacagaaacggctttttcaaaaatatggtattgataatcctgatatgaataaattgcagtttcatttgatgctcgatgagtttttctaatcagtactgacaataaaaagattcttgttttcaagaacttgtcatttgtatagtttttttatattgtagttgttctattttaatcaaatgttagcgtgatttatattttttttcgcctcgacatcatctgcccagatgcgaagttaagtgcgcagaaagtaatatcatgcgtcaatcgtatgtgaatgctggtcgctatactgttcatcttagagaatgtcagtgaggttatttctgagctaatcattaccttgcccggtacaggaatagggtgttaccttattaattacgacggtggtcaaaacgacgaaatttaccccatttttgagttacaagacctgaatttggaaatgatgaaacaattgtaccaagtcttggaggaccatgtaagtgggcttaatcctctcgagaagcaattcccaattgaacacagtaaaccgttatcagccactctgttctttcacttaaggtctcttttttacatggcgaagactcataagcgtactggaagacattacaacttgaaaaagattttcttgttcactaataacgataaaccttacaatggaaactctcagctgagagttcccttgaagaaaaccctggctgattacaatgacgtagacattactttgattccgtttcttctgaacaagccttcaggtgtcaagtttgacaagacggaatactcagaaattttgttctatgataaagatgcttgttcgatgtcaattgaggagatccgccaacgaatttctagacataaggagatcaagcgggtttacttcacctgtcctttgaaaatcgcaaataacttgtgcatttctgtgaaaggttattctatgttttatcatgaaactccaaggaagatcaaatttgtcgtcaatgagggttcaactttcaaagatgtggagacaaaatctcagtttgtcgatccaacatccggaaaagagttttccagtgaacagctgatcaaagcatatcctctaggtgccgatgcttacattcctttaaactcagagcaagtcaaaacaataaatcgatttaatgatatcatcaatatcccctctttggaaattctaggtttcagggatatatctaattggttgccacagtatcagtttggcaaagcatcgtttttatcccctaataa

SEQ ID NO: 160 - protein, 269 aa, synthetic; identical to SEQ ID NO: 158

SEQ ID NO: 161 - DNA, 3632 bp, synthetic
  misc_feature (1)..(3632): construct KU70(up)-pRPL3-kanMX-terminator-KU70(dw)
  misc_feature (1)..(1002): KU70 upstream region
  promoter (1003)..(1669): pRPL3 promoter
  CDS (1670)..(2479): kanMX
  terminator (2480)..(2682): terminator
  misc_feature (2480)..(2682): KU70 downstream region
gctcttcagaagcctaactttaatggggtaaaatatcagcagtaggctgaatatagagcatggcaacgtttacgtcaacagagtttaatagtgaaaactacgataggttcaggcctgtatacccagacgagttgtatcagcaattagtggattatcatgttggtgctaaaggattgtgtgtcgatgttggatgtggctctggccaggcaacgttcaccctgaaaaagtactttgacaaggtcataggatctgatatctcagaaaatcagttggcagtggctaggaaaagacagcctgctggaattgaatttaggttaggaacgggcgaggatttttcttggctaacggagacgccagatgtaatcaccgccgctgaatgcctgcactgggtagacccacagaaattcgttgcaaatgtcgccaattctctaagggatcatggcaccttgagttactggctttatacagaaccaatttttcagaacgaaagggccaatcaggtttacaacaaattcacctacgggtctgactacctgggcccatattgggatcctggccgtacacatttcagaaatcatttaaaggagttgaatcacatcttactggatagcgagctttttgacgaagtgaaaatttctaattttaaacaagaggaaggggtcaaaaacggagatatcttatacttggaaaaagagatgacaatcagtgatttcatcaattttgtatctagttggccttctgtgttttcgtggaagcagcaacgaggaaaggagggtatcctagatgatttttacaacgaactgaacgactgctttgaggggggtaacatgaaagtaatatggaactccgtcctagtatttgccaggaggaagcaaagggttgtataggctttagtacttatagaggaaacggggttacgtgcaagcgcgcatgcctgagctttgaggggggggactttcacatctcttcttctcacacttagccctaacacagagatcaactccaacgacttgaggaaatgacgattatttcttaagatattcatggtgaggttttccaaatgtgatctgaaatgtaatcttggcaagtttggttcataaaacgtcaaaagaccacctgaagataaaaaataaagtggaaggagaagaaaaagaggtttttttccagatgagtctatgactaagatttctcttcaaagaattttttcaaggtttgagagggatgaaagcgaggctgctgcacgattatcgatgtcattcaatagggaggtagaagagaactgagggagaaaaggctacaactgaacctaaaactaactgaatttggaatgaagcctattacacgagaggtgtggcgcctttccaaagtcatcaggttcaagttattgctttctggagcaataaatgatgtcaatcccatacggggtctccacccttatagaattacttatctaccggctaggtgttgcatcgcggaccagcccaatcgggtaattttagttgaaaaggtttttagcgcgagtctagttattacccggatagtctaatgctgaaaatttctcggacatttttgatccgtacgtatatttcagtacggagaatcatcaacaagaatctttcaatgccaccaaaaaaaaagacatttttcaccatcgcgcattcacagtagcatgggtaaggaaaagactcacgtttcgaggccgcgattaaattccaacatggatgctgatttatatgggtataaatgggctcgcgataatgtcgggcaatcaggtgcgacaatctatcgattgtatgggaagcccgatgcgccagagttgtttctgaaacatggcaaaggtagcgttgccaatgatgttacagatgagatggtcagactaaactggctgacggaatttatgcctcttccgaccatcaagcattttatccgtactcctgatgatgcatggttactcaccactgcgatccccggcaaaacagcattccaggtattagaagaatatcctgattcaggtgaaaatattgttgatgcgctggcagtgttcctgcgccggttgcattcgattcctgtttgtaattgtccttttaacagcgatcgcgtatttcgtctcgctcaggcgcaatcacgaatgaataacggtttggttgatgcgagtgattttgatgacgagcgtaatggctggcctgttgaacaagtctggaaagaaatgcataagcttttgccattctcaccggattcagtcgtcactcatggtgatttctcacttgataaccttatttttgacgaggggaaattaataggttgtattgatgttggacgagtcggaatcgcagaccgataccaggatcttgccatcctatggaactgcctcggtgagttttctccttcattacagaaacggctttttcaaaaatatggtattgataatcctgatatgaataaattgcagtttcatttgatgctcgatgagtttttctaatcagtactgacaataaaaagattcttgttttcaagaacttgtcatttgtatagtttttttatattgtagttgttctattttaatcaaatgttagcgtgatttatattttttttcgcctcgacatcatctgcccagatgcgaagttaagtgcgcagaaagtaatatcatgcgtcaatcgtatgtgaatgctggtcgctatactgttcatcttagagaatgtcagtgaggttatttctgagctaatcattaccttgcccggtacaggaatagggtgttaccttattaattacgacggtggtcaaaacgacgaaatttaccccatttttgagttacaagacctgaatttggaaatgatgaaacaattgtaccaagtcttggaggaccatgtaagtgggcttaatcctctcgagaagcaattcccaattgaacacagtaaaccgttatcagccactctgttctttcacttaaggtctcttttttacatggcgaagactcataagcgtactggaagacattacaacttgaaaaagattttcttgttcactaataacgataaaccttacaatggaaactctcagctgagagttcccttgaagaaaaccctggctgattacaatgacgtagacattactttgattccgtttcttctgaacaagccttcaggtgtcaagtttgacaagacggaatactcagaaattttgttctatgataaagatgcttgttcgatgtcaattgaggagatccgccaacgaatttctagacataaggagatcaagcgggtttacttcacctgtcctttgaaaatcgcaaataacttgtgcatttctgtgaaaggttattctatgttttatcatgaaactccaaggaagatcaaatttgtcgtcaatgagggttcaactttcaaagatgtggagacaaaatctcagtttgtcgatccaacatccggaaaagagttttccagtgaacagctgatcaaagcatatcctctaggtgccgatgcttacattcctttaaactcagagcaagtcaaaacaataaatcgatttaatgatatcatcaatatcccctctttggaaattctaggtttcagggatatatctaattggttgccacagtatcagtttggcaaagcatcgtttttatcccctaataa

SEQ ID NO: 162 - protein, 269 aa, synthetic; identical to SEQ ID NO: 158

SEQ ID NO: 163 - DNA, 3573 bp, synthetic
  misc_feature (1)..(3573): construct KU70(up)-pRPL6A-kanMX-terminator-KU70(dw)
  misc_feature (1)..(1002): KU70 upstream region
  promoter (1003)..(1610): promoter pRPL6A
  CDS (1611)..(2420): kanMX
  terminator (2421)..(2623): terminator
  misc_feature (2624)..(3573): KU70 downstream region
gctcttcagaagcctaactttaatggggtaaaatatcagcagtaggctgaatatagagcatggcaacgtttacgtcaacagagtttaatagtgaaaactacgataggttcaggcctgtatacccagacgagttgtatcagcaattagtggattatcatgttggtgctaaaggattgtgtgtcgatgttggatgtggctctggccaggcaacgttcaccctgaaaaagtactttgacaaggtcataggatctgatatctcagaaaatcagttggcagtggctaggaaaagacagcctgctggaattgaatttaggttaggaacgggcgaggatttttcttggctaacggagacgccagatgtaatcaccgccgctgaatgcctgcactgggtagacccacagaaattcgttgcaaatgtcgccaattctctaagggatcatggcaccttgagttactggctttatacagaaccaatttttcagaacgaaagggccaatcaggtttacaacaaattcacctacgggtctgactacctgggcccatattgggatcctggccgtacacatttcagaaatcatttaaaggagttgaatcacatcttactggatagcgagctttttgacgaagtgaaaatttctaattttaaacaagaggaaggggtcaaaaacggagatatcttatacttggaaaaagagatgacaatcagtgatttcatcaattttgtatctagttggccttctgtgttttcgtggaagcagcaacgaggaaaggagggtatcctagatgatttttacaacgaactgaacgactgctttgaggggggtaacatgaaagtaatatggaactccgtcctagtatttgccaggaggaagcaaagggttgtataggctttagtacttatagaggaaacggggttacgtgcaagcgcgcatgcctgagctttgaggggggggactttcacatctcttcttctcacacttagccctaacacagagatcaactcgcttcagcatttcgacagtgtaaagaagctcatctcacttgaccagaatgcttttgctatctgttatttcaaagacctagagtacctcccaattgccatagaagcttggaaactttatgaaccttcttctaaagtaccggtggtattcgctcaagtgacacaactccccaaatcagctccaatcgaatggagcgggtcagtgtatcaagagacaccaaactacgatgattactacggtgattcgtcagaaaatgaagatgagtccacacagattgccaacaacttgtcctcgctagaattacagggacaatcggtcacatttcaagacggctacgttagcttgacattcgccccaggcctatcagccacagcacacaacacggtaattttaaacaaggggcaggcaagcaagctggaaaccattccacaggaatattccgtcgacatcatccccgtcaacagactgttcgatttcacagggaaagatcaggacctagccgtactccacaggctgaacatctgagatcaggcatgagaatccttacaccatctatgttgctctagggctgtcaaccctattatgcacgtgacggtgcgactctttcaaatgggtaaggaaaagactcacgtttcgaggccgcgattaaattccaacatggatgctgatttatatgggtataaatgggctcgcgataatgtcgggcaatcaggtgcgacaatctatcgattgtatgggaagcccgatgcgccagagttgtttctgaaacatggcaaaggtagcgttgccaatgatgttacagatgagatggtcagactaaactggctgacggaatttatgcctcttccgaccatcaagcattttatccgtactcctgatgatgcatggttactcaccactgcgatccccggcaaaacagcattccaggtattagaagaatatcctgattcaggtgaaaatattgttgatgcgctggcagtgttcctgcgccggttgcattcgattcctgtttgtaattgtccttttaacagcgatcgcgtatttcgtctcgctcaggcgcaatcacgaatgaataacggtttggttgatgcgagtgattttgatgacgagcgtaatggctggcctgttgaacaagtctggaaagaaatgcataagcttttgccattctcaccggattcagtcgtcactcatggtgatttctcacttgataaccttatttttgacgaggggaaattaataggttgtattgatgttggacgagtcggaatcgcagaccgataccaggatcttgccatcctatggaactgcctcggtgagttttctccttcattacagaaacggctttttcaaaaatatggtattgataatcctgatatgaataaattgcagtttcatttgatgctcgatgagtttttctaatcagtactgacaataaaaagattcttgttttcaagaacttgtcatttgtatagtttttttatattgtagttgttctattttaatcaaatgttagcgtgatttatattttttttcgcctcgacatcatctgcccagatgcgaagttaagtgcgcagaaagtaatatcatgcgtcaatcgtatgtgaatgctggtcgctatactgttcatcttagagaatgtcagtgaggttatttctgagctaatcattaccttgcccggtacaggaatagggtgttaccttattaattacgacggtggtcaaaacgacgaaatttaccccatttttgagttacaagacctgaatttggaaatgatgaaacaattgtaccaagtcttggaggaccatgtaagtgggcttaatcctctcgagaagcaattcccaattgaacacagtaaaccgttatcagccactctgttctttcacttaaggtctcttttttacatggcgaagactcataagcgtactggaagacattacaacttgaaaaagattttcttgttcactaataacgataaaccttacaatggaaactctcagctgagagttcccttgaagaaaaccctggctgattacaatgacgtagacattactttgattccgtttcttctgaacaagccttcaggtgtcaagtttgacaagacggaatactcagaaattttgttctatgataaagatgcttgttcgatgtcaattgaggagatccgccaacgaatttctagacataaggagatcaagcgggtttacttcacctgtcctttgaaaatcgcaaataacttgtgcatttctgtgaaaggttattctatgttttatcatgaaactccaaggaagatcaaatttgtcgtcaatgagggttcaactttcaaagatgtggagacaaaatctcagtttgtcgatccaacatccggaaaagagttttccagtgaacagctgatcaaagcatatcctctaggtgccgatgcttacattcctttaaactcagagcaagtcaaaacaataaatcgatttaatgatatcatcaatatcccctctttggaaattctaggtttcagggatatatctaattggttgccacagtatcagtttggcaaagcatcgtttttatcccctaataa

SEQ ID NO: 164 - protein, 269 aa, synthetic; identical to SEQ ID NO: 158

SEQ ID NO: 165 - DNA, 786 bp, Bacillus
  CDS (1)..(786): Essential gene sufC in the iscU operon
atggctgcttcaacattaacgatcaaagatcttcacgttgaaatcgaagggaaagagatcttaaagggtgtaaaccttgaaataaaaggtggagaattccacgcagtaatgggcccgaacggaactggtaaatccactttatcagctgctattatggggcatcctaaatatgaagtaacaaaaggcagcatcacgcttgacggcaaagatgtactggagatggaagtggacgagcgtgcgcaggcaggcttattccttgcaatgcagtacccaagtgaaatcagcggtgtgacaaatgccgacttccttcgctcagcaatcaacgcgcgcagagaagaaggcgatgaaatttctctcatgaaattcatccgcaaaatggacgaaaacatggagttccttgaaatggaccctgaaatggctcagcgctatcttaacgaaggcttctcaggcggggagaaaaaacgcaacgaaatccttcaattaatgatgattgaaccgaaaatcgccatccttgatgaaattgactcaggccttgatattgacgctttgaaagttgtatcaaaagggatcaacaaaatgcgcagcgaaaacttcggctgcctgatgatcactcactatcagcgcctgttaaactacatcactccggatgttgttcacgttatgatgcaaggccgcgttgtaaaatccggcggtgcagagcttgcacagcgtcttgaagcagaaggttatgactggatcaaacaagaacttggcattgaagacgaaactgttggccaagaagcgtaa

SEQ ID NO: 166 - protein, 261 aa, Bacillus
MAASTLTIKDLHVEIEGKEILKGVNLEIKGGEFHAVMGPNGTGKSTLSAAIMGHPKYEVTKGSITLDGKDVLEMEVDERAQAGLFLAMQYPSEISGVTNADFLRSAINARREEGDEISLMKFIRKMDENMEFLEMDPEMAQRYLNEGFSGGEKKRNEILQLMMIEPKIAILDEIDSGLDIDALKVVSKGINKMRSENFGCLMITHYQRLLNYITPDVVHVMMQGRVVKSGGAELAQRLEAEGYDWIKQELGIEDETVGQEA

SEQ ID NO: 167 - DNA, 1314 bp, Bacillus
  CDS (1)..(1314): Essential gene sufD in the iscU operon
atgacactaggtacaaaactatccgtagatcaggagtatctcaaaagcttttccgaaaagcaccaagaacctgcctggctgaagaacctgcgcttacaggctcttgaacaagctgaggatctgccgatgccgaaacctgacaaaacaaaaatcacaaactggaacttcacgaatttcgcgaagcatacagtggataacgaaccgctttcttcattagaagatttgactgatgaagtaaaagcgctgatcgacattgaaaacgaagataaaacattatacgtacagcgtgaccagacgccggcacatctttctctttctcaagaattgaaagacaaaggcgtcatcttcactgatattctgactgctgcacgcgagcacagcgacttggtggagaaatactttatgaaggacggcgtgaaggttgacgaacataagttaactgcacttcacgcggctcttgttaacggaggagcattcctttatgttccgaaaaatgttcaggtggagacgccggttcaggctgtttatgtccacgaaagcaatgatacagctctattcaaccacgtgctgattgtggctgaagaccacagctctgtaacatatgtagaaaactacatcagcactgtaaacccgaaagacgctgtcttcaatattatcagtgaggtcatcacaggtgataatgccagcgtgacatacggtgcggtggataatctgtcaagcggtgtgacaacttatgtgaaccgccgcggtgctgcgcgcggacgcgacagcaaaatcgagtgggctctcggcctgatgaacgatggcgacacgatttccgaaaacacaacaaacctttacggtgacggcacatacggcgatacgaaaacggttgttgtcggaagaggagagcaaacagaaaacttcacaacacaaatcatccatttcggtaaagcttctgaaggctatatcttgaagcacggtgtgatgaaggattccgcttcttctatctttaacggaatcggcaaaatcgaacatggcgcttctaaagcgaatgcggagcaagaatcacgcgtgctgatgcttagcgaaaaagcacgcggagacgcaaaccctattcttttaattgacgaagacgatgtaactgcaggacatgcggcatctgtcggccgtgtggaccctattcagctttactacctgatgagccgcggaattccgaaagaagaagcagaacgcttagtcatttacggattccttgcaccggtagtaaatgaacttccgattgaaggcgttaagaaacaattagtttctgttatcgaaaggaaagtgaagtaa

SEQ ID NO: 168 - protein, 437 aa, Bacillus
MTLGTKLSVDQEYLKSFSEKHQEPAWLKNLRLQALEQAEDLPMPKPDKTKITNWNFTNFAKHTVDNEPLSSLEDLTDEVKALIDIENEDKTLYVQRDQTPAHLSLSQELKDKGVIFTDILTAAREHSDLVEKYFMKDGVKVDEHKLTALHAALVNGGAFLYVPKNVQVETPVQAVYVHESNDTALFNHVLIVAEDHSSVTYVENYISTVNPKDAVFNIISEVITGDNASVTYGAVDNLSSGVTTYVNRRGAARGRDSKIEWALGLMNDGDTISENTTNLYGDGTYGDTKTVVVGRGEQTENFTTQIIHFGKASEGYILKHGVMKDSASSIFNGIGKIEHGASKANAEQESRVLMLSEKARGDANPILLIDEDDVTAGHAASVGRVDPIQLYYLMSRGIPKEEAERLVIYGFLAPVVNELPIEGVKKQLVSVIERKVK

SEQ ID NO: 169 - DNA, 1221 bp, Bacilllus
  CDS (1)..(1221): Essential gene sufS in the iscU operon
atgaatatcacagatattcgtgaacagttcccgatccttcatcagcaagtgaacggacatgatctcgtttatctcgacagcgcggcgacttcccagaagccgcgtgctgtcattgaaacactggataagtattataaccaatacaattccaatgttcaccggggcgtccatacacttggaaccagagcgacagatggttatgaaggagcgcgtgaaaaagtccgcaagtttattaacgcgaagtcaatggctgagattattttcacaaaaggcacgaccacatcactgaatatggtggcgttaagctatgcgcgcgccaacctgaaacctggtgatgaagtggtcatcacctacatggagcatcatgcgaatatcattccgtggcagcaggctgtaaaagcaactggcgccacattaaaatatattccgttgcaggaagacggaacgatttctttagaagacgtcagagaaacggtcacaagcaacacaaaaattgttgcggtgtctcatgtatctaatgttctcggcacggtcaacccgattaaagaaatggcgaaaatcgctcatgacaatggggctgtcattgtggtggacggtgcacaaagcacgcctcacatgaaaattgacgtgcaggatctcgattgcgacttctttgcgctttcttcccataaaatgtgcggacctaccggtgttggtgtgctgtacggaaagaaagccctgctggaaaacatggagcctgccgaattcggcggtgaaatgatcgactttgtcgggctttatgaatcaacttggaaagagcttccgtggaaattcgaagcgggtacgccgattattgcaggagcaatcggcctcggtgccgccattgattttctcgaagaaatcggtcttgatgagatttcccgccatgagcacaagcttgcagcttatgcgcttgaacgcttccgccagcttgacggcgtaacggtttacgggccggaagagcgtgccgggcttgtcacatttaaccttgatgatgttcatccgcacgatgtggcgactgtgcttgatgcggagggaatcgcagtcagagccggccaccattgtgcgcagccgctgatgaaatggctggatgtaactgctactgcaagagcaagcttttatctgtataatacagaggaagagattgataagcttgtggaagctcttcaaaagacaaaggagtattttacaaatgtcttttaa

SEQ ID NO: 170 - protein, 406 aa, Bacilllus
MNITDIREQFPILHQQVNGHDLVYLDSAATSQKPRAVIETLDKYYNQYNSNVHRGVHTLGTRATDGYEGAREKVRKFINAKSMAEIIFTKGTTTSLNMVALSYARANLKPGDEVVITYMEHHANIIPWQQAVKATGATLKYIPLQEDGTISLEDVRETVTSNTKIVAVSHVSNVLGTVNPIKEMAKIAHDNGAVIVVDGAQSTPHMKIDVQDLDCDFFALSSHKMCGPTGVGVLYGKKALLENMEPAEFGGEMIDFVGLYESTWKELPWKFEAGTPIIAGAIGLGAAIDFLEEIGLDEISRHEHKLAAYALERFRQLDGVTVYGPEERAGLVTFNLDDVHPHDVATVLDAEGIAVRAGHHCAQPLMKWLDVTATARASFYLYNTEEEIDKLVEALQKTKEYFTNVF

SEQ ID NO: 171 - DNA, 444 bp, Bacillus
  CDS (1)..(444): Essential gene sufU (synonym iscU) in the iscU operon
atgtcttttaatgcaaacttagatacattgtacagacaggtgattatggatcattacaaaaacccgcgaaataaaggggttttaaatgacagcattgtcgtggatatgaacaatccgacatgcggcgaccgcatcagactgacaatgaagcttgacggagacatcgtggaagatgcgaagtttgaaggggaaggctgttccatttcaatggcatccgcttcgatgatgactcaggcgattaaagggaaagatattgaaactgccctttccatgtctaagattttctcggatatgatgcaagggaaagagtatgatgattctatagatctcggggatattgaagcccttcaaggcgtttcaaaattccctgcccgtatcaaatgtgcaaccctgtcatggaaagcacttgaaaaaggagtcgcgaaagaagaaggcggcaattaa

SEQ ID NO: 172 - protein, 147 aa, Bacillus
MSFNANLDTLYRQVIMDHYKNPRNKGVLNDSIVVDMNNPTCGDRIRLTMKLDGDIVEDAKFEGEGCSISMASASMMTQAIKGKDIETALSMSKIFSDMMQGKEYDDSIDLGDIEALQGVSKFPARIKCATLSWKALEKGVAKEEGGN

SEQ ID NO: 173 - DNA, 1398 bp, Bacillus
  CDS (1)..(1398): Essential gene sufB in the iscU operon
atggctaaaaaaatgcctgatattggtgaatacaagtatggttttcacgacaaggacgtttccattttccgttcagagcgcggattgacaaaagaaatcgtagaagaaatttctcgcatgaaagaagagcctcaatggatgcttgacttccgcttgaaatcacttgagcatttctacaatatgccgatgcctcaatggggcggagatttaaactcactgaactttgacgaaattacgtactacgtaaaaccgtctgagcgttcagagcgttcttgggatgaagttcctgaagaaattaaacaaacattcgacaagctcggtattcctgaagctgaacaaaaataccttgcgggtgtttctgctcagtacgaatctgaggttgtataccacaacatgaaagaagatcttgaagcacaaggcatcgtctttaaagacactgacagcgcgctgaaagagaatgaagatattttccgtgagcactgggcaaaagtaatcccgccgactgataacaagtttgcggcgcttaactcagctgtttggtccggcggttctttcatctacgtgcctaaaggcgtgaaggttgaaacaccgctacaagcttacttccgtatcaactctgagaacatgggtcagttcgaacgtacactgatcattgttgacgaagaagcaagcgttcattatgttgaaggctgtactgcgcctgtttacacaacaaactcacttcacagtgcggtcgttgagatcatcgtgaaaaaaggcggctactgccgttatacaacgatccaaaactgggcgaacaacgtttacaaccttgtaacaaagcgtacagtctgtgaagaaaacgcaacaatggaatggatcgacggcaacatcggttctaagctgacaatgaaatatccggcttgtatcctaaaaggcgaaggcgcgcgcggtatgacgctttctatcgctcttgcgggtaaaggccagcatcaggatgcaggtgcgaaaatgattcaccttgcaccaaacacatcatctacaatcgtatcaaaatcgatttcaaaacagggcggaaaagtaacgtaccgcggaatcgtccacttcggacgcaaagcggaaggcgcccgctctaacatcgagtgtgatacgctcattatggataacaaatcaacttctgacacaattccttacaatgaaatcttaaatgataacatttcattggagcacgaagcgaaagtgtctaaagtatctgaagagcagctcttctacttgatgagccgcggtatttctgaagaagaagcaactgaaatgatcgtaatgggctttatcgagccattcacaaaagagcttccgatggaatacgcagttgaaatgaaccgtttgattaagttcgaaatggaaggttctatcggttaa

SEQ ID NO: 174 - protein, 465 aa, Bacillus
MAKKMPDIGEYKYGFHDKDVSIFRSERGLTKEIVEEISRMKEEPQWMLDFRLKSLEHFYNMPMPQWGGDLNSLNFDEITYYVKPSERSERSWDEVPEEIKQTFDKLGIPEAEQKYLAGVSAQYESEVVYHNMKEDLEAQGIVFKDTDSALKENEDIFREHWAKVIPPTDNKFAALNSAVWSGGSFIYVPKGVKVETPLQAYFRINSENMGQFERTLIIVDEEASVHYVEGCTAPVYTTNSLHSAVVEIIVKKGGYCRYTTIQNWANNVYNLVTKRTVCEENATMEWIDGNIGSKLTMKYPACILKGEGARGMTLSIALAGKGQHQDAGAKMIHLAPNTSSTIVSKSISKQGGKVTYRGIVHFGRKAEGARSNIECDTLIMDNKSTSDTIPYNEILNDNISLEHEAKVSKVSEEQLFYLMSRGISEEEATEMIVMGFIEPFTKELPMEYAVEMNRLIKFEMEGSIG

SEQ ID NO: 175 - DNA, 480 bp, Bacillus
  CDS (1)..(480): Essential gene accB (in accC operon)
atgttaaatatcaaagaaatccacgagctgattaaagcaattgacgagtctacaattgacgaattcgtatatgaaaatgaaggtgtatccttaaaactgaaaaaacacgaagcaggcacggttcaagtcatgcagcaggcaccggcagcacctgtacaagcacaggctccgcaggcagttcagccgcaagcgcagcaagcagcggcacctgcccaagaagcaccaaagcaagatgagaatctgcataaaatcacttcaccaatggtaggaacattttatgcttcttcatcaccggaagctggcccgtatgtaacagccggttcaaaagtaaatgaaaacacagttgtctgcattgtagaagcgatgaagcttttcaacgaaatcgaagcagaagtgaaaggcgaaatcgttgaagtattagtagaaaacggccagctggtcgaatacggacaacctctatttcttgtaaaagcggagtaa

SEQ ID NO: 176 - protein, 159 aa, Bacillus
MLNIKEIHELIKAIDESTIDEFVYENEGVSLKLKKHEAGTVQVMQQAPAAPVQAQAPQAVQPQAQQAAAPAQEAPKQDENLHKITSPMVGTFYASSSPEAGPYVTAGSKVNENTVVCIVEAMKLFNEIEAEVKGEIVEVLVENGQLVEYGQPLFLVKAE

SEQ ID NO: 177 - DNA, 1353 bp, Bacillus
  CDS (1)..(1353): Essential gene accC (in accC operon)
atgattaaaaagctattgatcgccaacagaggagaaattgctgtcagaatcatcagagcctgcagagagctcggaattgagactgtcgctgtttattcagaagctgataaagatgcccttcatgttcaaatggccgatgaagctttttgtatcggaccgaaagcatcaaaagacagctatttaaacgttacaaatattgtgagtgttgcaaagctgactggcacggacgccattcatccgggatacggatttttagctgaaaatgctgatttcgctgaattatgtgaagaagtgaatgtcacgtttgtcggcccgagcgctgacgccatttcaaaaatgggaacaaaagacgttgcgcgggaaacgatgaaacaggccggcgtgccaatcgtaccgggttcacagggaattatagaaaatgtggaagaagcggtttcgcttgctaatgaaattgggtatcctgtaattataaaagccaccgcaggcggaggcggaaaaggaattagggttgcccgcactgaagaggaactgattaatggcattaagattacacagcaggaagcggcaactgcatttgggaatccaggtgtatacatcgaaaaatacatagaagattttcgccacgttgagatccaagtgcttgctgataactacggaaatacgatccatttgggcgaacgcgactgctcgatccaaagacgcctgcaaaagcttttggaagaatcaccatctcctgcccttgattcagaaatcagggagcaaatgggagatgcagcggtaaaggctgccaaagcggttggctatacaggtgctggaacagttgaatttatctatgactacaatgaacagcgctattacttcatggaaatgaacacgagaatccaggtggagcacccagtcacagaaatggtgacgggaactgacctgatcaaggaacaaatcaaagtggcttcaggaatggaactgagcctcaagcaagaagatgttgaatttgaaggctgggccatcgaatgccgaatcaacgcagaaaacccaagcaaaaatttcatgccgtcacctggtgaaattaaaatgtacctgcctcctggcggtcttggtgtccgtgtcgattcagctgcgtaccctggctattccatcccaccgtactatgacagcatgattgcaaaggtaatcacatacggaaaaacgagagatgaagcgattgcccgcatgaagcgcgcattgagcgaattcgtcatcgaaggcattgagacaacaatccctttccatttaaaactgcttgaacacgaaacatttgtgagcggagagtttaatacgaaatttttagaaacatatgatgtaatgggctcataa

SEQ ID NO: 178 - protein, 450 aa, Bacillus
MIKKLLIANRGEIAVRIIRACRELGIETVAVYSEADKDALHVQMADEAFCIGPKASKDSYLNVTNIVSVAKLTGTDAIHPGYGFLAENADFAELCEEVNVTFVGPSADAISKMGTKDVARETMKQAGVPIVPGSQGIIENVEEAVSLANEIGYPVIIKATAGGGGKGIRVARTEEELINGIKITQQEAATAFGNPGVYIEKYIEDFRHVEIQVLADNYGNTIHLGERDCSIQRRLQKLLEESPSPALDSEIREQMGDAAVKAAKAVGYTGAGTVEFIYDYNEQRYYFMEMNTRIQVEHPVTEMVTGTDLIKEQIKVASGMELSLKQEDVEFEGWAIECRINAENPSKNFMPSPGEIKMYLPPGGLGVRVDSAAYPGYSIPPYYDSMIAKVITYGKTRDEAIARMKRALSEFVIEGIETTIPFHLKLLEHETFVSGEFNTKFLETYDVMGS

SEQ ID NO: 179 - DNA, 408 bp, Bacillus
  CDS (1)..(408): Essential gene yghY (in accC operon)
atgaaagacaacagcttgcttaaaatggatcacgaagatacgcatttgggtaaggttgagattgcaccggaggtcattgaggtcattgccggcattgcagcatcagaagttgatggagttgccgaaatgcgcggaaactttgcgacaggcgtcgttgagcgctttggcaaagtgaatcatggcaaaggtgtcaaagtcgacctggcggatgacggaattacgatcgatgtatactgtgtcgttacatttggcgtttcgattccgaaagttgcagcatccgttcaggaaaacattcgtcaaaccttattaaatatgacgtctctttcgattaacgagatcaatattcacatcgtcggcattcaatttgacacaaaagcccaagaagtccaaatcgacgaagaaatgtaa

SEQ ID NO: 180 - protein, 135 aa, Bacillus
MKDNSLLKMDHEDTHLGKVEIAPEVIEVIAGIAASEVDGVAEMRGNFATGVVERFGKVNHGKGVKVDLADDGITIDVYCVVTFGVSIPKVAASVQENIRQTLLNMTSLSINEINIHIVGIQFDTKAQEVQIDEEM

SEQ ID NO: 181 - DNA, 1344 bp, Corynebacterium
  CDS (1)..(1344): Corynebacterium essential gene glmM
atgactcgactttttggaactgatggcgtccgcggactagccaatgaagtactcaccgcacctttggccctgaaactgggtgccgctgcagctcacgtacttaccgcagagaaacgcgtagatggacgccgcccggttgcgatcgttggtagggatcctcgagtctctggagagatgctcgcggcagcactttcagcaggcatggccagccagggtgttgatgtcattcgtgttggtgtcatcccaaccccagctgttgcattcctcaccgatgattatggcgctgatatgggcgtgatgatttctgcatcccacaacccaatgccggacaacggaatcaagttcttctccgcaggtggacacaagcttccagaccatgtggaagacgagattgagcgtgtcatggacagcttgcctgccgaaggcccaaccgggcatggagttggccgtgtcattgaagaagcaaccgatgcacaagaccgctacctggagcacctgaaggaagctgttcctacgtcacttgaaggcatcaagattgttgtggatgcagccaatggtgcagcaagcgttgtagctccaaaggcttatgaagcagcaggtgcaactgtaattgctattcataacaagccagactcctacaacatcaacatggattgcggttccacccacattgaccaggtgcaggcggcagttctgaagcacggtgctgaccttggactcgcacacgacggcgatgctgaccgttgtttggctgtggacaaagatggaaacctcattgacggtgatcagatcatggcaatgttagccattgcgatgaaagaaaacggcgagctgcgcaagaacaccctcgtgggcaccgtcatgagcaacttgggactgaagattgccatggatgaagccggaattacgctgcgaaccaccaaggtgggcgaccgctacgtgctggaagacctcaatgcgggtggattcagccttggtggcgagcagtctggacacattgttcttccagatcacggcaccactggcgatggaactttgactggtctttccatcatggcgcgcatggctgaaaccggaaaatccttgggcgagttggcacaagcgatgacggttctgccacaggttctgatcaatgtgccagtctctgataaatccaccatcgtttctcacccaagtgtcgttgcagcaatcgctgaagctgaagcggagttgggttctaccggtcgcgtgcttcttcgcgcttctggcaccgaggagcttttccgtgtgatggtcgaagctggcgataaggaacaagcacgccgcattgcgggacgtctttctgccgtggtcgcggaagtctaa

SEQ ID NO: 182 - protein, 447 aa, Corynebacterium
MTRLFGTDGVRGLANEVLTAPLALKLGAAAAHVLTAEKRVDGRRPVAIVGRDPRVSGEMLAAALSAGMASQGVDVIRVGVIPTPAVAFLTDDYGADMGVMISASHNPMPDNGIKFFSAGGHKLPDHVEDEIERVMDSLPAEGPTGHGVGRVIEEATDAQDRYLEHLKEAVPTSLEGIKIVVDAANGAASVVAPKAYEAAGATVIAIHNKPDSYNINMDCGSTHIDQVQAAVLKHGADLGLAHDGDADRCLAVDKDGNLIDGDQIMAMLAIAMKENGELRKNTLVGTVMSNLGLKIAMDEAGITLRTTKVGDRYVLEDLNAGGFSLGGEQSGHIVLPDHGTTGDGTLTGLSIMARMAETGKSLGELAQAMTVLPQVLINVPVSDKSTIVSHPSVVAAIAEAEAELGSTGRVLLRASGTEELFRVMVEAGDKEQARRIAGRLSAVVAEV

SEQ ID NO: 183 - DNA, 1086 bp, Corynebacterium
  CDS (1)..(1086): Corynebacterium essential gene alr
atgaacttgctgaccaccaaaattgacctggatgccatcgcccataacacgagggtgcttaaacaaatggcgggtccggcgaagctgatggcggtggtgaaggcgaatgcatataaccatggcgtggagaaggtcgctccggttattgctgcgcatggtgcggatgcgtttggtgtggcaactcttgcggaggctatgcagttgcgtgatatcggcatcagccaagaggttttgtgttggatttggacaccggagcaggatttccgcgccgccattgatcgcaatattgatttggctgttatttctcccgcgcatgccaaagccttgatcgacactgatgcggagcatattcgggtgtccatcaagattgattctgggttgcatcgttcgggtgtggatgagcaggagtgggagggcgtgttcagcgcgttggctgctgccccgcacattgaggtcacgggcatgttcacgcacttggcgtgcgcggatgagccagagaatccggaaactgatcgccaaattattgcttttcgacgcgcccttgcgctcgcccgcaagcacgggcttgagtgcccggtcaaccacgtatgcaactcacctgcatttttgactcgatctgatttacacatggagatggtccgaccgggtttggccttttatgggttggaacccgtggcgggacgagagcatggtttgaagccggcgatgacgtgggaggcgaaggtgagcgtcgtaaagcaaattgaagctggacaaggcacctcttatggcctgacctggcgcgctgaggatcgcggctttgtggctgtggtgcctgcgggctatgccgatggcatgccgcggcatgcccaggggaaattctccgtcacgattgatggcgtggactatccgcaggttggacgcgtgtgcatggatcagttcgttatttctttgggcgacaatccgcacggtgtggaagctggcgcgaaggccgtgatattcggtgagaatgggcatgacgcaactgattttgcggagcgtttagacaccattaactatgaggtagtgtgccgaccaaccggccgaactgtccgcgcatatgtttaa

SEQ ID NO: 184 - protein, 361 aa, Corynebacterium
MNLLTTKIDLDAIAHNTRVLKQMAGPAKLMAVVKANAYNHGVEKVAPVIAAHGADAFGVATLAEAMQLRDIGISQEVLCWIWTPEQDFRAAIDRNIDLAVISPAHAKALIDTDAEHIRVSIKIDSGLHRSGVDEQEWEGVFSALAAAPHIEVTGMFTHLACADEPENPETDRQIIAFRRALALARKHGLECPVNHVCNSPAFLTRSDLHMEMVRPGLAFYGLEPVAGREHGLKPAMTWEAKVSVVKQIEAGQGTSYGLTWRAEDRGFVAVVPAGYADGMPRHAQGKFSVTIDGVDYPQVGRVCMDQFVISLGDNPHGVEAGAKAVIFGENGHDATDFAERLDTINYEVVCRPTGRTVRAYV

SEQ ID NO: 185 - DNA, 1119 bp, Aspergillus oryzae
  CDS (1)..(1119): Aspergillus essential gene ARG3
atgacttgcggtctgaagctggccgccgctcgttacggcaaccataccttgcgccagaagattccactcaacgctgtgcgccgatacacttctcacactgctacttctacgactccccccacctcgccattcgctcctcgccattttctttccatcgctgatcttacctcaacggagttcgcaaccctcgtccgtaatgcatcttcacacaaacgaaccatcaagtcgggatcaatccctcagaacctgcttggttctatgaccggacagactgtagctatgctgttcagcaaacgcagtaccagaaccaggatatctactgaaggggctgtggtgcgcttgggaggacatccaatgtttctgggcaaggatgatattcaactcggtgtcaatgagtccttgtatgactctgcggttgtaatctcctccatggtctcttgtattgtagcccgagtcggcaagcacgctgaggttgcagaccttgccaagcattcaaccgtgcctgttatcaacgctctctgtgactccttccaccctctccaggccattgccgattttcagaccatctacgaaacatttacacctaaggcccatcgctctgacagtttgggtctggagggcctcaagattgcctgggtcggtgatgcaaacaacgttctgttcgacatggcaattgctgctaccaagatgggtattgatatcgccgttgcgactccgaagggctatgagattcctgccccgatgttggagctcatcaagcaggccagcaacggtgtctcaaagccaggaaagattattgagaccaacgttcctgaggaggcggttaagggtgcggatatcctggtaactgacacctgggtttccatgggacaggaggcagagtcgatcaagcgggtgaaggacttcgagggcttccagatcacttcggaacttgccaagcgcggtggtgcgaacgaaggctggaagttcatgcactgcctgcctcgtcaccctgaggaagtcagcgatgaagttttctacagcccacggtccttggtcttccccgaagcggagaatcggttgtgggctgcgatctcggccatggagggctttgttgtcaataagggaaggattgagtaa

SEQ ID NO: 186 - protein, 372 aa, Aspergillus oryzae
MTCGLKLAAARYGNHTLRQKIPLNAVRRYTSHTATSTTPPTSPFAPRHFLSIADLTSTEFATLVRNASSHKRTIKSGSIPQNLLGSMTGQTVAMLFSKRSTRTRISTEGAVVRLGGHPMFLGKDDIQLGVNESLYDSAVVISSMVSCIVARVGKHAEVADLAKHSTVPVINALCDSFHPLQAIADFQTIYETFTPKAHRSDSLGLEGLKIAWVGDANNVLFDMAIAATKMGIDIAVATPKGYEIPAPMLELIKQASNGVSKPGKIIETNVPEEAVKGADILVTDTWVSMGQEAESIKRVKDFEGFQITSELAKRGGANEGWKFMHCLPRHPEEVSDEVFYSPRSLVFPEAENRLWAAISAMEGFVVNKGRIE

SEQ ID NO: 187 - DNA, 2184 bp, Aspergillus oryzae
  CDS (1)..(2184): Aspergillus essential gene adeA
atgggtgctagactcacatatataaatagtatcattctcctatccgattgtaccatcgcacataatcttgtctcattccacgatttgaatgcggggttcagaaccaacattcatttacgtctccccaaacaaacatccgacttccacaccatgtcttcctctttgagcacgggttccttccaaaccctcacttttcaccctgacaacacggtgattatacaggataaaatctacggggagcacaccatctcagagccggttctagccgagctgcttcggtgtccagctctacttcgactcgcgggcatcggtcttcacggtcaaaccgatcttctgggtataacccatacagtgactcgactagagcactccataggcgcgtcgctattagtgcgcaaagtcggcggtagcatcggagagcaagtcgcaggtcttctgcacgacatcagccacacggtactcagccatgacgtcgatggggccttgtcgaagccaggggagagctatcatgaggtccaaaagtcacggtatatcatgaccactgagttgccacgaatactcaccaaacatggctttgttgatctaaagccgtttgatgaagagctttatcctctggtggagagacccgctcctcatctctgcgctgatcgtctcgattactctctacgagatgctgtcgcgttcggtaaacttgcgatagaggatgcgcgccgcgtgtatgactcattgacagcattcccggacgcgtcttcaccacatcgcttgctggttcttcgagacattgatctagccttagcttatgctagggcctatggtgaatgcgatagggatgtgtggtgcaatccggctcatgccgtcatgtccaggaagataggtcagttgattggggatctagtgcaacaaggatcgttgaaggaagaggtcctatggaatctatcggaccgcgaattttgggagctcctgaaaagtaaagttgactctaaaggattggagacgattaaacacatcgaagcagggccgcatgcggaagattatcatcgtctacctcgtggtaccaagattcgcacaatcgatcctgatctgctcctcccgggtgctgggcaaccctccccactgtcttttgtgaaacctgaatgggctaaggagagacaagacttcattcaggctcgccaggccttactagcatcttttactgtctacatcaacggcggcgtgagctgggaacaagatagtattcagccacaattcgagaacaataatcccatcatgtctgaagctctgacaaacaccgaccttcagggtgctctccctctcatcgctcgaggcaaggttcgcgacctgtacgatgtcgacgagaagaccctcctcttcgtcgcaacggaccgcatctccgcgtacgatgtgatcatggagaatggaatccccgagaaaggcatcctcctaactctatgcacgaaaacctggttcaagatcctctccgacaaaatcccctctctccgcacccacttcctcaccctcgacctcccgcctcagatccccgagtcgttgcgtcccgtcctccagaacagaagcatgcaggtgcgcaagctgaagatcctccccattgaggccatcgtccgcggttacatcaccggttccgcctggaacgagtacaagaaatccggcaccgtgcacgggatcaaggtcgccgagggtctgagggagagcgaggccttccctgatggtcctatttacactcccagtaccaaggcggagcagggcgagcatgatgagaacattcatccggatcaggctgtcgctattgttggtgaacgttatgcctctaagatcgcctctcttgcggttcagctttacaaggtcgctcacgagtatgcccttactcgtggtgtgatcattgccgacaccaagttcgagttcggtttggatcctgagactgacgaggttgtgctggccgacgaggtcctcacccccgattcatcgcgtttctggcctaaggactcgtacgagatcggtcgtggacagcagagcttcgataagcagttcttgcgtgactggttgacgagcgagggactgaagggcaagcctggtgtgcggatgaccgatgagattgcgcagaagaccagcgctaagtaccgggaggcatatgagcggatcactggtgagactaaggttcctgcggtctag

SEQ ID NO: 188 - protein, 727 aa, Aspergillus oryzae
MGARLTYINSIILLSDCTIAHNLVSFHDLNAGFRTNIHLRLPKQTSDFHTMSSSLSTGSFQTLTFHPDNTVIIQDKIYGEHTISEPVLAELLRCPALLRLAGIGLHGQTDLLGITHTVTRLEHSIGASLLVRKVGGSIGEQVAGLLHDISHTVLSHDVDGALSKPGESYHEVQKSRYIMTTELPRILTKHGFVDLKPFDEELYPLVERPAPHLCADRLDYSLRDAVAFGKLAIEDARRVYDSLTAFPDASSPHRLLVLRDIDLALAYARAYGECDRDVWCNPAHAVMSRKIGQLIGDLVQQGSLKEEVLWNLSDREFWELLKSKVDSKGLETIKHIEAGPHAEDYHRLPRGTKIRTIDPDLLLPGAGQPSPLSFVKPEWAKERQDFIQARQALLASFTVYINGGVSWEQDSIQPQFENNNPIMSEALTNTDLQGALPLIARGKVRDLYDVDEKTLLFVATDRISAYDVIMENGIPEKGILLTLCTKTWFKILSDKIPSLRTHFLTLDLPPQIPESLRPVLQNRSMQVRKLKILPIEAIVRGYITGSAWNEYKKSGTVHGIKVAEGLRESEAFPDGPIYTPSTKAEQGEHDENIHPDQAVAIVGERYASKIASLAVQLYKVAHEYALTRGVIIADTKFEFGLDPETDEVVLADEVLTPDSSRFWPKDSYEIGRGQQSFDKQFLRDWLTSEGLKGKPGVRMTDEIAQKTSAKYREAYERITGETKVPAV

SEQ ID NO: 189 - DNA, 750 bp, Aspergillus oryzae
  promoter (1)..(750): Aspergillus oryzae burden sensing promoter p(bibA)
ctatgtagaatagatagtagtaggggtgtcatcctccattatctgacaagcagataccagcatgtggccacgtgtagtgatgttgtgcaagtcattaagctgcagaggtcatgacttcacagtgactagagttgagtaacttgagatatggaaagtacacggtgtactcaaggtacagtacaattggaggttgacgacgtcctttgtccacgtatcctaaaggagcatatggccggggggctgaaaaatagggcaacttcaagaaagattacctaacaggggcttctagccaatgaaacacatttctagtatgttcggtggaccgcttgcagaagatccatgaacactttggggcaatttctacggcagaatacagggcggtggccaaggcggatgggtcattctggtccctgaaaggcgatgcaccaatcacaacgcgaggagtaacctgcagagcgatggccgtaccagccatgctgtccttttctctggcctcaagcattttaaaaaagctgatctcttcctctcacgtccttcgttcagcaacttctctcttttgcctcaactttcccttccttcccccttccattccgtcgcctgtggttgggttctctttttcttccttttgcttctctttcttgaatacaggaaactgtattgaagcacaagggatttactaccaacacgtctcccgataatcacacgcgtgccccttggcgaagaccaccactcgatatacacataggcaca

SEQ ID NO: 190 - DNA, 750 bp, Aspergillus oryzae
  promoter (1)..(750): Aspergillus oryzae burden sensing promoter p(clxA)
agtgtggtctgaagttttgcaaagtgagtgaggaggggaaaagaacgtcggcggggagaggggcaacgtgaagaactccattttttttttttctggatatggataattaactagtagcgggaagtagatcgcgcaatcggtatttgcaaggatagtatgcaattacttcgaagattaagaaaggaacaagaggaaaaatagaaaagaatttatttatattcatttgaaatttacattgactggattgaattgtcttatttgaattgggtgactagcatgtttgggagaagtgtactaatatgaatgaatggtatggagtactacaaataacatacagggacgctaagaccgtgacaaccaaagagagaaaacaaaaaaagcaataaaacggttctttagaatcaatggacactggacagaacattggagaatctgccactaatcctgtttgggtcggtggaactttaccccaaggggcaagcggcagcggaagaggccagattgaacttaagctaccttcccagcttcatataatcaacctccccaacactcgtcttctctttctcctctcctctctcttcttccttctgtcgtgcggttagcttgtggtacgctctcaccttgacactcttttccccctcgaacctctacggaggaccaattgcttgatcgtttgcttatttgtttctttctttcctaaagctactaccgagtcgggcttcttagtttgagagcccgttatcattcatc

SEQ ID NO: 191 - DNA, 300 bp, Corynebacterium glutamicum
  promoter (1)..(300): C. glutamicum burden sensing promoter p(groES)
gcgaagacatcacgttggatgaaattgagcgaattaaggacggcattcgcgccgctcgtaactaccgcgatgattatccagaggaattcaacctgtggcgcaacgctgtatataacctgcgtacgccctaaagtttggctgccatgtgaatttttagcaccctcaacagttgagtgctggcactctcgggggtagagtgccaaataggttgtttgacacacagttgttcacccgcgacgacggctgtgctggaaacccacaaccggcacacacaaaatttttctcatggagggattcacc

SEQ ID NO: 192 - DNA, 300 bp, Corynebacterium glutamicum
  promoter (1)..(300): C. glutamicum burden sensing promoter p(katA)
tttcccggatgaaatccgtgagagctgcgcgatcgccacggccggcggctagggccagctcggtgacgtgggcgtcgttacgctcttttgacttcacaattgctcagaataccagttcagaccggggtcaccataaaggtgtgtagggggtgtcaaagtgggcaaaaagtatcatacttttgtctttttgctggcagtttacgtaagggctgattatttggtggcgcgaagcgacattctgatgtagactatcaatcagacttaatccataggtaaccctcataaaaggaaggaatgcta

SEQ ID NO: 193 - DNA, 300 bp, Corynebacterium glutamicum
  promoter (1)..(300): C. glutamicum burden sensing promoter p(cplX)
ggaggtggcggtggtgcgacacacaacgcgcacgcccgatggttggcgttccatcgcgctaaactggggatcacagtagcgttctactatttctttgctgagtcgatgcgggcgaaggcccctgtttgtggtttcaatttcggttgcgccgtgaataaattcgggattcattagcttaagcgtaccgctctgcagagttcacaggtaaagcgctaagatggaacaacccattgccaatattgttggttagagttgtacgcagtaaatcttttcaatcgtggaagcgggtctcacagtcta

SEQ ID NO: 194 - DNA, 300 bp, Corynebacterium glutamicum
  promoter (1)..(300): C. glutamicum burden sensing promoter p(mutM)
tggataccaagttggcagagtttgaaacctcgctgtccaccacgttgcgttctgtcactgctgatcgttccgcactacgccgaggagctggagctactggccgcgagctgcgcgatgagcaaccggcagcgcgtggtgaatatgagcgggactacgagcgtgattatgaacgaggctacgaacgcgacgatcgagactactagtttccaagaaaccatttaggctttttcacctttccgtctagcgatcctcatctgatgtatgtagtcacgatgaggtacgagtaggatcttcctggtc

SEQ ID NO: 195 - DNA, 4694 bp, synthetic
  plasmid (1)..(4694): pEG151
  misc_feature (88)..(651): homology region; iscU upstream
  promoter (1833)..(2128): burden addiction promoter p(groES)
  RBS (2129)..(2134)
  misc_feature (2134)..(2134): N is A, T, C or G
  misc_feature (2144)..(2621): homology region; iscU downstream
aacaaaattctccagtcttcacatcggtttgaaaggaggaagcggaagaatgaagtaagagggatttttgactccgaagtaagtcttcattgaggaattcggaaacaccacgcattaagagaaggaatattccgaaaaaccattctcatttgttctgaaaggatgctttcgtctcatctgccgctatttcacgccaaatcgtttttgcggcatccaacgcagcactggtacaataaaaagcaaatatatgaagggattgattcattatttgcagcagccaggacagactgaacctcgattatacgtcagaaatggaaaaagcgatgcagctgtcacacggaattggatacgaggaatatggacgccggctggaaacaagaatgaaagtagagcggcagagagagcttgattatgaaaaaagcaagcggatttctgcgggagcttattgagaaaatcaatcttttaaaaaagggtgggaatccactctttttctttttcaatcgctttaataaagtgctgatctttgttaaacttgaggaatgtgcaaggcacgataaaaagttgtatttacttttcatttgttataaaattagaatgagaataaaatgagaataatgattatatatttttggaggtatagatatggctgctagttcggattagatccccctatgcaagggtttattgttttctaaaatctgattaccaattagaatgaatatttcccaaatattaaataataaaacaaaaaaattgaaaaaagtgtttccaccattttttcaatttttttataatttttttaatctgttatttaaatagtttatagttaaatttacattttcattagtccattcaatattctctccaagataactacgaactgctaacaaaattctctccctatgttctaatggagaagattcagccactgcatttcccgcaatatcttttggtatgattttacccgtgtccatagttaaaatcatacggcataaagttaatatagagttggtttcatcatcctgataattatctattaattcctctgacgaatccataatggctcttctcacatcagaaaatggaatatcaggtagtaattcctctaagtcataatttccgtatattcttttattttttcgttttgcttggtaaagcattatggttaaatctgaatttaattccttctgaggaatgtatccttgttcataaagctcttgtaaccattctccataaataaattcttgtttgggaggatgattccacggtaccatttcttgctgaataataattgttaattcaatatatcgtaagttgcttttatctcctattttttttgaaataggtctaattttttgtataagtatttctttactttgatctgtcaatggttcagatacgacgactaaaaagtcaagatcactatttggttttagtccactctcaactcctgatccaaacatgtaagtaccaataaggttattttttaaatgtttccgaagtatttttttcactttattaatttgttcgtatgtattcaaatatatcctcctcactattttgattagtacctattttatatccatagttgttaattaaataaacttaatttagtttatttatagatttcattggcttctaaattttttatctagataataattattttagttaattttattctagattatatatgatatgatctttcatttccataaaactaaagtaagtgtaaacctattcattgttttaaaaatatctcttgccagtcacgttacgttattagttatagttattataacatgtattcacgaacgaaaatcgcatcgattaatgcggaaaactgcatgatgatatatgtcaaaataataaaccaatactgttttctcaaatggtatgtactcctttgttaagtgggtttcgttcatctacagctattgtaacataatcggtacgggggtgaaaaagctaacggaaaagggagcggaaaagaatgatgtaagcgtgaaaaattttttatcttatcacttgaaattggaagggagattctttattataagaattgtgttagcactctttagtgctgagtgctaaaattacatattcatactattgaggaggttatttcacgagntgaaatcatatggctgcttcaacattaacgatcaaagatcttcacgttgaaatcgaagggaaagagatcttaaagggtgtaaaccttgaaataaaaggtggagaattccacgcagtaatgggcccgaacggaactggtaaatccactttatcagctgctattatggggcatcctaaatatgaagtaacaaaaggcagcatcacgcttgacggcaaagatgtactggagatggaagtggacgagcgtgcgcaggcaggcttattccttgcaatgcagtacccaagtgaaatcagcggtgtgacaaatgccgacttccttcgctcagcaatcaacgcgcgcagagaagaaggcgatgaaatttctctcatgaaattcatccgcaaaatggacgaaaacatggagttccttgaaatggaccctgaaatggctcagcgctatcttaacgaaggcttctcaggcggggagaaaaaacgcaacgaaatccttcaattttattgcaataacaggtgcttacttttctggagttctttagcaaatttttttattagctgaacttagtattagtggccatactcctccaatccaaagctatttagaaagattactatatcctcaaacaggcggtaaccggcctcttcatcgggaatgcgcgcgaccttcagcatcgccggcatgtccccctggcggacgggaagtatccagctcgaggtcgggccgcgttgctggcgtttttccataggctccgcccccctgacgagcatcacaaaaatcgacgctcaagtcagaggtggcgaaacccgacaggactataaagataccaggcgtttccccctggaagctccctcgtgcgctctcctgttccgaccctgccgcttaccggatacctgtccgcctttctcccttcgggaagcgtggcgctttctcatagctcacgctgtaggtatctcagttcggtgtaggtcgttcgctccaagctgggctgtgtgcacgaaccccccgttcagcccgaccgctgcgccttatccggtaactatcgtcttgagtccaacccggtaagacacgacttatcgccactggcagcagccactggtaacaggattagcagagcgaggtatgtaggcggtgctacagagttcttgaagtggtggcctaactacggctacactagaaggacagtatttggtatctgcgctctgctgaagccagttaccttcggaaaaagagttgatagctcttgatccggcaaacaaaccaccgctggtagcggtggtttttttgtttgcaagcagcagattacgcgcagaaaaaaaggatctcaagaagatcctttgatcttttctacggggtctgacgctcagtggaacgaaaactcacgttaagggattttggtcatgagattatcaaaaaggatcttcacctagatccttttaaattaaaaatgaagttttaaatcaatctaaagtatatatgagtaaacttggtctgacagttaccaatgcttaatcagtgaggcacctatctcagcgatctgtctatttcgttcatccatagttgcctgactccccgtcgtgtagataactacgatacgggagggcttaccatctggccccagtgctgcaatgataccgcgagacccacgctcaccggctccagatttatcagcaataaaccagccagccggaagggccgagcgcagaagtggtcctgcaactttatccgcctccatccagtctattaattgttgccgggaagctagagtaagtagttcgccagttaatagtttgcgcaacgttgttgccattgctgcaggcatcgtggtgtcacgctcgtcgtttggtatggcttcattcagctccggttcccaacgatcaaggcgagttacatgatcccccatgttgtgcaaaaaagcggttagctccttcggtcctccgatcgttgtcagaagtaagttggccgcagtgttatcactcatggttatggcagcactgcataattctcttactgtcatgccatccgtaagatgcttttctgtgactggtgagtactcaaccaagtcattctgagaatagtgtatgcggcgaccgagttgctcttgcccggcgtcaacacgggataataccgcgccacatagcagaactttaaaagtgctcatcattggaaaacgttcttcggggcgaaaactctcaaggatcttaccgctgttgagatccagttcgatgtaacccactcgtgcacccaactgatcttcagcatcttttactttcaccagcgtttctgggtgagcaaaaacaggaaggcaaaatgccgcaaaaaagggaataagggcgacacggaaatgttgaatactcatactcttcctttttcaatattattgaagcatttatcagggttattgtctcatgagcggatacatatttgaatgtatttagaaaaataaacaaataggggttccgcgcacatttccccgaaaagtgccacctgacgtctaagaaaccattattatcatgacattaacctataaaaataggcgtatcacgaggccctttcgtcttcaagaatt

SEQ ID NO: 196 - DNA, 4697 bp, synthetic
  plasmid (1)..(4697): Plasmid pEG152
  misc_feature (88)..(651): Homology region iscU upstream
  promoter (1833)..(2131): burden addiction promoter p(ctsR)
  rbs (2132)..(2137): RBS
  misc_feature (2137)..(2137): N is A, T, C or G
  misc_feature (2147)..(2624): Homology region iscU downstream
aacaaaattctccagtcttcacatcggtttgaaaggaggaagcggaagaatgaagtaagagggatttttgactccgaagtaagtcttcattgaggaattcggaaacaccacgcattaagagaaggaatattccgaaaaaccattctcatttgttctgaaaggatgctttcgtctcatctgccgctatttcacgccaaatcgtttttgcggcatccaacgcagcactggtacaataaaaagcaaatatatgaagggattgattcattatttgcagcagccaggacagactgaacctcgattatacgtcagaaatggaaaaagcgatgcagctgtcacacggaattggatacgaggaatatggacgccggctggaaacaagaatgaaagtagagcggcagagagagcttgattatgaaaaaagcaagcggatttctgcgggagcttattgagaaaatcaatcttttaaaaaagggtgggaatccactctttttctttttcaatcgctttaataaagtgctgatctttgttaaacttgaggaatgtgcaaggcacgataaaaagttgtatttacttttcatttgttataaaattagaatgagaataaaatgagaataatgattatatatttttggaggtatagatatggctgctagttcggattagatccccctatgcaagggtttattgttttctaaaatctgattaccaattagaatgaatatttcccaaatattaaataataaaacaaaaaaattgaaaaaagtgtttccaccattttttcaatttttttataatttttttaatctgttatttaaatagtttatagttaaatttacattttcattagtccattcaatattctctccaagataactacgaactgctaacaaaattctctccctatgttctaatggagaagattcagccactgcatttcccgcaatatcttttggtatgattttacccgtgtccatagttaaaatcatacggcataaagttaatatagagttggtttcatcatcctgataattatctattaattcctctgacgaatccataatggctcttctcacatcagaaaatggaatatcaggtagtaattcctctaagtcataatttccgtatattcttttattttttcgttttgcttggtaaagcattatggttaaatctgaatttaattccttctgaggaatgtatccttgttcataaagctcttgtaaccattctccataaataaattcttgtttgggaggatgattccacggtaccatttcttgctgaataataattgttaattcaatatatcgtaagttgcttttatctcctattttttttgaaataggtctaattttttgtataagtatttctttactttgatctgtcaatggttcagatacgacgactaaaaagtcaagatcactatttggttttagtccactctcaactcctgatccaaacatgtaagtaccaataaggttattttttaaatgtttccgaagtatttttttcactttattaatttgttcgtatgtattcaaatatatcctcctcactattttgattagtacctattttatatccatagttgttaattaaataaacttaatttagtttatttatagatttcattggcttctaaattttttatctagataataattattttagttaattttattctagattatatatgatatgatctttcatttccataaaactaaagtaagtgtaaacctattcattgttttaaaaatatctcttgccagtcacgttacgttattagttatagttattataacatgtattcacgaacgaaaatcgcatcgattgctcttcagcgccgatggtagtcgggggtttccccctgtgagagtaggacgccgccaagcaagcttaaacccagctcaatgagctgggttttttgtattttggtttattggtatcataaaattccacttaactgtataatataataactttataccgaattttaaatcagcaatcaggttttgtggaccgggaaaatggaaataatgaaggatagagcgagaaagttgaaaattctcgagaaacggcttatagtaagattaaagtcaaatatagtcaaagtcagtaaaggagggggttgacgagntgaaatcatatggctgcttcaacattaacgatcaaagatcttcacgttgaaatcgaagggaaagagatcttaaagggtgtaaaccttgaaataaaaggtggagaattccacgcagtaatgggcccgaacggaactggtaaatccactttatcagctgctattatggggcatcctaaatatgaagtaacaaaaggcagcatcacgcttgacggcaaagatgtactggagatggaagtggacgagcgtgcgcaggcaggcttattccttgcaatgcagtacccaagtgaaatcagcggtgtgacaaatgccgacttccttcgctcagcaatcaacgcgcgcagagaagaaggcgatgaaatttctctcatgaaattcatccgcaaaatggacgaaaacatggagttccttgaaatggaccctgaaatggctcagcgctatcttaacgaaggcttctcaggcggggagaaaaaacgcaacgaaatccttcaattttattgcaataacaggtgcttacttttctggagttctttagcaaatttttttattagctgaacttagtattagtggccatactcctccaatccaaagctatttagaaagattactatatcctcaaacaggcggtaaccggcctcttcatcgggaatgcgcgcgaccttcagcatcgccggcatgtccccctggcggacgggaagtatccagctcgaggtcgggccgcgttgctggcgtttttccataggctccgcccccctgacgagcatcacaaaaatcgacgctcaagtcagaggtggcgaaacccgacaggactataaagataccaggcgtttccccctggaagctccctcgtgcgctctcctgttccgaccctgccgcttaccggatacctgtccgcctttctcccttcgggaagcgtggcgctttctcatagctcacgctgtaggtatctcagttcggtgtaggtcgttcgctccaagctgggctgtgtgcacgaaccccccgttcagcccgaccgctgcgccttatccggtaactatcgtcttgagtccaacccggtaagacacgacttatcgccactggcagcagccactggtaacaggattagcagagcgaggtatgtaggcggtgctacagagttcttgaagtggtggcctaactacggctacactagaaggacagtatttggtatctgcgctctgctgaagccagttaccttcggaaaaagagttgatagctcttgatccggcaaacaaaccaccgctggtagcggtggtttttttgtttgcaagcagcagattacgcgcagaaaaaaaggatctcaagaagatcctttgatcttttctacggggtctgacgctcagtggaacgaaaactcacgttaagggattttggtcatgagattatcaaaaaggatcttcacctagatccttttaaattaaaaatgaagttttaaatcaatctaaagtatatatgagtaaacttggtctgacagttaccaatgcttaatcagtgaggcacctatctcagcgatctgtctatttcgttcatccatagttgcctgactccccgtcgtgtagataactacgatacgggagggcttaccatctggccccagtgctgcaatgataccgcgagacccacgctcaccggctccagatttatcagcaataaaccagccagccggaagggccgagcgcagaagtggtcctgcaactttatccgcctccatccagtctattaattgttgccgggaagctagagtaagtagttcgccagttaatagtttgcgcaacgttgttgccattgctgcaggcatcgtggtgtcacgctcgtcgtttggtatggcttcattcagctccggttcccaacgatcaaggcgagttacatgatcccccatgttgtgcaaaaaagcggttagctccttcggtcctccgatcgttgtcagaagtaagttggccgcagtgttatcactcatggttatggcagcactgcataattctcttactgtcatgccatccgtaagatgcttttctgtgactggtgagtactcaaccaagtcattctgagaatagtgtatgcggcgaccgagttgctcttgcccggcgtcaacacgggataataccgcgccacatagcagaactttaaaagtgctcatcattggaaaacgttcttcggggcgaaaactctcaaggatcttaccgctgttgagatccagttcgatgtaacccactcgtgcacccaactgatcttcagcatcttttactttcaccagcgtttctgggtgagcaaaaacaggaaggcaaaatgccgcaaaaaagggaataagggcgacacggaaatgttgaatactcatactcttcctttttcaatattattgaagcatttatcagggttattgtctcatgagcggatacatatttgaatgtatttagaaaaataaacaaataggggttccgcgcacatttccccgaaaagtgccacctgacgtctaagaaaccattattatcatgacattaacctataaaaataggcgtatcacgaggccctttcgtcttcaagaatt

SEQ ID NO: 197 - DNA, 4697 bp, synthetic
  plasmid (1)..(4697): Plasmid pEG153
  misc_feature (88)..(651): Homology region iscU upstream
  promoter (1833)..(2131): burden addiction promoter p(dnaK)
  rbs (2132)..(2137): rbs
  misc_feature (2132)..(2137): N is A, T, C or G
  misc_feature (2147)..(2624): Homology region iscU downstream
aacaaaattctccagtcttcacatcggtttgaaaggaggaagcggaagaatgaagtaagagggatttttgactccgaagtaagtcttcattgaggaattcggaaacaccacgcattaagagaaggaatattccgaaaaaccattctcatttgttctgaaaggatgctttcgtctcatctgccgctatttcacgccaaatcgtttttgcggcatccaacgcagcactggtacaataaaaagcaaatatatgaagggattgattcattatttgcagcagccaggacagactgaacctcgattatacgtcagaaatggaaaaagcgatgcagctgtcacacggaattggatacgaggaatatggacgccggctggaaacaagaatgaaagtagagcggcagagagagcttgattatgaaaaaagcaagcggatttctgcgggagcttattgagaaaatcaatcttttaaaaaagggtgggaatccactctttttctttttcaatcgctttaataaagtgctgatctttgttaaacttgaggaatgtgcaaggcacgataaaaagttgtatttacttttcatttgttataaaattagaatgagaataaaatgagaataatgattatatatttttggaggtatagatatggctgctagttcggattagatccccctatgcaagggtttattgttttctaaaatctgattaccaattagaatgaatatttcccaaatattaaataataaaacaaaaaaattgaaaaaagtgtttccaccattttttcaatttttttataatttttttaatctgttatttaaatagtttatagttaaatttacattttcattagtccattcaatattctctccaagataactacgaactgctaacaaaattctctccctatgttctaatggagaagattcagccactgcatttcccgcaatatcttttggtatgattttacccgtgtccatagttaaaatcatacggcataaagttaatatagagttggtttcatcatcctgataattatctattaattcctctgacgaatccataatggctcttctcacatcagaaaatggaatatcaggtagtaattcctctaagtcataatttccgtatattcttttattttttcgttttgcttggtaaagcattatggttaaatctgaatttaattccttctgaggaatgtatccttgttcataaagctcttgtaaccattctccataaataaattcttgtttgggaggatgattccacggtaccatttcttgctgaataataattgttaattcaatatatcgtaagttgcttttatctcctattttttttgaaataggtctaattttttgtataagtatttctttactttgatctgtcaatggttcagatacgacgactaaaaagtcaagatcactatttggttttagtccactctcaactcctgatccaaacatgtaagtaccaataaggttattttttaaatgtttccgaagtatttttttcactttattaatttgttcgtatgtattcaaatatatcctcctcactattttgattagtacctattttatatccatagttgttaattaaataaacttaatttagtttatttatagatttcattggcttctaaattttttatctagataataattattttagttaattttattctagattatatatgatatgatctttcatttccataaaactaaagtaagtgtaaacctattcattgttttaaaaatatctcttgccagtcacgttacgttattagttatagttattataacatgtattcacgaacgaaaatcgcatcgattggttcaatccccgcacacgggaatttcgattaaaatcggaaaagaaaacgactatgaagagatggaaaattgcagtctgattacggcttcttattccgtagaccagaagcagatcggctcaattgcgattatcggcccgacccgcatgaattattccagggttgtcagcctgcttcagcatgtgacttcggacttgtcaaaagcattaacaagtctgtatgatgaataagggaattttggcaaattttatcgaagggcagcacctgtccttctccttacactttgagggaggtgaacacacgagntgaaatcatatggctgcttcaacattaacgatcaaagatcttcacgttgaaatcgaagggaaagagatcttaaagggtgtaaaccttgaaataaaaggtggagaattccacgcagtaatgggcccgaacggaactggtaaatccactttatcagctgctattatggggcatcctaaatatgaagtaacaaaaggcagcatcacgcttgacggcaaagatgtactggagatggaagtggacgagcgtgcgcaggcaggcttattccttgcaatgcagtacccaagtgaaatcagcggtgtgacaaatgccgacttccttcgctcagcaatcaacgcgcgcagagaagaaggcgatgaaatttctctcatgaaattcatccgcaaaatggacgaaaacatggagttccttgaaatggaccctgaaatggctcagcgctatcttaacgaaggcttctcaggcggggagaaaaaacgcaacgaaatccttcaattttattgcaataacaggtgcttacttttctggagttctttagcaaatttttttattagctgaacttagtattagtggccatactcctccaatccaaagctatttagaaagattactatatcctcaaacaggcggtaaccggcctcttcatcgggaatgcgcgcgaccttcagcatcgccggcatgtccccctggcggacgggaagtatccagctcgaggtcgggccgcgttgctggcgtttttccataggctccgcccccctgacgagcatcacaaaaatcgacgctcaagtcagaggtggcgaaacccgacaggactataaagataccaggcgtttccccctggaagctccctcgtgcgctctcctgttccgaccctgccgcttaccggatacctgtccgcctttctcccttcgggaagcgtggcgctttctcatagctcacgctgtaggtatctcagttcggtgtaggtcgttcgctccaagctgggctgtgtgcacgaaccccccgttcagcccgaccgctgcgccttatccggtaactatcgtcttgagtccaacccggtaagacacgacttatcgccactggcagcagccactggtaacaggattagcagagcgaggtatgtaggcggtgctacagagttcttgaagtggtggcctaactacggctacactagaaggacagtatttggtatctgcgctctgctgaagccagttaccttcggaaaaagagttgatagctcttgatccggcaaacaaaccaccgctggtagcggtggtttttttgtttgcaagcagcagattacgcgcagaaaaaaaggatctcaagaagatcctttgatcttttctacggggtctgacgctcagtggaacgaaaactcacgttaagggattttggtcatgagattatcaaaaaggatcttcacctagatccttttaaattaaaaatgaagttttaaatcaatctaaagtatatatgagtaaacttggtctgacagttaccaatgcttaatcagtgaggcacctatctcagcgatctgtctatttcgttcatccatagttgcctgactccccgtcgtgtagataactacgatacgggagggcttaccatctggccccagtgctgcaatgataccgcgagacccacgctcaccggctccagatttatcagcaataaaccagccagccggaagggccgagcgcagaagtggtcctgcaactttatccgcctccatccagtctattaattgttgccgggaagctagagtaagtagttcgccagttaatagtttgcgcaacgttgttgccattgctgcaggcatcgtggtgtcacgctcgtcgtttggtatggcttcattcagctccggttcccaacgatcaaggcgagttacatgatcccccatgttgtgcaaaaaagcggttagctccttcggtcctccgatcgttgtcagaagtaagttggccgcagtgttatcactcatggttatggcagcactgcataattctcttactgtcatgccatccgtaagatgcttttctgtgactggtgagtactcaaccaagtcattctgagaatagtgtatgcggcgaccgagttgctcttgcccggcgtcaacacgggataataccgcgccacatagcagaactttaaaagtgctcatcattggaaaacgttcttcggggcgaaaactctcaaggatcttaccgctgttgagatccagttcgatgtaacccactcgtgcacccaactgatcttcagcatcttttactttcaccagcgtttctgggtgagcaaaaacaggaaggcaaaatgccgcaaaaaagggaataagggcgacacggaaatgttgaatactcatactcttcctttttcaatattattgaagcatttatcagggttattgtctcatgagcggatacatatttgaatgtatttagaaaaataaacaaataggggttccgcgcacatttccccgaaaagtgccacctgacgtctaagaaaccattattatcatgacattaacctataaaaataggcgtatcacgaggccctttcgtcttcaagaatt

SEQ ID NO: 198 - DNA, 4697 bp, synthetic
  plasmid (1)..(4697): plasmid pEG154
  misc_feature (88)..(651): homology region iscU upstream
  promoter (1833)..(2131): burden addiction promoter p(perR)
  rbs (2132)..(2137): rbs
  misc_feature (2137)..(2137): N is A, T, C or G
  misc_feature (2147)..(2624): homology region iscU downstream
aacaaaattctccagtcttcacatcggtttgaaaggaggaagcggaagaatgaagtaagagggatttttgactccgaagtaagtcttcattgaggaattcggaaacaccacgcattaagagaaggaatattccgaaaaaccattctcatttgttctgaaaggatgctttcgtctcatctgccgctatttcacgccaaatcgtttttgcggcatccaacgcagcactggtacaataaaaagcaaatatatgaagggattgattcattatttgcagcagccaggacagactgaacctcgattatacgtcagaaatggaaaaagcgatgcagctgtcacacggaattggatacgaggaatatggacgccggctggaaacaagaatgaaagtagagcggcagagagagcttgattatgaaaaaagcaagcggatttctgcgggagcttattgagaaaatcaatcttttaaaaaagggtgggaatccactctttttctttttcaatcgctttaataaagtgctgatctttgttaaacttgaggaatgtgcaaggcacgataaaaagttgtatttacttttcatttgttataaaattagaatgagaataaaatgagaataatgattatatatttttggaggtatagatatggctgctagttcggattagatccccctatgcaagggtttattgttttctaaaatctgattaccaattagaatgaatatttcccaaatattaaataataaaacaaaaaaattgaaaaaagtgtttccaccattttttcaatttttttataatttttttaatctgttatttaaatagtttatagttaaatttacattttcattagtccattcaatattctctccaagataactacgaactgctaacaaaattctctccctatgttctaatggagaagattcagccactgcatttcccgcaatatcttttggtatgattttacccgtgtccatagttaaaatcatacggcataaagttaatatagagttggtttcatcatcctgataattatctattaattcctctgacgaatccataatggctcttctcacatcagaaaatggaatatcaggtagtaattcctctaagtcataatttccgtatattcttttattttttcgttttgcttggtaaagcattatggttaaatctgaatttaattccttctgaggaatgtatccttgttcataaagctcttgtaaccattctccataaataaattcttgtttgggaggatgattccacggtaccatttcttgctgaataataattgttaattcaatatatcgtaagttgcttttatctcctattttttttgaaataggtctaattttttgtataagtatttctttactttgatctgtcaatggttcagatacgacgactaaaaagtcaagatcactatttggttttagtccactctcaactcctgatccaaacatgtaagtaccaataaggttattttttaaatgtttccgaagtatttttttcactttattaatttgttcgtatgtattcaaatatatcctcctcactattttgattagtacctattttatatccatagttgttaattaaataaacttaatttagtttatttatagatttcattggcttctaaattttttatctagataataattattttagttaattttattctagattatatatgatatgatctttcatttccataaaactaaagtaagtgtaaacctattcattgttttaaaaatatctcttgccagtcacgttacgttattagttatagttattataacatgtattcacgaacgaaaatcgcatcgattggaagcatttgatgtgtggaagctgaagaaaaacttcggaaaagagtatatgggaatcgagcgttccacttttttaattgataaagaaggccggctcattaaagaatggagaaaagtaaaagtaaaggaccatgtagccgaagcgcttcaaaccctcaaagatatgtctgaaaagtaaatctctatgagcctatgcttacttttaccctgatatcaattgacaaattatcgtagaaagagttacactaattataaacattacaatgtaagaattttttttagaagagaggtgcatgacggcgagntgaaatcatatggctgcttcaacattaacgatcaaagatcttcacgttgaaatcgaagggaaagagatcttaaagggtgtaaaccttgaaataaaaggtggagaattccacgcagtaatgggcccgaacggaactggtaaatccactttatcagctgctattatggggcatcctaaatatgaagtaacaaaaggcagcatcacgcttgacggcaaagatgtactggagatggaagtggacgagcgtgcgcaggcaggcttattccttgcaatgcagtacccaagtgaaatcagcggtgtgacaaatgccgacttccttcgctcagcaatcaacgcgcgcagagaagaaggcgatgaaatttctctcatgaaattcatccgcaaaatggacgaaaacatggagttccttgaaatggaccctgaaatggctcagcgctatcttaacgaaggcttctcaggcggggagaaaaaacgcaacgaaatccttcaattttattgcaataacaggtgcttacttttctggagttctttagcaaatttttttattagctgaacttagtattagtggccatactcctccaatccaaagctatttagaaagattactatatcctcaaacaggcggtaaccggcctcttcatcgggaatgcgcgcgaccttcagcatcgccggcatgtccccctggcggacgggaagtatccagctcgaggtcgggccgcgttgctggcgtttttccataggctccgcccccctgacgagcatcacaaaaatcgacgctcaagtcagaggtggcgaaacccgacaggactataaagataccaggcgtttccccctggaagctccctcgtgcgctctcctgttccgaccctgccgcttaccggatacctgtccgcctttctcccttcgggaagcgtggcgctttctcatagctcacgctgtaggtatctcagttcggtgtaggtcgttcgctccaagctgggctgtgtgcacgaaccccccgttcagcccgaccgctgcgccttatccggtaactatcgtcttgagtccaacccggtaagacacgacttatcgccactggcagcagccactggtaacaggattagcagagcgaggtatgtaggcggtgctacagagttcttgaagtggtggcctaactacggctacactagaaggacagtatttggtatctgcgctctgctgaagccagttaccttcggaaaaagagttgatagctcttgatccggcaaacaaaccaccgctggtagcggtggtttttttgtttgcaagcagcagattacgcgcagaaaaaaaggatctcaagaagatcctttgatcttttctacggggtctgacgctcagtggaacgaaaactcacgttaagggattttggtcatgagattatcaaaaaggatcttcacctagatccttttaaattaaaaatgaagttttaaatcaatctaaagtatatatgagtaaacttggtctgacagttaccaatgcttaatcagtgaggcacctatctcagcgatctgtctatttcgttcatccatagttgcctgactccccgtcgtgtagataactacgatacgggagggcttaccatctggccccagtgctgcaatgataccgcgagacccacgctcaccggctccagatttatcagcaataaaccagccagccggaagggccgagcgcagaagtggtcctgcaactttatccgcctccatccagtctattaattgttgccgggaagctagagtaagtagttcgccagttaatagtttgcgcaacgttgttgccattgctgcaggcatcgtggtgtcacgctcgtcgtttggtatggcttcattcagctccggttcccaacgatcaaggcgagttacatgatcccccatgttgtgcaaaaaagcggttagctccttcggtcctccgatcgttgtcagaagtaagttggccgcagtgttatcactcatggttatggcagcactgcataattctcttactgtcatgccatccgtaagatgcttttctgtgactggtgagtactcaaccaagtcattctgagaatagtgtatgcggcgaccgagttgctcttgcccggcgtcaacacgggataataccgcgccacatagcagaactttaaaagtgctcatcattggaaaacgttcttcggggcgaaaactctcaaggatcttaccgctgttgagatccagttcgatgtaacccactcgtgcacccaactgatcttcagcatcttttactttcaccagcgtttctgggtgagcaaaaacaggaaggcaaaatgccgcaaaaaagggaataagggcgacacggaaatgttgaatactcatactcttcctttttcaatattattgaagcatttatcagggttattgtctcatgagcggatacatatttgaatgtatttagaaaaataaacaaataggggttccgcgcacatttccccgaaaagtgccacctgacgtctaagaaaccattattatcatgacattaacctataaaaataggcgtatcacgaggccctttcgtcttcaagaatt

SEQ ID NO: 199 - DNA, 4697 bp, synthetic
  plasmid (1)..(4697): plasmid pEG155
  misc_feature (88)..(651): homology region iscU upstream
  promoter (1823)..(2131): burden addiction promoter p(hrcA)
  promoter (1823)..(2131): burden addiction promoter p(hrcA)
  rbs (2132)..(2137): rbs
  misc_feature (2132)..(2137): N is A, T, C or G
  misc_feature (2147)..(2624): homology region iscU downstream
aacaaaattctccagtcttcacatcggtttgaaaggaggaagcggaagaatgaagtaagagggatttttgactccgaagtaagtcttcattgaggaattcggaaacaccacgcattaagagaaggaatattccgaaaaaccattctcatttgttctgaaaggatgctttcgtctcatctgccgctatttcacgccaaatcgtttttgcggcatccaacgcagcactggtacaataaaaagcaaatatatgaagggattgattcattatttgcagcagccaggacagactgaacctcgattatacgtcagaaatggaaaaagcgatgcagctgtcacacggaattggatacgaggaatatggacgccggctggaaacaagaatgaaagtagagcggcagagagagcttgattatgaaaaaagcaagcggatttctgcgggagcttattgagaaaatcaatcttttaaaaaagggtgggaatccactctttttctttttcaatcgctttaataaagtgctgatctttgttaaacttgaggaatgtgcaaggcacgataaaaagttgtatttacttttcatttgttataaaattagaatgagaataaaatgagaataatgattatatatttttggaggtatagatatggctgctagttcggattagatccccctatgcaagggtttattgttttctaaaatctgattaccaattagaatgaatatttcccaaatattaaataataaaacaaaaaaattgaaaaaagtgtttccaccattttttcaatttttttataatttttttaatctgttatttaaatagtttatagttaaatttacattttcattagtccattcaatattctctccaagataactacgaactgctaacaaaattctctccctatgttctaatggagaagattcagccactgcatttcccgcaatatcttttggtatgattttacccgtgtccatagttaaaatcatacggcataaagttaatatagagttggtttcatcatcctgataattatctattaattcctctgacgaatccataatggctcttctcacatcagaaaatggaatatcaggtagtaattcctctaagtcataatttccgtatattcttttattttttcgttttgcttggtaaagcattatggttaaatctgaatttaattccttctgaggaatgtatccttgttcataaagctcttgtaaccattctccataaataaattcttgtttgggaggatgattccacggtaccatttcttgctgaataataattgttaattcaatatatcgtaagttgcttttatctcctattttttttgaaataggtctaattttttgtataagtatttctttactttgatctgtcaatggttcagatacgacgactaaaaagtcaagatcactatttggttttagtccactctcaactcctgatccaaacatgtaagtaccaataaggttattttttaaatgtttccgaagtatttttttcactttattaatttgttcgtatgtattcaaatatatcctcctcactattttgattagtacctattttatatccatagttgttaattaaataaacttaatttagtttatttatagatttcattggcttctaaattttttatctagataataattattttagttaattttattctagattatatatgatatgatctttcatttccataaaactaaagtaagtgtaaacctattcattgttttaaaaatatctcttgccagtcacgttacgttattagttatagttattataacatgtattcacgaacgaaaatcgcatcgatttgaggaagaaatgtttttaggtttgagaaaaacagccggtgtcagcaaaaaacgattcgcagaaaaatacggccgttccctggatggacttttcccaagcgtgttaaaagacctcgctgaaaaagggctgattcacaattcggagtctgccgtttatttgactcatcaagggaaattattaggcaatgaagtttttggcgcttttttgggtgagttataattgacatttttcttgtggtttgatacttttgttatagaattagcactcgcttattgagagtgctaacagaggtgatgatgcgagntgaaatcatatggctgcttcaacattaacgatcaaagatcttcacgttgaaatcgaagggaaagagatcttaaagggtgtaaaccttgaaataaaaggtggagaattccacgcagtaatgggcccgaacggaactggtaaatccactttatcagctgctattatggggcatcctaaatatgaagtaacaaaaggcagcatcacgcttgacggcaaagatgtactggagatggaagtggacgagcgtgcgcaggcaggcttattccttgcaatgcagtacccaagtgaaatcagcggtgtgacaaatgccgacttccttcgctcagcaatcaacgcgcgcagagaagaaggcgatgaaatttctctcatgaaattcatccgcaaaatggacgaaaacatggagttccttgaaatggaccctgaaatggctcagcgctatcttaacgaaggcttctcaggcggggagaaaaaacgcaacgaaatccttcaattttattgcaataacaggtgcttacttttctggagttctttagcaaatttttttattagctgaacttagtattagtggccatactcctccaatccaaagctatttagaaagattactatatcctcaaacaggcggtaaccggcctcttcatcgggaatgcgcgcgaccttcagcatcgccggcatgtccccctggcggacgggaagtatccagctcgaggtcgggccgcgttgctggcgtttttccataggctccgcccccctgacgagcatcacaaaaatcgacgctcaagtcagaggtggcgaaacccgacaggactataaagataccaggcgtttccccctggaagctccctcgtgcgctctcctgttccgaccctgccgcttaccggatacctgtccgcctttctcccttcgggaagcgtggcgctttctcatagctcacgctgtaggtatctcagttcggtgtaggtcgttcgctccaagctgggctgtgtgcacgaaccccccgttcagcccgaccgctgcgccttatccggtaactatcgtcttgagtccaacccggtaagacacgacttatcgccactggcagcagccactggtaacaggattagcagagcgaggtatgtaggcggtgctacagagttcttgaagtggtggcctaactacggctacactagaaggacagtatttggtatctgcgctctgctgaagccagttaccttcggaaaaagagttgatagctcttgatccggcaaacaaaccaccgctggtagcggtggtttttttgtttgcaagcagcagattacgcgcagaaaaaaaggatctcaagaagatcctttgatcttttctacggggtctgacgctcagtggaacgaaaactcacgttaagggattttggtcatgagattatcaaaaaggatcttcacctagatccttttaaattaaaaatgaagttttaaatcaatctaaagtatatatgagtaaacttggtctgacagttaccaatgcttaatcagtgaggcacctatctcagcgatctgtctatttcgttcatccatagttgcctgactccccgtcgtgtagataactacgatacgggagggcttaccatctggccccagtgctgcaatgataccgcgagacccacgctcaccggctccagatttatcagcaataaaccagccagccggaagggccgagcgcagaagtggtcctgcaactttatccgcctccatccagtctattaattgttgccgggaagctagagtaagtagttcgccagttaatagtttgcgcaacgttgttgccattgctgcaggcatcgtggtgtcacgctcgtcgtttggtatggcttcattcagctccggttcccaacgatcaaggcgagttacatgatcccccatgttgtgcaaaaaagcggttagctccttcggtcctccgatcgttgtcagaagtaagttggccgcagtgttatcactcatggttatggcagcactgcataattctcttactgtcatgccatccgtaagatgcttttctgtgactggtgagtactcaaccaagtcattctgagaatagtgtatgcggcgaccgagttgctcttgcccggcgtcaacacgggataataccgcgccacatagcagaactttaaaagtgctcatcattggaaaacgttcttcggggcgaaaactctcaaggatcttaccgctgttgagatccagttcgatgtaacccactcgtgcacccaactgatcttcagcatcttttactttcaccagcgtttctgggtgagcaaaaacaggaaggcaaaatgccgcaaaaaagggaataagggcgacacggaaatgttgaatactcatactcttcctttttcaatattattgaagcatttatcagggttattgtctcatgagcggatacatatttgaatgtatttagaaaaataaacaaataggggttccgcgcacatttccccgaaaagtgccacctgacgtctaagaaaccattattatcatgacattaacctataaaaataggcgtatcacgaggccctttcgtcttcaagaatt

SEQ ID NO: 200 - DNA, 4697 bp, synthetic
  plasmid (1)..(4697): plasmid pEG156
  misc_feature (88)..(651): homology region iscU upstream
  promoter (1833)..(2131): burden addiction promoter p(spxA)
  rbs (2132)..(2137): rbs
  misc_feature (2137)..(2137): N is A, T, C or G
  misc_feature (2147)..(2624): homology region iscU downstream
aacaaaattctccagtcttcacatcggtttgaaaggaggaagcggaagaatgaagtaagagggatttttgactccgaagtaagtcttcattgaggaattcggaaacaccacgcattaagagaaggaatattccgaaaaaccattctcatttgttctgaaaggatgctttcgtctcatctgccgctatttcacgccaaatcgtttttgcggcatccaacgcagcactggtacaataaaaagcaaatatatgaagggattgattcattatttgcagcagccaggacagactgaacctcgattatacgtcagaaatggaaaaagcgatgcagctgtcacacggaattggatacgaggaatatggacgccggctggaaacaagaatgaaagtagagcggcagagagagcttgattatgaaaaaagcaagcggatttctgcgggagcttattgagaaaatcaatcttttaaaaaagggtgggaatccactctttttctttttcaatcgctttaataaagtgctgatctttgttaaacttgaggaatgtgcaaggcacgataaaaagttgtatttacttttcatttgttataaaattagaatgagaataaaatgagaataatgattatatatttttggaggtatagatatggctgctagttcggattagatccccctatgcaagggtttattgttttctaaaatctgattaccaattagaatgaatatttcccaaatattaaataataaaacaaaaaaattgaaaaaagtgtttccaccattttttcaatttttttataatttttttaatctgttatttaaatagtttatagttaaatttacattttcattagtccattcaatattctctccaagataactacgaactgctaacaaaattctctccctatgttctaatggagaagattcagccactgcatttcccgcaatatcttttggtatgattttacccgtgtccatagttaaaatcatacggcataaagttaatatagagttggtttcatcatcctgataattatctattaattcctctgacgaatccataatggctcttctcacatcagaaaatggaatatcaggtagtaattcctctaagtcataatttccgtatattcttttattttttcgttttgcttggtaaagcattatggttaaatctgaatttaattccttctgaggaatgtatccttgttcataaagctcttgtaaccattctccataaataaattcttgtttgggaggatgattccacggtaccatttcttgctgaataataattgttaattcaatatatcgtaagttgcttttatctcctattttttttgaaataggtctaattttttgtataagtatttctttactttgatctgtcaatggttcagatacgacgactaaaaagtcaagatcactatttggttttagtccactctcaactcctgatccaaacatgtaagtaccaataaggttattttttaaatgtttccgaagtatttttttcactttattaatttgttcgtatgtattcaaatatatcctcctcactattttgattagtacctattttatatccatagttgttaattaaataaacttaatttagtttatttatagatttcattggcttctaaattttttatctagataataattattttagttaattttattctagattatatatgatatgatctttcatttccataaaactaaagtaagtgtaaacctattcattgttttaaaaatatctcttgccagtcacgttacgttattagttatagttattataacatgtattcacgaacgaaaatcgcatcgattgaaaacattcatacttataaagatgagaaatggtacggagaatcgtacgaaaaaacggatgaggtcttggaaatcatcgatgaagaaaaacaaaaaaatattttcgatcagttaagctaattgagaataagaacatatcatgaacattaaaaatttgctggattgacacatttttttcttaggatactgttcacacttacttttttatagtataatacctgtaaagattccttttttagagtaatttcaatttaagaataaaatagatgttcatcctactaattagaggagtgaagatgacgagntgaaatcatatggctgcttcaacattaacgatcaaagatcttcacgttgaaatcgaagggaaagagatcttaaagggtgtaaaccttgaaataaaaggtggagaattccacgcagtaatgggcccgaacggaactggtaaatccactttatcagctgctattatggggcatcctaaatatgaagtaacaaaaggcagcatcacgcttgacggcaaagatgtactggagatggaagtggacgagcgtgcgcaggcaggcttattccttgcaatgcagtacccaagtgaaatcagcggtgtgacaaatgccgacttccttcgctcagcaatcaacgcgcgcagagaagaaggcgatgaaatttctctcatgaaattcatccgcaaaatggacgaaaacatggagttccttgaaatggaccctgaaatggctcagcgctatcttaacgaaggcttctcaggcggggagaaaaaacgcaacgaaatccttcaattttattgcaataacaggtgcttacttttctggagttctttagcaaatttttttattagctgaacttagtattagtggccatactcctccaatccaaagctatttagaaagattactatatcctcaaacaggcggtaaccggcctcttcatcgggaatgcgcgcgaccttcagcatcgccggcatgtccccctggcggacgggaagtatccagctcgaggtcgggccgcgttgctggcgtttttccataggctccgcccccctgacgagcatcacaaaaatcgacgctcaagtcagaggtggcgaaacccgacaggactataaagataccaggcgtttccccctggaagctccctcgtgcgctctcctgttccgaccctgccgcttaccggatacctgtccgcctttctcccttcgggaagcgtggcgctttctcatagctcacgctgtaggtatctcagttcggtgtaggtcgttcgctccaagctgggctgtgtgcacgaaccccccgttcagcccgaccgctgcgccttatccggtaactatcgtcttgagtccaacccggtaagacacgacttatcgccactggcagcagccactggtaacaggattagcagagcgaggtatgtaggcggtgctacagagttcttgaagtggtggcctaactacggctacactagaaggacagtatttggtatctgcgctctgctgaagccagttaccttcggaaaaagagttgatagctcttgatccggcaaacaaaccaccgctggtagcggtggtttttttgtttgcaagcagcagattacgcgcagaaaaaaaggatctcaagaagatcctttgatcttttctacggggtctgacgctcagtggaacgaaaactcacgttaagggattttggtcatgagattatcaaaaaggatcttcacctagatccttttaaattaaaaatgaagttttaaatcaatctaaagtatatatgagtaaacttggtctgacagttaccaatgcttaatcagtgaggcacctatctcagcgatctgtctatttcgttcatccatagttgcctgactccccgtcgtgtagataactacgatacgggagggcttaccatctggccccagtgctgcaatgataccgcgagacccacgctcaccggctccagatttatcagcaataaaccagccagccggaagggccgagcgcagaagtggtcctgcaactttatccgcctccatccagtctattaattgttgccgggaagctagagtaagtagttcgccagttaatagtttgcgcaacgttgttgccattgctgcaggcatcgtggtgtcacgctcgtcgtttggtatggcttcattcagctccggttcccaacgatcaaggcgagttacatgatcccccatgttgtgcaaaaaagcggttagctccttcggtcctccgatcgttgtcagaagtaagttggccgcagtgttatcactcatggttatggcagcactgcataattctcttactgtcatgccatccgtaagatgcttttctgtgactggtgagtactcaaccaagtcattctgagaatagtgtatgcggcgaccgagttgctcttgcccggcgtcaacacgggataataccgcgccacatagcagaactttaaaagtgctcatcattggaaaacgttcttcggggcgaaaactctcaaggatcttaccgctgttgagatccagttcgatgtaacccactcgtgcacccaactgatcttcagcatcttttactttcaccagcgtttctgggtgagcaaaaacaggaaggcaaaatgccgcaaaaaagggaataagggcgacacggaaatgttgaatactcatactcttcctttttcaatattattgaagcatttatcagggttattgtctcatgagcggatacatatttgaatgtatttagaaaaataaacaaataggggttccgcgcacatttccccgaaaagtgccacctgacgtctaagaaaccattattatcatgacattaacctataaaaataggcgtatcacgaggccctttcgtcttcaagaatt

SEQ ID NO: 201 - DNA, 4697 bp, synthetic
  plasmid (1)..(4697): pEG157
  misc_feature (88)..(651): homology region iscU upstream
  promoter (1833)..(2131): burden addiction promoter p(sigB)
  rbs (2132)..(2137): rbs
  misc_feature (2132)..(2137): N is A, T, C or G
  misc_feature (2147)..(2624): homology region iscU downstream
aacaaaattctccagtcttcacatcggtttgaaaggaggaagcggaagaatgaagtaagagggatttttgactccgaagtaagtcttcattgaggaattcggaaacaccacgcattaagagaaggaatattccgaaaaaccattctcatttgttctgaaaggatgctttcgtctcatctgccgctatttcacgccaaatcgtttttgcggcatccaacgcagcactggtacaataaaaagcaaatatatgaagggattgattcattatttgcagcagccaggacagactgaacctcgattatacgtcagaaatggaaaaagcgatgcagctgtcacacggaattggatacgaggaatatggacgccggctggaaacaagaatgaaagtagagcggcagagagagcttgattatgaaaaaagcaagcggatttctgcgggagcttattgagaaaatcaatcttttaaaaaagggtgggaatccactctttttctttttcaatcgctttaataaagtgctgatctttgttaaacttgaggaatgtgcaaggcacgataaaaagttgtatttacttttcatttgttataaaattagaatgagaataaaatgagaataatgattatatatttttggaggtatagatatggctgctagttcggattagatccccctatgcaagggtttattgttttctaaaatctgattaccaattagaatgaatatttcccaaatattaaataataaaacaaaaaaattgaaaaaagtgtttccaccattttttcaatttttttataatttttttaatctgttatttaaatagtttatagttaaatttacattttcattagtccattcaatattctctccaagataactacgaactgctaacaaaattctctccctatgttctaatggagaagattcagccactgcatttcccgcaatatcttttggtatgattttacccgtgtccatagttaaaatcatacggcataaagttaatatagagttggtttcatcatcctgataattatctattaattcctctgacgaatccataatggctcttctcacatcagaaaatggaatatcaggtagtaattcctctaagtcataatttccgtatattcttttattttttcgttttgcttggtaaagcattatggttaaatctgaatttaattccttctgaggaatgtatccttgttcataaagctcttgtaaccattctccataaataaattcttgtttgggaggatgattccacggtaccatttcttgctgaataataattgttaattcaatatatcgtaagttgcttttatctcctattttttttgaaataggtctaattttttgtataagtatttctttactttgatctgtcaatggttcagatacgacgactaaaaagtcaagatcactatttggttttagtccactctcaactcctgatccaaacatgtaagtaccaataaggttattttttaaatgtttccgaagtatttttttcactttattaatttgttcgtatgtattcaaatatatcctcctcactattttgattagtacctattttatatccatagttgttaattaaataaacttaatttagtttatttatagatttcattggcttctaaattttttatctagataataattattttagttaattttattctagattatatatgatatgatctttcatttccataaaactaaagtaagtgtaaacctattcattgttttaaaaatatctcttgccagtcacgttacgttattagttatagttattataacatgtattcacgaacgaaaatcgcatcgattaacaattcgatcagcatctggaaaagggcgatatgattgttttattttctgacggcgtcacagaatgcagaacggaaaacggtttcttggagcgtcctgatctgcagaagctcattgaggaacatatgtgttcctctgcgcaggaaatggtcaaaaacatttatgacagcctcctcaaattgcaggattttcagcttcacgatgattttacgttaattgttttgcggagaaaggtttaacgtctgtcagacgagggtataaagcaactagtgatttgaaggaaaatttgaggtgatacgacgagntgaaatcatatggctgcttcaacattaacgatcaaagatcttcacgttgaaatcgaagggaaagagatcttaaagggtgtaaaccttgaaataaaaggtggagaattccacgcagtaatgggcccgaacggaactggtaaatccactttatcagctgctattatggggcatcctaaatatgaagtaacaaaaggcagcatcacgcttgacggcaaagatgtactggagatggaagtggacgagcgtgcgcaggcaggcttattccttgcaatgcagtacccaagtgaaatcagcggtgtgacaaatgccgacttccttcgctcagcaatcaacgcgcgcagagaagaaggcgatgaaatttctctcatgaaattcatccgcaaaatggacgaaaacatggagttccttgaaatggaccctgaaatggctcagcgctatcttaacgaaggcttctcaggcggggagaaaaaacgcaacgaaatccttcaattttattgcaataacaggtgcttacttttctggagttctttagcaaatttttttattagctgaacttagtattagtggccatactcctccaatccaaagctatttagaaagattactatatcctcaaacaggcggtaaccggcctcttcatcgggaatgcgcgcgaccttcagcatcgccggcatgtccccctggcggacgggaagtatccagctcgaggtcgggccgcgttgctggcgtttttccataggctccgcccccctgacgagcatcacaaaaatcgacgctcaagtcagaggtggcgaaacccgacaggactataaagataccaggcgtttccccctggaagctccctcgtgcgctctcctgttccgaccctgccgcttaccggatacctgtccgcctttctcccttcgggaagcgtggcgctttctcatagctcacgctgtaggtatctcagttcggtgtaggtcgttcgctccaagctgggctgtgtgcacgaaccccccgttcagcccgaccgctgcgccttatccggtaactatcgtcttgagtccaacccggtaagacacgacttatcgccactggcagcagccactggtaacaggattagcagagcgaggtatgtaggcggtgctacagagttcttgaagtggtggcctaactacggctacactagaaggacagtatttggtatctgcgctctgctgaagccagttaccttcggaaaaagagttgatagctcttgatccggcaaacaaaccaccgctggtagcggtggtttttttgtttgcaagcagcagattacgcgcagaaaaaaaggatctcaagaagatcctttgatcttttctacggggtctgacgctcagtggaacgaaaactcacgttaagggattttggtcatgagattatcaaaaaggatcttcacctagatccttttaaattaaaaatgaagttttaaatcaatctaaagtatatatgagtaaacttggtctgacagttaccaatgcttaatcagtgaggcacctatctcagcgatctgtctatttcgttcatccatagttgcctgactccccgtcgtgtagataactacgatacgggagggcttaccatctggccccagtgctgcaatgataccgcgagacccacgctcaccggctccagatttatcagcaataaaccagccagccggaagggccgagcgcagaagtggtcctgcaactttatccgcctccatccagtctattaattgttgccgggaagctagagtaagtagttcgccagttaatagtttgcgcaacgttgttgccattgctgcaggcatcgtggtgtcacgctcgtcgtttggtatggcttcattcagctccggttcccaacgatcaaggcgagttacatgatcccccatgttgtgcaaaaaagcggttagctccttcggtcctccgatcgttgtcagaagtaagttggccgcagtgttatcactcatggttatggcagcactgcataattctcttactgtcatgccatccgtaagatgcttttctgtgactggtgagtactcaaccaagtcattctgagaatagtgtatgcggcgaccgagttgctcttgcccggcgtcaacacgggataataccgcgccacatagcagaactttaaaagtgctcatcattggaaaacgttcttcggggcgaaaactctcaaggatcttaccgctgttgagatccagttcgatgtaacccactcgtgcacccaactgatcttcagcatcttttactttcaccagcgtttctgggtgagcaaaaacaggaaggcaaaatgccgcaaaaaagggaataagggcgacacggaaatgttgaatactcatactcttcctttttcaatattattgaagcatttatcagggttattgtctcatgagcggatacatatttgaatgtatttagaaaaataaacaaataggggttccgcgcacatttccccgaaaagtgccacctgacgtctaagaaaccattattatcatgacattaacctataaaaataggcgtatcacgaggccctttcgtcttcaagaatt

SEQ ID NO: 202 - DNA, 4697 bp, synthetic
  plasmid (1)..(4697): plasmid pEG158
  misc_feature (88)..(651): homology region iscU upstream
  promoter (1833)..(2131): burden adiction promoter p(yflT)
  rbs (2132)..(2137): rbs
  misc_feature (2137)..(2137): N is A, T, C or G
  misc_feature (2147)..(2624): homology region iscU downstream
aacaaaattctccagtcttcacatcggtttgaaaggaggaagcggaagaatgaagtaagagggatttttgactccgaagtaagtcttcattgaggaattcggaaacaccacgcattaagagaaggaatattccgaaaaaccattctcatttgttctgaaaggatgctttcgtctcatctgccgctatttcacgccaaatcgtttttgcggcatccaacgcagcactggtacaataaaaagcaaatatatgaagggattgattcattatttgcagcagccaggacagactgaacctcgattatacgtcagaaatggaaaaagcgatgcagctgtcacacggaattggatacgaggaatatggacgccggctggaaacaagaatgaaagtagagcggcagagagagcttgattatgaaaaaagcaagcggatttctgcgggagcttattgagaaaatcaatcttttaaaaaagggtgggaatccactctttttctttttcaatcgctttaataaagtgctgatctttgttaaacttgaggaatgtgcaaggcacgataaaaagttgtatttacttttcatttgttataaaattagaatgagaataaaatgagaataatgattatatatttttggaggtatagatatggctgctagttcggattagatccccctatgcaagggtttattgttttctaaaatctgattaccaattagaatgaatatttcccaaatattaaataataaaacaaaaaaattgaaaaaagtgtttccaccattttttcaatttttttataatttttttaatctgttatttaaatagtttatagttaaatttacattttcattagtccattcaatattctctccaagataactacgaactgctaacaaaattctctccctatgttctaatggagaagattcagccactgcatttcccgcaatatcttttggtatgattttacccgtgtccatagttaaaatcatacggcataaagttaatatagagttggtttcatcatcctgataattatctattaattcctctgacgaatccataatggctcttctcacatcagaaaatggaatatcaggtagtaattcctctaagtcataatttccgtatattcttttattttttcgttttgcttggtaaagcattatggttaaatctgaatttaattccttctgaggaatgtatccttgttcataaagctcttgtaaccattctccataaataaattcttgtttgggaggatgattccacggtaccatttcttgctgaataataattgttaattcaatatatcgtaagttgcttttatctcctattttttttgaaataggtctaattttttgtataagtatttctttactttgatctgtcaatggttcagatacgacgactaaaaagtcaagatcactatttggttttagtccactctcaactcctgatccaaacatgtaagtaccaataaggttattttttaaatgtttccgaagtatttttttcactttattaatttgttcgtatgtattcaaatatatcctcctcactattttgattagtacctattttatatccatagttgttaattaaataaacttaatttagtttatttatagatttcattggcttctaaattttttatctagataataattattttagttaattttattctagattatatatgatatgatctttcatttccataaaactaaagtaagtgtaaacctattcattgttttaaaaatatctcttgccagtcacgttacgttattagttatagttattataacatgtattcacgaacgaaaatcgcatcgattgactaaatcactcacaatccaagcattgtattgctgttctggtgaaaagtattgcattagacatacctcctgctcgtacggataaaggcagcgtttcatggtcgtgtgctccgtgcagcggcttctccttaattttgatttttctgaaaataggtcccgttcctatcactttaccatggacggaaaacaaatagctactaccattcctcctgtttttctcttcaatgttctggaatctgtttcaggtacagacgatcgggtatgaaagaaatatagaaaacatgaaggaggaatatcgaccgagntgaaatcatatggctgcttcaacattaacgatcaaagatcttcacgttgaaatcgaagggaaagagatcttaaagggtgtaaaccttgaaataaaaggtggagaattccacgcagtaatgggcccgaacggaactggtaaatccactttatcagctgctattatggggcatcctaaatatgaagtaacaaaaggcagcatcacgcttgacggcaaagatgtactggagatggaagtggacgagcgtgcgcaggcaggcttattccttgcaatgcagtacccaagtgaaatcagcggtgtgacaaatgccgacttccttcgctcagcaatcaacgcgcgcagagaagaaggcgatgaaatttctctcatgaaattcatccgcaaaatggacgaaaacatggagttccttgaaatggaccctgaaatggctcagcgctatcttaacgaaggcttctcaggcggggagaaaaaacgcaacgaaatccttcaattttattgcaataacaggtgcttacttttctggagttctttagcaaatttttttattagctgaacttagtattagtggccatactcctccaatccaaagctatttagaaagattactatatcctcaaacaggcggtaaccggcctcttcatcgggaatgcgcgcgaccttcagcatcgccggcatgtccccctggcggacgggaagtatccagctcgaggtcgggccgcgttgctggcgtttttccataggctccgcccccctgacgagcatcacaaaaatcgacgctcaagtcagaggtggcgaaacccgacaggactataaagataccaggcgtttccccctggaagctccctcgtgcgctctcctgttccgaccctgccgcttaccggatacctgtccgcctttctcccttcgggaagcgtggcgctttctcatagctcacgctgtaggtatctcagttcggtgtaggtcgttcgctccaagctgggctgtgtgcacgaaccccccgttcagcccgaccgctgcgccttatccggtaactatcgtcttgagtccaacccggtaagacacgacttatcgccactggcagcagccactggtaacaggattagcagagcgaggtatgtaggcggtgctacagagttcttgaagtggtggcctaactacggctacactagaaggacagtatttggtatctgcgctctgctgaagccagttaccttcggaaaaagagttgatagctcttgatccggcaaacaaaccaccgctggtagcggtggtttttttgtttgcaagcagcagattacgcgcagaaaaaaaggatctcaagaagatcctttgatcttttctacggggtctgacgctcagtggaacgaaaactcacgttaagggattttggtcatgagattatcaaaaaggatcttcacctagatccttttaaattaaaaatgaagttttaaatcaatctaaagtatatatgagtaaacttggtctgacagttaccaatgcttaatcagtgaggcacctatctcagcgatctgtctatttcgttcatccatagttgcctgactccccgtcgtgtagataactacgatacgggagggcttaccatctggccccagtgctgcaatgataccgcgagacccacgctcaccggctccagatttatcagcaataaaccagccagccggaagggccgagcgcagaagtggtcctgcaactttatccgcctccatccagtctattaattgttgccgggaagctagagtaagtagttcgccagttaatagtttgcgcaacgttgttgccattgctgcaggcatcgtggtgtcacgctcgtcgtttggtatggcttcattcagctccggttcccaacgatcaaggcgagttacatgatcccccatgttgtgcaaaaaagcggttagctccttcggtcctccgatcgttgtcagaagtaagttggccgcagtgttatcactcatggttatggcagcactgcataattctcttactgtcatgccatccgtaagatgcttttctgtgactggtgagtactcaaccaagtcattctgagaatagtgtatgcggcgaccgagttgctcttgcccggcgtcaacacgggataataccgcgccacatagcagaactttaaaagtgctcatcattggaaaacgttcttcggggcgaaaactctcaaggatcttaccgctgttgagatccagttcgatgtaacccactcgtgcacccaactgatcttcagcatcttttactttcaccagcgtttctgggtgagcaaaaacaggaaggcaaaatgccgcaaaaaagggaataagggcgacacggaaatgttgaatactcatactcttcctttttcaatattattgaagcatttatcagggttattgtctcatgagcggatacatatttgaatgtatttagaaaaataaacaaataggggttccgcgcacatttccccgaaaagtgccacctgacgtctaagaaaccattattatcatgacattaacctataaaaataggcgtatcacgaggccctttcgtcttcaagaatt

SEQ ID NO: 203 - DNA, 4696 bp, synthetic
  plasmid (1)..(4696): plasmid pEG159
  misc_feature (88)..(676): homology region aaC upstream
  promoter (1858)..(2153): burden adiction promoter p(groES)
  rbs (2154)..(2159): rbs
  misc_feature (2154)..(2159): N is A, T, C or G
  misc_feature (2169)..(2623): homology region aaC downstream
aacaaaattctccagtcttcacatcggtttgaaaggaggaagcggaagaatgaagtaagagggatttttgactccgaagtaagtcttagggaacgaaagattcatcagcagacaaggaaacatccgctgaagccagtgaaaaaggaactgttgttacggaaacagccgatgatgatttgtttacaacgtaccgtcttgatttagaagatgccagaagcaaagaaagagaagagctgaatgccattgtgtcaagcgatgatgcaacagccaaggagaaaagcgaagcatacgataaaatgacggctctcagtgaagtggaaggaacagaaaaacagctggaaacgctgattaaaacacaaggttacgaggatgcgcttgttaatgctgaaggagataaaatcaatattacagtcaaatcagacaaacactctaaatcgaaggcgacagccattatagaccttgtggcaaaagaaatcaaaacaatgaaagatgtcgctgtcacatttgaaccctctaaataagaatgagggaaaaaagcccgctaaacaagcgggctttttgcgttgctgtcatattagagttgaattcaaaagtccgctcctgtaagatgaacatagtatgtacttttagtagtaacctataaaaaaagaaatttcatacataggagtgcgattgaagttcggattagatccccctatgcaagggtttattgttttctaaaatctgattaccaattagaatgaatatttcccaaatattaaataataaaacaaaaaaattgaaaaaagtgtttccaccattttttcaatttttttataatttttttaatctgttatttaaatagtttatagttaaatttacattttcattagtccattcaatattctctccaagataactacgaactgctaacaaaattctctccctatgttctaatggagaagattcagccactgcatttcccgcaatatcttttggtatgattttacccgtgtccatagttaaaatcatacggcataaagttaatatagagttggtttcatcatcctgataattatctattaattcctctgacgaatccataatggctcttctcacatcagaaaatggaatatcaggtagtaattcctctaagtcataatttccgtatattcttttattttttcgttttgcttggtaaagcattatggttaaatctgaatttaattccttctgaggaatgtatccttgttcataaagctcttgtaaccattctccataaataaattcttgtttgggaggatgattccacggtaccatttcttgctgaataataattgttaattcaatatatcgtaagttgcttttatctcctattttttttgaaataggtctaattttttgtataagtatttctttactttgatctgtcaatggttcagatacgacgactaaaaagtcaagatcactatttggttttagtccactctcaactcctgatccaaacatgtaagtaccaataaggttattttttaaatgtttccgaagtatttttttcactttattaatttgttcgtatgtattcaaatatatcctcctcactattttgattagtacctattttatatccatagttgttaattaaataaacttaatttagtttatttatagatttcattggcttctaaattttttatctagataataattattttagttaattttattctagattatatatgatatgatctttcatttccataaaactaaagtaagtgtaaacctattcattgttttaaaaatatctcttgccagtcacgttacgttattagttatagttattataacatgtattcacgaacgaaaatcgcatcgattaatgcggaaaactgcatgatgatatatgtcaaaataataaaccaatactgttttctcaaatggtatgtactcctttgttaagtgggtttcgttcatctacagctattgtaacataatcggtacgggggtgaaaaagctaacggaaaagggagcggaaaagaatgatgtaagcgtgaaaaattttttatcttatcacttgaaattggaagggagattctttattataagaattgtgttagcactctttagtgctgagtgctaaaattacatattcatactattgaggaggttatttcacgagntgaaatcatatgttaaatatcaaagaaatccacgagctgattaaagcaattgacgagtctacaattgacgaattcgtatatgaaaatgaaggtgtatccttaaaactgaaaaaacacgaagcaggcacggttcaagtcatgcagcaggcaccggcagcacctgtacaagcacaggctccgcaggcagttcagccgcaagcgcagcaagcagcggcacctgcccaagaagcaccaaagcaagatgagaatctgcataaaatcacttcaccaatggtaggaacattttatgcttcttcatcaccggaagctggcccgtatgtaacagccggttcaaaagtaaatgaaaacacagttgtctgcattgtagaagcgatgaagcttttcaacgaaatcgaagcagaagtgaaaggcgaaatcgttgaagtattagtagaaaacggccagctggtcgaatacggacaaccaattttattgcaataacaggtgcttacttttctggagttctttagcaaatttttttattagctgaacttagtattagtggccatactcctccaatccaaagctatttagaaagattactatatcctcaaacaggcggtaaccggcctcttcatcgggaatgcgcgcgaccttcagcatcgccggcatgtccccctggcggacgggaagtatccagctcgaggtcgggccgcgttgctggcgtttttccataggctccgcccccctgacgagcatcacaaaaatcgacgctcaagtcagaggtggcgaaacccgacaggactataaagataccaggcgtttccccctggaagctccctcgtgcgctctcctgttccgaccctgccgcttaccggatacctgtccgcctttctcccttcgggaagcgtggcgctttctcatagctcacgctgtaggtatctcagttcggtgtaggtcgttcgctccaagctgggctgtgtgcacgaaccccccgttcagcccgaccgctgcgccttatccggtaactatcgtcttgagtccaacccggtaagacacgacttatcgccactggcagcagccactggtaacaggattagcagagcgaggtatgtaggcggtgctacagagttcttgaagtggtggcctaactacggctacactagaaggacagtatttggtatctgcgctctgctgaagccagttaccttcggaaaaagagttgatagctcttgatccggcaaacaaaccaccgctggtagcggtggtttttttgtttgcaagcagcagattacgcgcagaaaaaaaggatctcaagaagatcctttgatcttttctacggggtctgacgctcagtggaacgaaaactcacgttaagggattttggtcatgagattatcaaaaaggatcttcacctagatccttttaaattaaaaatgaagttttaaatcaatctaaagtatatatgagtaaacttggtctgacagttaccaatgcttaatcagtgaggcacctatctcagcgatctgtctatttcgttcatccatagttgcctgactccccgtcgtgtagataactacgatacgggagggcttaccatctggccccagtgctgcaatgataccgcgagacccacgctcaccggctccagatttatcagcaataaaccagccagccggaagggccgagcgcagaagtggtcctgcaactttatccgcctccatccagtctattaattgttgccgggaagctagagtaagtagttcgccagttaatagtttgcgcaacgttgttgccattgctgcaggcatcgtggtgtcacgctcgtcgtttggtatggcttcattcagctccggttcccaacgatcaaggcgagttacatgatcccccatgttgtgcaaaaaagcggttagctccttcggtcctccgatcgttgtcagaagtaagttggccgcagtgttatcactcatggttatggcagcactgcataattctcttactgtcatgccatccgtaagatgcttttctgtgactggtgagtactcaaccaagtcattctgagaatagtgtatgcggcgaccgagttgctcttgcccggcgtcaacacgggataataccgcgccacatagcagaactttaaaagtgctcatcattggaaaacgttcttcggggcgaaaactctcaaggatcttaccgctgttgagatccagttcgatgtaacccactcgtgcacccaactgatcttcagcatcttttactttcaccagcgtttctgggtgagcaaaaacaggaaggcaaaatgccgcaaaaaagggaataagggcgacacggaaatgttgaatactcatactcttcctttttcaatattattgaagcatttatcagggttattgtctcatgagcggatacatatttgaatgtatttagaaaaataaacaaataggggttccgcgcacatttccccgaaaagtgccacctgacgtctaagaaaccattattatcatgacattaacctataaaaataggcgtatcacgaggccctttcgtcttcaagaatt

SEQ ID NO: 204 - DNA, 4699 bp, synthetic
  plasmid (1)..(4699): plasmid pEG160
  misc_feature (88)..(676): homology region accC upstream
  promoter (1858)..(2156): burden adiction promoter p(ctsR)
  rbs (2157)..(2162): rbs
  misc_feature (2162)..(2162): N is A, T, C or G
  misc_feature (2172)..(2626): homology region accC downstream
aacaaaattctccagtcttcacatcggtttgaaaggaggaagcggaagaatgaagtaagagggatttttgactccgaagtaagtcttagggaacgaaagattcatcagcagacaaggaaacatccgctgaagccagtgaaaaaggaactgttgttacggaaacagccgatgatgatttgtttacaacgtaccgtcttgatttagaagatgccagaagcaaagaaagagaagagctgaatgccattgtgtcaagcgatgatgcaacagccaaggagaaaagcgaagcatacgataaaatgacggctctcagtgaagtggaaggaacagaaaaacagctggaaacgctgattaaaacacaaggttacgaggatgcgcttgttaatgctgaaggagataaaatcaatattacagtcaaatcagacaaacactctaaatcgaaggcgacagccattatagaccttgtggcaaaagaaatcaaaacaatgaaagatgtcgctgtcacatttgaaccctctaaataagaatgagggaaaaaagcccgctaaacaagcgggctttttgcgttgctgtcatattagagttgaattcaaaagtccgctcctgtaagatgaacatagtatgtacttttagtagtaacctataaaaaaagaaatttcatacataggagtgcgattgaagttcggattagatccccctatgcaagggtttattgttttctaaaatctgattaccaattagaatgaatatttcccaaatattaaataataaaacaaaaaaattgaaaaaagtgtttccaccattttttcaatttttttataatttttttaatctgttatttaaatagtttatagttaaatttacattttcattagtccattcaatattctctccaagataactacgaactgctaacaaaattctctccctatgttctaatggagaagattcagccactgcatttcccgcaatatcttttggtatgattttacccgtgtccatagttaaaatcatacggcataaagttaatatagagttggtttcatcatcctgataattatctattaattcctctgacgaatccataatggctcttctcacatcagaaaatggaatatcaggtagtaattcctctaagtcataatttccgtatattcttttattttttcgttttgcttggtaaagcattatggttaaatctgaatttaattccttctgaggaatgtatccttgttcataaagctcttgtaaccattctccataaataaattcttgtttgggaggatgattccacggtaccatttcttgctgaataataattgttaattcaatatatcgtaagttgcttttatctcctattttttttgaaataggtctaattttttgtataagtatttctttactttgatctgtcaatggttcagatacgacgactaaaaagtcaagatcactatttggttttagtccactctcaactcctgatccaaacatgtaagtaccaataaggttattttttaaatgtttccgaagtatttttttcactttattaatttgttcgtatgtattcaaatatatcctcctcactattttgattagtacctattttatatccatagttgttaattaaataaacttaatttagtttatttatagatttcattggcttctaaattttttatctagataataattattttagttaattttattctagattatatatgatatgatctttcatttccataaaactaaagtaagtgtaaacctattcattgttttaaaaatatctcttgccagtcacgttacgttattagttatagttattataacatgtattcacgaacgaaaatcgcatcgattgctcttcagcgccgatggtagtcgggggtttccccctgtgagagtaggacgccgccaagcaagcttaaacccagctcaatgagctgggttttttgtattttggtttattggtatcataaaattccacttaactgtataatataataactttataccgaattttaaatcagcaatcaggttttgtggaccgggaaaatggaaataatgaaggatagagcgagaaagttgaaaattctcgagaaacggcttatagtaagattaaagtcaaatatagtcaaagtcagtaaaggagggggttgacgagntgaaatcatatgttaaatatcaaagaaatccacgagctgattaaagcaattgacgagtctacaattgacgaattcgtatatgaaaatgaaggtgtatccttaaaactgaaaaaacacgaagcaggcacggttcaagtcatgcagcaggcaccggcagcacctgtacaagcacaggctccgcaggcagttcagccgcaagcgcagcaagcagcggcacctgcccaagaagcaccaaagcaagatgagaatctgcataaaatcacttcaccaatggtaggaacattttatgcttcttcatcaccggaagctggcccgtatgtaacagccggttcaaaagtaaatgaaaacacagttgtctgcattgtagaagcgatgaagcttttcaacgaaatcgaagcagaagtgaaaggcgaaatcgttgaagtattagtagaaaacggccagctggtcgaatacggacaaccaattttattgcaataacaggtgcttacttttctggagttctttagcaaatttttttattagctgaacttagtattagtggccatactcctccaatccaaagctatttagaaagattactatatcctcaaacaggcggtaaccggcctcttcatcgggaatgcgcgcgaccttcagcatcgccggcatgtccccctggcggacgggaagtatccagctcgaggtcgggccgcgttgctggcgtttttccataggctccgcccccctgacgagcatcacaaaaatcgacgctcaagtcagaggtggcgaaacccgacaggactataaagataccaggcgtttccccctggaagctccctcgtgcgctctcctgttccgaccctgccgcttaccggatacctgtccgcctttctcccttcgggaagcgtggcgctttctcatagctcacgctgtaggtatctcagttcggtgtaggtcgttcgctccaagctgggctgtgtgcacgaaccccccgttcagcccgaccgctgcgccttatccggtaactatcgtcttgagtccaacccggtaagacacgacttatcgccactggcagcagccactggtaacaggattagcagagcgaggtatgtaggcggtgctacagagttcttgaagtggtggcctaactacggctacactagaaggacagtatttggtatctgcgctctgctgaagccagttaccttcggaaaaagagttgatagctcttgatccggcaaacaaaccaccgctggtagcggtggtttttttgtttgcaagcagcagattacgcgcagaaaaaaaggatctcaagaagatcctttgatcttttctacggggtctgacgctcagtggaacgaaaactcacgttaagggattttggtcatgagattatcaaaaaggatcttcacctagatccttttaaattaaaaatgaagttttaaatcaatctaaagtatatatgagtaaacttggtctgacagttaccaatgcttaatcagtgaggcacctatctcagcgatctgtctatttcgttcatccatagttgcctgactccccgtcgtgtagataactacgatacgggagggcttaccatctggccccagtgctgcaatgataccgcgagacccacgctcaccggctccagatttatcagcaataaaccagccagccggaagggccgagcgcagaagtggtcctgcaactttatccgcctccatccagtctattaattgttgccgggaagctagagtaagtagttcgccagttaatagtttgcgcaacgttgttgccattgctgcaggcatcgtggtgtcacgctcgtcgtttggtatggcttcattcagctccggttcccaacgatcaaggcgagttacatgatcccccatgttgtgcaaaaaagcggttagctccttcggtcctccgatcgttgtcagaagtaagttggccgcagtgttatcactcatggttatggcagcactgcataattctcttactgtcatgccatccgtaagatgcttttctgtgactggtgagtactcaaccaagtcattctgagaatagtgtatgcggcgaccgagttgctcttgcccggcgtcaacacgggataataccgcgccacatagcagaactttaaaagtgctcatcattggaaaacgttcttcggggcgaaaactctcaaggatcttaccgctgttgagatccagttcgatgtaacccactcgtgcacccaactgatcttcagcatcttttactttcaccagcgtttctgggtgagcaaaaacaggaaggcaaaatgccgcaaaaaagggaataagggcgacacggaaatgttgaatactcatactcttcctttttcaatattattgaagcatttatcagggttattgtctcatgagcggatacatatttgaatgtatttagaaaaataaacaaataggggttccgcgcacatttccccgaaaagtgccacctgacgtctaagaaaccattattatcatgacattaacctataaaaataggcgtatcacgaggccctttcgtcttcaagaatt

SEQ ID NO: 205 - DNA, 4699 bp, synthetic
  plasmid (1)..(4699): plasmid pEG161
  misc_feature (88)..(676): homology region accC upstream
  promoter (1858)..(2156): burden adiction promoter p(dnaK)
  rbs (2157)..(2162): rbs
  misc_feature (2162)..(2162): N is A, T, C or G
  misc_feature (2172)..(2626): homology region accC downstream
aacaaaattctccagtcttcacatcggtttgaaaggaggaagcggaagaatgaagtaagagggatttttgactccgaagtaagtcttagggaacgaaagattcatcagcagacaaggaaacatccgctgaagccagtgaaaaaggaactgttgttacggaaacagccgatgatgatttgtttacaacgtaccgtcttgatttagaagatgccagaagcaaagaaagagaagagctgaatgccattgtgtcaagcgatgatgcaacagccaaggagaaaagcgaagcatacgataaaatgacggctctcagtgaagtggaaggaacagaaaaacagctggaaacgctgattaaaacacaaggttacgaggatgcgcttgttaatgctgaaggagataaaatcaatattacagtcaaatcagacaaacactctaaatcgaaggcgacagccattatagaccttgtggcaaaagaaatcaaaacaatgaaagatgtcgctgtcacatttgaaccctctaaataagaatgagggaaaaaagcccgctaaacaagcgggctttttgcgttgctgtcatattagagttgaattcaaaagtccgctcctgtaagatgaacatagtatgtacttttagtagtaacctataaaaaaagaaatttcatacataggagtgcgattgaagttcggattagatccccctatgcaagggtttattgttttctaaaatctgattaccaattagaatgaatatttcccaaatattaaataataaaacaaaaaaattgaaaaaagtgtttccaccattttttcaatttttttataatttttttaatctgttatttaaatagtttatagttaaatttacattttcattagtccattcaatattctctccaagataactacgaactgctaacaaaattctctccctatgttctaatggagaagattcagccactgcatttcccgcaatatcttttggtatgattttacccgtgtccatagttaaaatcatacggcataaagttaatatagagttggtttcatcatcctgataattatctattaattcctctgacgaatccataatggctcttctcacatcagaaaatggaatatcaggtagtaattcctctaagtcataatttccgtatattcttttattttttcgttttgcttggtaaagcattatggttaaatctgaatttaattccttctgaggaatgtatccttgttcataaagctcttgtaaccattctccataaataaattcttgtttgggaggatgattccacggtaccatttcttgctgaataataattgttaattcaatatatcgtaagttgcttttatctcctattttttttgaaataggtctaattttttgtataagtatttctttactttgatctgtcaatggttcagatacgacgactaaaaagtcaagatcactatttggttttagtccactctcaactcctgatccaaacatgtaagtaccaataaggttattttttaaatgtttccgaagtatttttttcactttattaatttgttcgtatgtattcaaatatatcctcctcactattttgattagtacctattttatatccatagttgttaattaaataaacttaatttagtttatttatagatttcattggcttctaaattttttatctagataataattattttagttaattttattctagattatatatgatatgatctttcatttccataaaactaaagtaagtgtaaacctattcattgttttaaaaatatctcttgccagtcacgttacgttattagttatagttattataacatgtattcacgaacgaaaatcgcatcgattggttcaatccccgcacacgggaatttcgattaaaatcggaaaagaaaacgactatgaagagatggaaaattgcagtctgattacggcttcttattccgtagaccagaagcagatcggctcaattgcgattatcggcccgacccgcatgaattattccagggttgtcagcctgcttcagcatgtgacttcggacttgtcaaaagcattaacaagtctgtatgatgaataagggaattttggcaaattttatcgaagggcagcacctgtccttctccttacactttgagggaggtgaacacacgagntgaaatcatatgttaaatatcaaagaaatccacgagctgattaaagcaattgacgagtctacaattgacgaattcgtatatgaaaatgaaggtgtatccttaaaactgaaaaaacacgaagcaggcacggttcaagtcatgcagcaggcaccggcagcacctgtacaagcacaggctccgcaggcagttcagccgcaagcgcagcaagcagcggcacctgcccaagaagcaccaaagcaagatgagaatctgcataaaatcacttcaccaatggtaggaacattttatgcttcttcatcaccggaagctggcccgtatgtaacagccggttcaaaagtaaatgaaaacacagttgtctgcattgtagaagcgatgaagcttttcaacgaaatcgaagcagaagtgaaaggcgaaatcgttgaagtattagtagaaaacggccagctggtcgaatacggacaaccaattttattgcaataacaggtgcttacttttctggagttctttagcaaatttttttattagctgaacttagtattagtggccatactcctccaatccaaagctatttagaaagattactatatcctcaaacaggcggtaaccggcctcttcatcgggaatgcgcgcgaccttcagcatcgccggcatgtccccctggcggacgggaagtatccagctcgaggtcgggccgcgttgctggcgtttttccataggctccgcccccctgacgagcatcacaaaaatcgacgctcaagtcagaggtggcgaaacccgacaggactataaagataccaggcgtttccccctggaagctccctcgtgcgctctcctgttccgaccctgccgcttaccggatacctgtccgcctttctcccttcgggaagcgtggcgctttctcatagctcacgctgtaggtatctcagttcggtgtaggtcgttcgctccaagctgggctgtgtgcacgaaccccccgttcagcccgaccgctgcgccttatccggtaactatcgtcttgagtccaacccggtaagacacgacttatcgccactggcagcagccactggtaacaggattagcagagcgaggtatgtaggcggtgctacagagttcttgaagtggtggcctaactacggctacactagaaggacagtatttggtatctgcgctctgctgaagccagttaccttcggaaaaagagttgatagctcttgatccggcaaacaaaccaccgctggtagcggtggtttttttgtttgcaagcagcagattacgcgcagaaaaaaaggatctcaagaagatcctttgatcttttctacggggtctgacgctcagtggaacgaaaactcacgttaagggattttggtcatgagattatcaaaaaggatcttcacctagatccttttaaattaaaaatgaagttttaaatcaatctaaagtatatatgagtaaacttggtctgacagttaccaatgcttaatcagtgaggcacctatctcagcgatctgtctatttcgttcatccatagttgcctgactccccgtcgtgtagataactacgatacgggagggcttaccatctggccccagtgctgcaatgataccgcgagacccacgctcaccggctccagatttatcagcaataaaccagccagccggaagggccgagcgcagaagtggtcctgcaactttatccgcctccatccagtctattaattgttgccgggaagctagagtaagtagttcgccagttaatagtttgcgcaacgttgttgccattgctgcaggcatcgtggtgtcacgctcgtcgtttggtatggcttcattcagctccggttcccaacgatcaaggcgagttacatgatcccccatgttgtgcaaaaaagcggttagctccttcggtcctccgatcgttgtcagaagtaagttggccgcagtgttatcactcatggttatggcagcactgcataattctcttactgtcatgccatccgtaagatgcttttctgtgactggtgagtactcaaccaagtcattctgagaatagtgtatgcggcgaccgagttgctcttgcccggcgtcaacacgggataataccgcgccacatagcagaactttaaaagtgctcatcattggaaaacgttcttcggggcgaaaactctcaaggatcttaccgctgttgagatccagttcgatgtaacccactcgtgcacccaactgatcttcagcatcttttactttcaccagcgtttctgggtgagcaaaaacaggaaggcaaaatgccgcaaaaaagggaataagggcgacacggaaatgttgaatactcatactcttcctttttcaatattattgaagcatttatcagggttattgtctcatgagcggatacatatttgaatgtatttagaaaaataaacaaataggggttccgcgcacatttccccgaaaagtgccacctgacgtctaagaaaccattattatcatgacattaacctataaaaataggcgtatcacgaggccctttcgtcttcaagaatt

SEQ ID NO: 206 - DNA, 4699 bp, synthetic
  plasmid (1)..(4699): plasmid pEG162
  misc_feature (88)..(676): homology region accC upstream
  promoter (1858)..(2156): burden adictionpromoter p(perR)
  rbs (2157)..(2162): rbs
  misc_feature (2162)..(2162): N is A, T, C or G
  misc_feature (2172)..(2626): homology region accC downstream
aacaaaattctccagtcttcacatcggtttgaaaggaggaagcggaagaatgaagtaagagggatttttgactccgaagtaagtcttagggaacgaaagattcatcagcagacaaggaaacatccgctgaagccagtgaaaaaggaactgttgttacggaaacagccgatgatgatttgtttacaacgtaccgtcttgatttagaagatgccagaagcaaagaaagagaagagctgaatgccattgtgtcaagcgatgatgcaacagccaaggagaaaagcgaagcatacgataaaatgacggctctcagtgaagtggaaggaacagaaaaacagctggaaacgctgattaaaacacaaggttacgaggatgcgcttgttaatgctgaaggagataaaatcaatattacagtcaaatcagacaaacactctaaatcgaaggcgacagccattatagaccttgtggcaaaagaaatcaaaacaatgaaagatgtcgctgtcacatttgaaccctctaaataagaatgagggaaaaaagcccgctaaacaagcgggctttttgcgttgctgtcatattagagttgaattcaaaagtccgctcctgtaagatgaacatagtatgtacttttagtagtaacctataaaaaaagaaatttcatacataggagtgcgattgaagttcggattagatccccctatgcaagggtttattgttttctaaaatctgattaccaattagaatgaatatttcccaaatattaaataataaaacaaaaaaattgaaaaaagtgtttccaccattttttcaatttttttataatttttttaatctgttatttaaatagtttatagttaaatttacattttcattagtccattcaatattctctccaagataactacgaactgctaacaaaattctctccctatgttctaatggagaagattcagccactgcatttcccgcaatatcttttggtatgattttacccgtgtccatagttaaaatcatacggcataaagttaatatagagttggtttcatcatcctgataattatctattaattcctctgacgaatccataatggctcttctcacatcagaaaatggaatatcaggtagtaattcctctaagtcataatttccgtatattcttttattttttcgttttgcttggtaaagcattatggttaaatctgaatttaattccttctgaggaatgtatccttgttcataaagctcttgtaaccattctccataaataaattcttgtttgggaggatgattccacggtaccatttcttgctgaataataattgttaattcaatatatcgtaagttgcttttatctcctattttttttgaaataggtctaattttttgtataagtatttctttactttgatctgtcaatggttcagatacgacgactaaaaagtcaagatcactatttggttttagtccactctcaactcctgatccaaacatgtaagtaccaataaggttattttttaaatgtttccgaagtatttttttcactttattaatttgttcgtatgtattcaaatatatcctcctcactattttgattagtacctattttatatccatagttgttaattaaataaacttaatttagtttatttatagatttcattggcttctaaattttttatctagataataattattttagttaattttattctagattatatatgatatgatctttcatttccataaaactaaagtaagtgtaaacctattcattgttttaaaaatatctcttgccagtcacgttacgttattagttatagttattataacatgtattcacgaacgaaaatcgcatcgattggaagcatttgatgtgtggaagctgaagaaaaacttcggaaaagagtatatgggaatcgagcgttccacttttttaattgataaagaaggccggctcattaaagaatggagaaaagtaaaagtaaaggaccatgtagccgaagcgcttcaaaccctcaaagatatgtctgaaaagtaaatctctatgagcctatgcttacttttaccctgatatcaattgacaaattatcgtagaaagagttacactaattataaacattacaatgtaagaattttttttagaagagaggtgcatgacggcgagntgaaatcatatgttaaatatcaaagaaatccacgagctgattaaagcaattgacgagtctacaattgacgaattcgtatatgaaaatgaaggtgtatccttaaaactgaaaaaacacgaagcaggcacggttcaagtcatgcagcaggcaccggcagcacctgtacaagcacaggctccgcaggcagttcagccgcaagcgcagcaagcagcggcacctgcccaagaagcaccaaagcaagatgagaatctgcataaaatcacttcaccaatggtaggaacattttatgcttcttcatcaccggaagctggcccgtatgtaacagccggttcaaaagtaaatgaaaacacagttgtctgcattgtagaagcgatgaagcttttcaacgaaatcgaagcagaagtgaaaggcgaaatcgttgaagtattagtagaaaacggccagctggtcgaatacggacaaccaattttattgcaataacaggtgcttacttttctggagttctttagcaaatttttttattagctgaacttagtattagtggccatactcctccaatccaaagctatttagaaagattactatatcctcaaacaggcggtaaccggcctcttcatcgggaatgcgcgcgaccttcagcatcgccggcatgtccccctggcggacgggaagtatccagctcgaggtcgggccgcgttgctggcgtttttccataggctccgcccccctgacgagcatcacaaaaatcgacgctcaagtcagaggtggcgaaacccgacaggactataaagataccaggcgtttccccctggaagctccctcgtgcgctctcctgttccgaccctgccgcttaccggatacctgtccgcctttctcccttcgggaagcgtggcgctttctcatagctcacgctgtaggtatctcagttcggtgtaggtcgttcgctccaagctgggctgtgtgcacgaaccccccgttcagcccgaccgctgcgccttatccggtaactatcgtcttgagtccaacccggtaagacacgacttatcgccactggcagcagccactggtaacaggattagcagagcgaggtatgtaggcggtgctacagagttcttgaagtggtggcctaactacggctacactagaaggacagtatttggtatctgcgctctgctgaagccagttaccttcggaaaaagagttgatagctcttgatccggcaaacaaaccaccgctggtagcggtggtttttttgtttgcaagcagcagattacgcgcagaaaaaaaggatctcaagaagatcctttgatcttttctacggggtctgacgctcagtggaacgaaaactcacgttaagggattttggtcatgagattatcaaaaaggatcttcacctagatccttttaaattaaaaatgaagttttaaatcaatctaaagtatatatgagtaaacttggtctgacagttaccaatgcttaatcagtgaggcacctatctcagcgatctgtctatttcgttcatccatagttgcctgactccccgtcgtgtagataactacgatacgggagggcttaccatctggccccagtgctgcaatgataccgcgagacccacgctcaccggctccagatttatcagcaataaaccagccagccggaagggccgagcgcagaagtggtcctgcaactttatccgcctccatccagtctattaattgttgccgggaagctagagtaagtagttcgccagttaatagtttgcgcaacgttgttgccattgctgcaggcatcgtggtgtcacgctcgtcgtttggtatggcttcattcagctccggttcccaacgatcaaggcgagttacatgatcccccatgttgtgcaaaaaagcggttagctccttcggtcctccgatcgttgtcagaagtaagttggccgcagtgttatcactcatggttatggcagcactgcataattctcttactgtcatgccatccgtaagatgcttttctgtgactggtgagtactcaaccaagtcattctgagaatagtgtatgcggcgaccgagttgctcttgcccggcgtcaacacgggataataccgcgccacatagcagaactttaaaagtgctcatcattggaaaacgttcttcggggcgaaaactctcaaggatcttaccgctgttgagatccagttcgatgtaacccactcgtgcacccaactgatcttcagcatcttttactttcaccagcgtttctgggtgagcaaaaacaggaaggcaaaatgccgcaaaaaagggaataagggcgacacggaaatgttgaatactcatactcttcctttttcaatattattgaagcatttatcagggttattgtctcatgagcggatacatatttgaatgtatttagaaaaataaacaaataggggttccgcgcacatttccccgaaaagtgccacctgacgtctaagaaaccattattatcatgacattaacctataaaaataggcgtatcacgaggccctttcgtcttcaagaatt

SEQ ID NO: 207 - DNA, 4699 bp, synthetic
  plasmid (1)..(4699): plasmid pEG163
  misc_feature (88)..(676): homology region accC upstream
  promoter (1858)..(2156): burden adiction promoter p(hrcA)
  rbs (2157)..(2162): rbs
  misc_feature (2162)..(2162): N is A, T , C or G
  misc_feature (2172)..(2626): homology region accC downstream
aacaaaattctccagtcttcacatcggtttgaaaggaggaagcggaagaatgaagtaagagggatttttgactccgaagtaagtcttagggaacgaaagattcatcagcagacaaggaaacatccgctgaagccagtgaaaaaggaactgttgttacggaaacagccgatgatgatttgtttacaacgtaccgtcttgatttagaagatgccagaagcaaagaaagagaagagctgaatgccattgtgtcaagcgatgatgcaacagccaaggagaaaagcgaagcatacgataaaatgacggctctcagtgaagtggaaggaacagaaaaacagctggaaacgctgattaaaacacaaggttacgaggatgcgcttgttaatgctgaaggagataaaatcaatattacagtcaaatcagacaaacactctaaatcgaaggcgacagccattatagaccttgtggcaaaagaaatcaaaacaatgaaagatgtcgctgtcacatttgaaccctctaaataagaatgagggaaaaaagcccgctaaacaagcgggctttttgcgttgctgtcatattagagttgaattcaaaagtccgctcctgtaagatgaacatagtatgtacttttagtagtaacctataaaaaaagaaatttcatacataggagtgcgattgaagttcggattagatccccctatgcaagggtttattgttttctaaaatctgattaccaattagaatgaatatttcccaaatattaaataataaaacaaaaaaattgaaaaaagtgtttccaccattttttcaatttttttataatttttttaatctgttatttaaatagtttatagttaaatttacattttcattagtccattcaatattctctccaagataactacgaactgctaacaaaattctctccctatgttctaatggagaagattcagccactgcatttcccgcaatatcttttggtatgattttacccgtgtccatagttaaaatcatacggcataaagttaatatagagttggtttcatcatcctgataattatctattaattcctctgacgaatccataatggctcttctcacatcagaaaatggaatatcaggtagtaattcctctaagtcataatttccgtatattcttttattttttcgttttgcttggtaaagcattatggttaaatctgaatttaattccttctgaggaatgtatccttgttcataaagctcttgtaaccattctccataaataaattcttgtttgggaggatgattccacggtaccatttcttgctgaataataattgttaattcaatatatcgtaagttgcttttatctcctattttttttgaaataggtctaattttttgtataagtatttctttactttgatctgtcaatggttcagatacgacgactaaaaagtcaagatcactatttggttttagtccactctcaactcctgatccaaacatgtaagtaccaataaggttattttttaaatgtttccgaagtatttttttcactttattaatttgttcgtatgtattcaaatatatcctcctcactattttgattagtacctattttatatccatagttgttaattaaataaacttaatttagtttatttatagatttcattggcttctaaattttttatctagataataattattttagttaattttattctagattatatatgatatgatctttcatttccataaaactaaagtaagtgtaaacctattcattgttttaaaaatatctcttgccagtcacgttacgttattagttatagttattataacatgtattcacgaacgaaaatcgcatcgatttgaggaagaaatgtttttaggtttgagaaaaacagccggtgtcagcaaaaaacgattcgcagaaaaatacggccgttccctggatggacttttcccaagcgtgttaaaagacctcgctgaaaaagggctgattcacaattcggagtctgccgtttatttgactcatcaagggaaattattaggcaatgaagtttttggcgcttttttgggtgagttataattgacatttttcttgtggtttgatacttttgttatagaattagcactcgcttattgagagtgctaacagaggtgatgatgcgagntgaaatcatatgttaaatatcaaagaaatccacgagctgattaaagcaattgacgagtctacaattgacgaattcgtatatgaaaatgaaggtgtatccttaaaactgaaaaaacacgaagcaggcacggttcaagtcatgcagcaggcaccggcagcacctgtacaagcacaggctccgcaggcagttcagccgcaagcgcagcaagcagcggcacctgcccaagaagcaccaaagcaagatgagaatctgcataaaatcacttcaccaatggtaggaacattttatgcttcttcatcaccggaagctggcccgtatgtaacagccggttcaaaagtaaatgaaaacacagttgtctgcattgtagaagcgatgaagcttttcaacgaaatcgaagcagaagtgaaaggcgaaatcgttgaagtattagtagaaaacggccagctggtcgaatacggacaaccaattttattgcaataacaggtgcttacttttctggagttctttagcaaatttttttattagctgaacttagtattagtggccatactcctccaatccaaagctatttagaaagattactatatcctcaaacaggcggtaaccggcctcttcatcgggaatgcgcgcgaccttcagcatcgccggcatgtccccctggcggacgggaagtatccagctcgaggtcgggccgcgttgctggcgtttttccataggctccgcccccctgacgagcatcacaaaaatcgacgctcaagtcagaggtggcgaaacccgacaggactataaagataccaggcgtttccccctggaagctccctcgtgcgctctcctgttccgaccctgccgcttaccggatacctgtccgcctttctcccttcgggaagcgtggcgctttctcatagctcacgctgtaggtatctcagttcggtgtaggtcgttcgctccaagctgggctgtgtgcacgaaccccccgttcagcccgaccgctgcgccttatccggtaactatcgtcttgagtccaacccggtaagacacgacttatcgccactggcagcagccactggtaacaggattagcagagcgaggtatgtaggcggtgctacagagttcttgaagtggtggcctaactacggctacactagaaggacagtatttggtatctgcgctctgctgaagccagttaccttcggaaaaagagttgatagctcttgatccggcaaacaaaccaccgctggtagcggtggtttttttgtttgcaagcagcagattacgcgcagaaaaaaaggatctcaagaagatcctttgatcttttctacggggtctgacgctcagtggaacgaaaactcacgttaagggattttggtcatgagattatcaaaaaggatcttcacctagatccttttaaattaaaaatgaagttttaaatcaatctaaagtatatatgagtaaacttggtctgacagttaccaatgcttaatcagtgaggcacctatctcagcgatctgtctatttcgttcatccatagttgcctgactccccgtcgtgtagataactacgatacgggagggcttaccatctggccccagtgctgcaatgataccgcgagacccacgctcaccggctccagatttatcagcaataaaccagccagccggaagggccgagcgcagaagtggtcctgcaactttatccgcctccatccagtctattaattgttgccgggaagctagagtaagtagttcgccagttaatagtttgcgcaacgttgttgccattgctgcaggcatcgtggtgtcacgctcgtcgtttggtatggcttcattcagctccggttcccaacgatcaaggcgagttacatgatcccccatgttgtgcaaaaaagcggttagctccttcggtcctccgatcgttgtcagaagtaagttggccgcagtgttatcactcatggttatggcagcactgcataattctcttactgtcatgccatccgtaagatgcttttctgtgactggtgagtactcaaccaagtcattctgagaatagtgtatgcggcgaccgagttgctcttgcccggcgtcaacacgggataataccgcgccacatagcagaactttaaaagtgctcatcattggaaaacgttcttcggggcgaaaactctcaaggatcttaccgctgttgagatccagttcgatgtaacccactcgtgcacccaactgatcttcagcatcttttactttcaccagcgtttctgggtgagcaaaaacaggaaggcaaaatgccgcaaaaaagggaataagggcgacacggaaatgttgaatactcatactcttcctttttcaatattattgaagcatttatcagggttattgtctcatgagcggatacatatttgaatgtatttagaaaaataaacaaataggggttccgcgcacatttccccgaaaagtgccacctgacgtctaagaaaccattattatcatgacattaacctataaaaataggcgtatcacgaggccctttcgtcttcaagaatt

SEQ ID NO: 208 - DNA, 4699 bp, synthetic
  plasmid (1)..(4699): plasmid pEG164
  misc_feature (88)..(676): homology region accC upstream
  promoter (1858)..(2156): burden adiction promoter p(spxA)
  rbs (2157)..(2162): rbs
  misc_feature (2162)..(2162): N is A, T, C or G
  misc_feature (2172)..(2626): homology region accC downstream
aacaaaattctccagtcttcacatcggtttgaaaggaggaagcggaagaatgaagtaagagggatttttgactccgaagtaagtcttagggaacgaaagattcatcagcagacaaggaaacatccgctgaagccagtgaaaaaggaactgttgttacggaaacagccgatgatgatttgtttacaacgtaccgtcttgatttagaagatgccagaagcaaagaaagagaagagctgaatgccattgtgtcaagcgatgatgcaacagccaaggagaaaagcgaagcatacgataaaatgacggctctcagtgaagtggaaggaacagaaaaacagctggaaacgctgattaaaacacaaggttacgaggatgcgcttgttaatgctgaaggagataaaatcaatattacagtcaaatcagacaaacactctaaatcgaaggcgacagccattatagaccttgtggcaaaagaaatcaaaacaatgaaagatgtcgctgtcacatttgaaccctctaaataagaatgagggaaaaaagcccgctaaacaagcgggctttttgcgttgctgtcatattagagttgaattcaaaagtccgctcctgtaagatgaacatagtatgtacttttagtagtaacctataaaaaaagaaatttcatacataggagtgcgattgaagttcggattagatccccctatgcaagggtttattgttttctaaaatctgattaccaattagaatgaatatttcccaaatattaaataataaaacaaaaaaattgaaaaaagtgtttccaccattttttcaatttttttataatttttttaatctgttatttaaatagtttatagttaaatttacattttcattagtccattcaatattctctccaagataactacgaactgctaacaaaattctctccctatgttctaatggagaagattcagccactgcatttcccgcaatatcttttggtatgattttacccgtgtccatagttaaaatcatacggcataaagttaatatagagttggtttcatcatcctgataattatctattaattcctctgacgaatccataatggctcttctcacatcagaaaatggaatatcaggtagtaattcctctaagtcataatttccgtatattcttttattttttcgttttgcttggtaaagcattatggttaaatctgaatttaattccttctgaggaatgtatccttgttcataaagctcttgtaaccattctccataaataaattcttgtttgggaggatgattccacggtaccatttcttgctgaataataattgttaattcaatatatcgtaagttgcttttatctcctattttttttgaaataggtctaattttttgtataagtatttctttactttgatctgtcaatggttcagatacgacgactaaaaagtcaagatcactatttggttttagtccactctcaactcctgatccaaacatgtaagtaccaataaggttattttttaaatgtttccgaagtatttttttcactttattaatttgttcgtatgtattcaaatatatcctcctcactattttgattagtacctattttatatccatagttgttaattaaataaacttaatttagtttatttatagatttcattggcttctaaattttttatctagataataattattttagttaattttattctagattatatatgatatgatctttcatttccataaaactaaagtaagtgtaaacctattcattgttttaaaaatatctcttgccagtcacgttacgttattagttatagttattataacatgtattcacgaacgaaaatcgcatcgattgaaaacattcatacttataaagatgagaaatggtacggagaatcgtacgaaaaaacggatgaggtcttggaaatcatcgatgaagaaaaacaaaaaaatattttcgatcagttaagctaattgagaataagaacatatcatgaacattaaaaatttgctggattgacacatttttttcttaggatactgttcacacttacttttttatagtataatacctgtaaagattccttttttagagtaatttcaatttaagaataaaatagatgttcatcctactaattagaggagtgaagatgacgagntgaaatcatatgttaaatatcaaagaaatccacgagctgattaaagcaattgacgagtctacaattgacgaattcgtatatgaaaatgaaggtgtatccttaaaactgaaaaaacacgaagcaggcacggttcaagtcatgcagcaggcaccggcagcacctgtacaagcacaggctccgcaggcagttcagccgcaagcgcagcaagcagcggcacctgcccaagaagcaccaaagcaagatgagaatctgcataaaatcacttcaccaatggtaggaacattttatgcttcttcatcaccggaagctggcccgtatgtaacagccggttcaaaagtaaatgaaaacacagttgtctgcattgtagaagcgatgaagcttttcaacgaaatcgaagcagaagtgaaaggcgaaatcgttgaagtattagtagaaaacggccagctggtcgaatacggacaaccaattttattgcaataacaggtgcttacttttctggagttctttagcaaatttttttattagctgaacttagtattagtggccatactcctccaatccaaagctatttagaaagattactatatcctcaaacaggcggtaaccggcctcttcatcgggaatgcgcgcgaccttcagcatcgccggcatgtccccctggcggacgggaagtatccagctcgaggtcgggccgcgttgctggcgtttttccataggctccgcccccctgacgagcatcacaaaaatcgacgctcaagtcagaggtggcgaaacccgacaggactataaagataccaggcgtttccccctggaagctccctcgtgcgctctcctgttccgaccctgccgcttaccggatacctgtccgcctttctcccttcgggaagcgtggcgctttctcatagctcacgctgtaggtatctcagttcggtgtaggtcgttcgctccaagctgggctgtgtgcacgaaccccccgttcagcccgaccgctgcgccttatccggtaactatcgtcttgagtccaacccggtaagacacgacttatcgccactggcagcagccactggtaacaggattagcagagcgaggtatgtaggcggtgctacagagttcttgaagtggtggcctaactacggctacactagaaggacagtatttggtatctgcgctctgctgaagccagttaccttcggaaaaagagttgatagctcttgatccggcaaacaaaccaccgctggtagcggtggtttttttgtttgcaagcagcagattacgcgcagaaaaaaaggatctcaagaagatcctttgatcttttctacggggtctgacgctcagtggaacgaaaactcacgttaagggattttggtcatgagattatcaaaaaggatcttcacctagatccttttaaattaaaaatgaagttttaaatcaatctaaagtatatatgagtaaacttggtctgacagttaccaatgcttaatcagtgaggcacctatctcagcgatctgtctatttcgttcatccatagttgcctgactccccgtcgtgtagataactacgatacgggagggcttaccatctggccccagtgctgcaatgataccgcgagacccacgctcaccggctccagatttatcagcaataaaccagccagccggaagggccgagcgcagaagtggtcctgcaactttatccgcctccatccagtctattaattgttgccgggaagctagagtaagtagttcgccagttaatagtttgcgcaacgttgttgccattgctgcaggcatcgtggtgtcacgctcgtcgtttggtatggcttcattcagctccggttcccaacgatcaaggcgagttacatgatcccccatgttgtgcaaaaaagcggttagctccttcggtcctccgatcgttgtcagaagtaagttggccgcagtgttatcactcatggttatggcagcactgcataattctcttactgtcatgccatccgtaagatgcttttctgtgactggtgagtactcaaccaagtcattctgagaatagtgtatgcggcgaccgagttgctcttgcccggcgtcaacacgggataataccgcgccacatagcagaactttaaaagtgctcatcattggaaaacgttcttcggggcgaaaactctcaaggatcttaccgctgttgagatccagttcgatgtaacccactcgtgcacccaactgatcttcagcatcttttactttcaccagcgtttctgggtgagcaaaaacaggaaggcaaaatgccgcaaaaaagggaataagggcgacacggaaatgttgaatactcatactcttcctttttcaatattattgaagcatttatcagggttattgtctcatgagcggatacatatttgaatgtatttagaaaaataaacaaataggggttccgcgcacatttccccgaaaagtgccacctgacgtctaagaaaccattattatcatgacattaacctataaaaataggcgtatcacgaggccctttcgtcttcaagaatt

SEQ ID NO: 209 - DNA, 4699 bp, synthetic
  plasmid (1)..(4699): plasmid pEG165
  misc_feature (88)..(676): homology region accC upstream
  promoter (1858)..(2156): burden adiction promoter p(sigB)
  rbs (2157)..(2162): rbs
  misc_feature (2162)..(2162): N is A, T, C or G
  misc_feature (2172)..(2626): homology region accC downstream
aacaaaattctccagtcttcacatcggtttgaaaggaggaagcggaagaatgaagtaagagggatttttgactccgaagtaagtcttagggaacgaaagattcatcagcagacaaggaaacatccgctgaagccagtgaaaaaggaactgttgttacggaaacagccgatgatgatttgtttacaacgtaccgtcttgatttagaagatgccagaagcaaagaaagagaagagctgaatgccattgtgtcaagcgatgatgcaacagccaaggagaaaagcgaagcatacgataaaatgacggctctcagtgaagtggaaggaacagaaaaacagctggaaacgctgattaaaacacaaggttacgaggatgcgcttgttaatgctgaaggagataaaatcaatattacagtcaaatcagacaaacactctaaatcgaaggcgacagccattatagaccttgtggcaaaagaaatcaaaacaatgaaagatgtcgctgtcacatttgaaccctctaaataagaatgagggaaaaaagcccgctaaacaagcgggctttttgcgttgctgtcatattagagttgaattcaaaagtccgctcctgtaagatgaacatagtatgtacttttagtagtaacctataaaaaaagaaatttcatacataggagtgcgattgaagttcggattagatccccctatgcaagggtttattgttttctaaaatctgattaccaattagaatgaatatttcccaaatattaaataataaaacaaaaaaattgaaaaaagtgtttccaccattttttcaatttttttataatttttttaatctgttatttaaatagtttatagttaaatttacattttcattagtccattcaatattctctccaagataactacgaactgctaacaaaattctctccctatgttctaatggagaagattcagccactgcatttcccgcaatatcttttggtatgattttacccgtgtccatagttaaaatcatacggcataaagttaatatagagttggtttcatcatcctgataattatctattaattcctctgacgaatccataatggctcttctcacatcagaaaatggaatatcaggtagtaattcctctaagtcataatttccgtatattcttttattttttcgttttgcttggtaaagcattatggttaaatctgaatttaattccttctgaggaatgtatccttgttcataaagctcttgtaaccattctccataaataaattcttgtttgggaggatgattccacggtaccatttcttgctgaataataattgttaattcaatatatcgtaagttgcttttatctcctattttttttgaaataggtctaattttttgtataagtatttctttactttgatctgtcaatggttcagatacgacgactaaaaagtcaagatcactatttggttttagtccactctcaactcctgatccaaacatgtaagtaccaataaggttattttttaaatgtttccgaagtatttttttcactttattaatttgttcgtatgtattcaaatatatcctcctcactattttgattagtacctattttatatccatagttgttaattaaataaacttaatttagtttatttatagatttcattggcttctaaattttttatctagataataattattttagttaattttattctagattatatatgatatgatctttcatttccataaaactaaagtaagtgtaaacctattcattgttttaaaaatatctcttgccagtcacgttacgttattagttatagttattataacatgtattcacgaacgaaaatcgcatcgattaacaattcgatcagcatctggaaaagggcgatatgattgttttattttctgacggcgtcacagaatgcagaacggaaaacggtttcttggagcgtcctgatctgcagaagctcattgaggaacatatgtgttcctctgcgcaggaaatggtcaaaaacatttatgacagcctcctcaaattgcaggattttcagcttcacgatgattttacgttaattgttttgcggagaaaggtttaacgtctgtcagacgagggtataaagcaactagtgatttgaaggaaaatttgaggtgatacgacgagntgaaatcatatgttaaatatcaaagaaatccacgagctgattaaagcaattgacgagtctacaattgacgaattcgtatatgaaaatgaaggtgtatccttaaaactgaaaaaacacgaagcaggcacggttcaagtcatgcagcaggcaccggcagcacctgtacaagcacaggctccgcaggcagttcagccgcaagcgcagcaagcagcggcacctgcccaagaagcaccaaagcaagatgagaatctgcataaaatcacttcaccaatggtaggaacattttatgcttcttcatcaccggaagctggcccgtatgtaacagccggttcaaaagtaaatgaaaacacagttgtctgcattgtagaagcgatgaagcttttcaacgaaatcgaagcagaagtgaaaggcgaaatcgttgaagtattagtagaaaacggccagctggtcgaatacggacaaccaattttattgcaataacaggtgcttacttttctggagttctttagcaaatttttttattagctgaacttagtattagtggccatactcctccaatccaaagctatttagaaagattactatatcctcaaacaggcggtaaccggcctcttcatcgggaatgcgcgcgaccttcagcatcgccggcatgtccccctggcggacgggaagtatccagctcgaggtcgggccgcgttgctggcgtttttccataggctccgcccccctgacgagcatcacaaaaatcgacgctcaagtcagaggtggcgaaacccgacaggactataaagataccaggcgtttccccctggaagctccctcgtgcgctctcctgttccgaccctgccgcttaccggatacctgtccgcctttctcccttcgggaagcgtggcgctttctcatagctcacgctgtaggtatctcagttcggtgtaggtcgttcgctccaagctgggctgtgtgcacgaaccccccgttcagcccgaccgctgcgccttatccggtaactatcgtcttgagtccaacccggtaagacacgacttatcgccactggcagcagccactggtaacaggattagcagagcgaggtatgtaggcggtgctacagagttcttgaagtggtggcctaactacggctacactagaaggacagtatttggtatctgcgctctgctgaagccagttaccttcggaaaaagagttgatagctcttgatccggcaaacaaaccaccgctggtagcggtggtttttttgtttgcaagcagcagattacgcgcagaaaaaaaggatctcaagaagatcctttgatcttttctacggggtctgacgctcagtggaacgaaaactcacgttaagggattttggtcatgagattatcaaaaaggatcttcacctagatccttttaaattaaaaatgaagttttaaatcaatctaaagtatatatgagtaaacttggtctgacagttaccaatgcttaatcagtgaggcacctatctcagcgatctgtctatttcgttcatccatagttgcctgactccccgtcgtgtagataactacgatacgggagggcttaccatctggccccagtgctgcaatgataccgcgagacccacgctcaccggctccagatttatcagcaataaaccagccagccggaagggccgagcgcagaagtggtcctgcaactttatccgcctccatccagtctattaattgttgccgggaagctagagtaagtagttcgccagttaatagtttgcgcaacgttgttgccattgctgcaggcatcgtggtgtcacgctcgtcgtttggtatggcttcattcagctccggttcccaacgatcaaggcgagttacatgatcccccatgttgtgcaaaaaagcggttagctccttcggtcctccgatcgttgtcagaagtaagttggccgcagtgttatcactcatggttatggcagcactgcataattctcttactgtcatgccatccgtaagatgcttttctgtgactggtgagtactcaaccaagtcattctgagaatagtgtatgcggcgaccgagttgctcttgcccggcgtcaacacgggataataccgcgccacatagcagaactttaaaagtgctcatcattggaaaacgttcttcggggcgaaaactctcaaggatcttaccgctgttgagatccagttcgatgtaacccactcgtgcacccaactgatcttcagcatcttttactttcaccagcgtttctgggtgagcaaaaacaggaaggcaaaatgccgcaaaaaagggaataagggcgacacggaaatgttgaatactcatactcttcctttttcaatattattgaagcatttatcagggttattgtctcatgagcggatacatatttgaatgtatttagaaaaataaacaaataggggttccgcgcacatttccccgaaaagtgccacctgacgtctaagaaaccattattatcatgacattaacctataaaaataggcgtatcacgaggccctttcgtcttcaagaatt

SEQ ID NO: 210 - DNA, 4699 bp, synthetic
  plasmid (1)..(4699): plasmid pEG166
  misc_feature (88)..(676): homology region accC upstream
  promoter (1858)..(2156): burden adiction promoter p(yflT)
  rbs (2157)..(2162): rbs
  misc_feature (2162)..(2162): N is A, T, C or G
  misc_feature (2172)..(2626): homology region accC downstream
aacaaaattctccagtcttcacatcggtttgaaaggaggaagcggaagaatgaagtaagagggatttttgactccgaagtaagtcttagggaacgaaagattcatcagcagacaaggaaacatccgctgaagccagtgaaaaaggaactgttgttacggaaacagccgatgatgatttgtttacaacgtaccgtcttgatttagaagatgccagaagcaaagaaagagaagagctgaatgccattgtgtcaagcgatgatgcaacagccaaggagaaaagcgaagcatacgataaaatgacggctctcagtgaagtggaaggaacagaaaaacagctggaaacgctgattaaaacacaaggttacgaggatgcgcttgttaatgctgaaggagataaaatcaatattacagtcaaatcagacaaacactctaaatcgaaggcgacagccattatagaccttgtggcaaaagaaatcaaaacaatgaaagatgtcgctgtcacatttgaaccctctaaataagaatgagggaaaaaagcccgctaaacaagcgggctttttgcgttgctgtcatattagagttgaattcaaaagtccgctcctgtaagatgaacatagtatgtacttttagtagtaacctataaaaaaagaaatttcatacataggagtgcgattgaagttcggattagatccccctatgcaagggtttattgttttctaaaatctgattaccaattagaatgaatatttcccaaatattaaataataaaacaaaaaaattgaaaaaagtgtttccaccattttttcaatttttttataatttttttaatctgttatttaaatagtttatagttaaatttacattttcattagtccattcaatattctctccaagataactacgaactgctaacaaaattctctccctatgttctaatggagaagattcagccactgcatttcccgcaatatcttttggtatgattttacccgtgtccatagttaaaatcatacggcataaagttaatatagagttggtttcatcatcctgataattatctattaattcctctgacgaatccataatggctcttctcacatcagaaaatggaatatcaggtagtaattcctctaagtcataatttccgtatattcttttattttttcgttttgcttggtaaagcattatggttaaatctgaatttaattccttctgaggaatgtatccttgttcataaagctcttgtaaccattctccataaataaattcttgtttgggaggatgattccacggtaccatttcttgctgaataataattgttaattcaatatatcgtaagttgcttttatctcctattttttttgaaataggtctaattttttgtataagtatttctttactttgatctgtcaatggttcagatacgacgactaaaaagtcaagatcactatttggttttagtccactctcaactcctgatccaaacatgtaagtaccaataaggttattttttaaatgtttccgaagtatttttttcactttattaatttgttcgtatgtattcaaatatatcctcctcactattttgattagtacctattttatatccatagttgttaattaaataaacttaatttagtttatttatagatttcattggcttctaaattttttatctagataataattattttagttaattttattctagattatatatgatatgatctttcatttccataaaactaaagtaagtgtaaacctattcattgttttaaaaatatctcttgccagtcacgttacgttattagttatagttattataacatgtattcacgaacgaaaatcgcatcgattgactaaatcactcacaatccaagcattgtattgctgttctggtgaaaagtattgcattagacatacctcctgctcgtacggataaaggcagcgtttcatggtcgtgtgctccgtgcagcggcttctccttaattttgatttttctgaaaataggtcccgttcctatcactttaccatggacggaaaacaaatagctactaccattcctcctgtttttctcttcaatgttctggaatctgtttcaggtacagacgatcgggtatgaaagaaatatagaaaacatgaaggaggaatatcgaccgagntgaaatcatatgttaaatatcaaagaaatccacgagctgattaaagcaattgacgagtctacaattgacgaattcgtatatgaaaatgaaggtgtatccttaaaactgaaaaaacacgaagcaggcacggttcaagtcatgcagcaggcaccggcagcacctgtacaagcacaggctccgcaggcagttcagccgcaagcgcagcaagcagcggcacctgcccaagaagcaccaaagcaagatgagaatctgcataaaatcacttcaccaatggtaggaacattttatgcttcttcatcaccggaagctggcccgtatgtaacagccggttcaaaagtaaatgaaaacacagttgtctgcattgtagaagcgatgaagcttttcaacgaaatcgaagcagaagtgaaaggcgaaatcgttgaagtattagtagaaaacggccagctggtcgaatacggacaaccaattttattgcaataacaggtgcttacttttctggagttctttagcaaatttttttattagctgaacttagtattagtggccatactcctccaatccaaagctatttagaaagattactatatcctcaaacaggcggtaaccggcctcttcatcgggaatgcgcgcgaccttcagcatcgccggcatgtccccctggcggacgggaagtatccagctcgaggtcgggccgcgttgctggcgtttttccataggctccgcccccctgacgagcatcacaaaaatcgacgctcaagtcagaggtggcgaaacccgacaggactataaagataccaggcgtttccccctggaagctccctcgtgcgctctcctgttccgaccctgccgcttaccggatacctgtccgcctttctcccttcgggaagcgtggcgctttctcatagctcacgctgtaggtatctcagttcggtgtaggtcgttcgctccaagctgggctgtgtgcacgaaccccccgttcagcccgaccgctgcgccttatccggtaactatcgtcttgagtccaacccggtaagacacgacttatcgccactggcagcagccactggtaacaggattagcagagcgaggtatgtaggcggtgctacagagttcttgaagtggtggcctaactacggctacactagaaggacagtatttggtatctgcgctctgctgaagccagttaccttcggaaaaagagttgatagctcttgatccggcaaacaaaccaccgctggtagcggtggtttttttgtttgcaagcagcagattacgcgcagaaaaaaaggatctcaagaagatcctttgatcttttctacggggtctgacgctcagtggaacgaaaactcacgttaagggattttggtcatgagattatcaaaaaggatcttcacctagatccttttaaattaaaaatgaagttttaaatcaatctaaagtatatatgagtaaacttggtctgacagttaccaatgcttaatcagtgaggcacctatctcagcgatctgtctatttcgttcatccatagttgcctgactccccgtcgtgtagataactacgatacgggagggcttaccatctggccccagtgctgcaatgataccgcgagacccacgctcaccggctccagatttatcagcaataaaccagccagccggaagggccgagcgcagaagtggtcctgcaactttatccgcctccatccagtctattaattgttgccgggaagctagagtaagtagttcgccagttaatagtttgcgcaacgttgttgccattgctgcaggcatcgtggtgtcacgctcgtcgtttggtatggcttcattcagctccggttcccaacgatcaaggcgagttacatgatcccccatgttgtgcaaaaaagcggttagctccttcggtcctccgatcgttgtcagaagtaagttggccgcagtgttatcactcatggttatggcagcactgcataattctcttactgtcatgccatccgtaagatgcttttctgtgactggtgagtactcaaccaagtcattctgagaatagtgtatgcggcgaccgagttgctcttgcccggcgtcaacacgggataataccgcgccacatagcagaactttaaaagtgctcatcattggaaaacgttcttcggggcgaaaactctcaaggatcttaccgctgttgagatccagttcgatgtaacccactcgtgcacccaactgatcttcagcatcttttactttcaccagcgtttctgggtgagcaaaaacaggaaggcaaaatgccgcaaaaaagggaataagggcgacacggaaatgttgaatactcatactcttcctttttcaatattattgaagcatttatcagggttattgtctcatgagcggatacatatttgaatgtatttagaaaaataaacaaataggggttccgcgcacatttccccgaaaagtgccacctgacgtctaagaaaccattattatcatgacattaacctataaaaataggcgtatcacgaggccctttcgtcttcaagaatt

SEQ ID NO: 211 - DNA, 783 bp, synthetic
  misc_feature (1)..(783): Gene encoding SpcR (resistance marker)
gtactaatcaaaatagtgaggaggatatatttgaatacatacgaacaaattaataaagtgaaaaaaatacttcggaaacatttaaaaaataaccttattggtacttacatgtttggatcaggagttgagagtggactaaaaccaaatagtgatcttgactttttagtcgtcgtatctgaaccattgacagatcaaagtaaagaaatacttatacaaaaaattagacctatttcaaaaaaaataggagataaaagcaacttacgatatattgaattaacaattattattcagcaagaaatggtaccgtggaatcatcctcccaaacaagaatttatttatggagaatggttacaagagctttatgaacaaggatacattcctcagaaggaattaaattcagatttaaccataatgctttaccaagcaaaacgaaaaaataaaagaatatacggaaattatgacttagaggaattactacctgatattccattttctgatgtgagaagagccattatggattcgtcagaggaattaatagataattatcaggatgatgaaaccaactctatattaactttatgccgtatgattttaactatggacacgggtaaaatcataccaaaagatattgcgggaaatgcagtggctgaatcttctccattagaacatagggagagaattttgttagcagttcgtagttatcttggagagaatattgaatggactaatgaaaatgtaaatttaactataaactatttaaataacagattaaaaaaattataa

SEQ ID NO: 212 - DNA, 296 bp, Bacillus
  promoter (1)..(296): Bacillus bruden sensing promoter p(groES)
aatgcggaaaactgcatgatgatatatgtcaaaataataaaccaatactgttttctcaaatggtatgtactcctttgttaagtgggtttcgttcatctacagctattgtaacataatcggtacgggggtgaaaaagctaacggaaaagggagcggaaaagaatgatgtaagcgtgaaaaattttttatcttatcacttgaaattggaagggagattctttattataagaattgtgttagcactctttagtgctgagtgctaaaattacatattcatactattgaggaggttatttc

SEQ ID NO: 213 - DNA, 299 bp, Bacillus
  promoter (1)..(299): Bacillus burden sensing promoter p(ctsR)
gctcttcagcgccgatggtagtcgggggtttccccctgtgagagtaggacgccgccaagcaagcttaaacccagctcaatgagctgggttttttgtattttggtttattggtatcataaaattccacttaactgtataatataataactttataccgaattttaaatcagcaatcaggttttgtggaccgggaaaatggaaataatgaaggatagagcgagaaagttgaaaattctcgagaaacggcttatagtaagattaaagtcaaatatagtcaaagtcagtaaaggagggggttg

SEQ ID NO: 214 - DNA, 299 bp, Bacillus
  promoter (1)..(299): Bacillus burden sensing promoter p(dnaK)
ggttcaatccccgcacacgggaatttcgattaaaatcggaaaagaaaacgactatgaagagatggaaaattgcagtctgattacggcttcttattccgtagaccagaagcagatcggctcaattgcgattatcggcccgacccgcatgaattattccagggttgtcagcctgcttcagcatgtgacttcggacttgtcaaaagcattaacaagtctgtatgatgaataagggaattttggcaaattttatcgaagggcagcacctgtccttctccttacactttgagggaggtgaacac

SEQ ID NO: 215 - DNA, 299 bp, Bacillus
  promoter (1)..(299): Bacillus burden addiction sensing p(perR)
ggaagcatttgatgtgtggaagctgaagaaaaacttcggaaaagagtatatgggaatcgagcgttccacttttttaattgataaagaaggccggctcattaaagaatggagaaaagtaaaagtaaaggaccatgtagccgaagcgcttcaaaccctcaaagatatgtctgaaaagtaaatctctatgagcctatgcttacttttaccctgatatcaattgacaaattatcgtagaaagagttacactaattataaacattacaatgtaagaattttttttagaagagaggtgcatgacg

SEQ ID NO: 216 - DNA, 299 bp, Bacillus
  promoter (1)..(299): Bacillus burden sensing promoter p(hrcA)
tgaggaagaaatgtttttaggtttgagaaaaacagccggtgtcagcaaaaaacgattcgcagaaaaatacggccgttccctggatggacttttcccaagcgtgttaaaagacctcgctgaaaaagggctgattcacaattcggagtctgccgtttatttgactcatcaagggaaattattaggcaatgaagtttttggcgcttttttgggtgagttataattgacatttttcttgtggtttgatacttttgttatagaattagcactcgcttattgagagtgctaacagaggtgatgat

SEQ ID NO: 217 - DNA, 299 bp, Bacillus
  promoter (1)..(299): Bacillus burden sensing promoter p(spxA)
gaaaacattcatacttataaagatgagaaatggtacggagaatcgtacgaaaaaacggatgaggtcttggaaatcatcgatgaagaaaaacaaaaaaatattttcgatcagttaagctaattgagaataagaacatatcatgaacattaaaaatttgctggattgacacatttttttcttaggatactgttcacacttacttttttatagtataatacctgtaaagattccttttttagagtaatttcaatttaagaataaaatagatgttcatcctactaattagaggagtgaagatg

SEQ ID NO: 218 - DNA, 299 bp, Bacillus
  promoter (1)..(299): Bacillus burden sensing promoter p(sigB)
aacaattcgatcagcatctggaaaagggcgatatgattgttttattttctgacggcgtcacagaatgcagaacggaaaacggtttcttggagcgtcctgatctgcagaagctcattgaggaacatatgtgttcctctgcgcaggaaatggtcaaaaacatttatgacagcctcctcaaattgcaggattttcagcttcacgatgattttacgttaattgttttgcggagaaaggtttaacgtctgtcagacgagggtataaagcaactagtgatttgaaggaaaatttgaggtgatacg

SEQ ID NO: 219 - DNA, 299 bp, Bacillus
  promoter (1)..(299): Bacillus burden sensing promoter p(yflT)
gactaaatcactcacaatccaagcattgtattgctgttctggtgaaaagtattgcattagacatacctcctgctcgtacggataaaggcagcgtttcatggtcgtgtgctccgtgcagcggcttctccttaattttgatttttctgaaaataggtcccgttcctatcactttaccatggacggaaaacaaatagctactaccattcctcctgtttttctcttcaatgttctggaatctgtttcaggtacagacgatcgggtatgaaagaaatatagaaaacatgaaggaggaatatcga

SEQ ID NO: 220 - DNA, 651 bp, synthetic
  CDS (1)..(651): chlR gene encoding camR resistance marker
atgaactttaataaaattgatttagacaattggaagagaaaagagatatttaatcattatttgaaccaacaaacgacttttagtataaccacagaaattgatattagtgttttataccgaaacataaaacaagaaggatataaattttaccctgcatttattttcttagtgacaagggtgataaactcaaatacagcttttagaactggttacaatagcgacggagagttaggttattgggataagttagagccactttatacaatttttgatggtgtatctaaaacattctctggtatttggactcctgtaaagaatgacttcaaagagttttatgatttatacctttctgatgtagagaaatataatggttcggggaaattgtttcccaaaacacctatacctgaaaatgctttttctctttctattattccatggacttcatttactgggtttaacttaaatatcaataataatagtaattaccttctacccattattacagcaggaaaattcattaataaaggtaattcaatatatttaccgctatctttacaggtacatcattctgtttgtgatggttatcatgcaggattgtttatgaactctattcaggaattgtcagataggcctaatgactggcttttataa

SEQ ID NO: 221 - protein, 216 aa, synthetic
MNFNKIDLDNWKRKEIFNHYLNQQTTFSITTEIDISVLYRNIKQEGYKFYPAFIFLVTRVINSNTAFRTGYNSDGELGYWDKLEPLYTIFDGVSKTFSGIWTPVKNDFKEFYDLYLSDVEKYNGSGKLFPKTPIPENAFSLSIIPWTSFTGFNLNINNNSNYLLPIITAGKFINKGNSIYLPLSLQVHHSVCDGYHAGLFMNSIQELSDRPNDWLL

SEQ ID NO: 222 - DNA, 10063 bp, synthetic
  plasmid (1)..(10063): plasmid pEG062
  misc_feature (1)..(637): homology region amyE upstream
  misc_feature (789)..(1583): resistance marker KanR (on complementary strand)
  terminator (1744)..(1796): terminator T7
  promoter (1866)..(2655): promoter P3P
  misc_feature (2680)..(3861): gene encoding IgA-V3
  misc_feature (3862)..(3867): glycine linker
  misc_feature (3868)..(4584): gene encoding sfGFP
  misc_feature (4585)..(4602): purification tag 6-his
  terminator (4614)..(4682): terminator
  misc_feature (5070)..(6262): homology region amyE downstream
  misc_feature (7207)..(7989): spc gene encoding resistance marker spectinomycun adenyltransferase
  misc_feature (8995)..(9855): bla gene encoding beta-lactamase for ampicillin resistance (on complementary strand)
ttaacaaaattctccagtcttcacatcggtttgaaaggaggaagcggaagaatgaagtaagagggatttttgactccgaagtaagtcttcaaaaaatcaaataaggagtgtcaagaatgtttgcaaaacgattcaaaacctctttactgccgttattcgctggatttttattgctgtttcatttggttctggcaggaccggcggctgcgagtgctgaaacggcgaacaaatcgaatgagcttacagcaccgtcgatcaaaagcggaaccattcttcatgcatggaattggtcgttcaatacgttaaaacacaatatgaaggatattcatgatgcaggatatacagccattcagacatctccgattaaccaagtaaaggaagggaatcaaggagataaaagcatgtcgaactggtactggctgtatcagccgacatcgtatcaaattggcaaccgttacttaggtactgaacaagaatttaaagaaatgtgtgcagccgctgaagaatatggcataaaggtcattgttgacgcggtcatcaatcataccaccagtgattatgccgcgatttccaatgaggttaagagtattccaaactggacacatggaaacacacaaattaaaaactggtctgatcggatcctagaagcttatcgaattctcatgtttgacagcttatcatcggcaatagttcggataatgagtttataaaataaaaaaagcacctgaaaaggtgtctttttttgatggttttgaacttgaagctttttagacatctaaatctaggtactaaaacaattcatccagtaaaatataatattttattttctcccaatcaggcttgatccccagtaagtcaaaaaatagctcgacatactgttcttccccgatatcctccctgatcgaccggacgcagaaggcaatgtcataccacttgtccgccctgccgcttctcccaagatcaataaagccacttactttgccatctttcacaaagatgttgctgtctcccaggtcgccgtgggaaaagacaagttcctcttcgggcttttccgtctttaaaaaatcatacagctcgcgcggatctttaaatggagtgtcttcttcccagttttcgcaatccacatcggccagatcgttattcagtaagtaatccaattcggctaagcggctgtctaagctattcgtatagggacaatccgatatgtcgatggagtgaaagagcctgatgcactccgcatacagctcgataatcttttcagggctttgttcatcttcatactcttccgagcaaaggacgccatcggcctcactcatgagcagattgctccagccatcatgccgttcaaagtgcaggacctttggaacaggcagctttccttccagccatagcatcatgtccttttcccgttccacatcataggtggtccctttataccggctgtccgtcatttttaaatataggttttcattttctcccaccagcttatataccttagcaggagacattccttccgtatcttttacgcagcggtatttttcgatcagttttttcaattccggtgatattctcattttagccatttattatttccttcctcttttctacagtatttaaagataccccaagaagctaattataacaagacgaactccaattcactgttccttgcattctaaaaccttaaataccagaaaacagacccaggtctttttcaaagttgttttgaaagttggcccgcatcccccctagcataaccccttggggcctctaaacgggtcttgaggggttttttggagctcaaacaattaatgtgagttagctcactcattaggcaccccaggctttacactttatgcgtctattcttttggaagaaaatatagggaaaatggtatttgttaaaaattctgaatatttatacaatatcatatgtttcacattgaaatatgctgtccagactgtccgctgtgtaaaaaataggaataaaggggggttgttattattttactgatatgtaaaatataatttgtataagaaaattcgaaacgtaagatgaaaccttagataaaagtgctttttttgttgcaattgaagaattattaatgttaagcttaattaaagataatatctttgaattgtaacgcccctcaaaagtaagaactacaaaaaaagaatacgttatatagaaatatgtttgaaccttcttcagattacaaatatattcggacggactctacctcaaatgcttatctaactatagaatgacatacaagcacaaccttgaaaatttgaaaatataactaccaatgaacttgttcatgtgaattatcgctgtatttaattttctcaattcaatatataatatgccaatacattgttacaagtagaaattaagacacccttgatagccttactatacctaacatgatgtagtattaaatgaatatgtaaatatatttatgataagaagcgacttatttataatcattacatatttttctattggaatgattaagattccaatagaatagtgtataaattatttatcttgaaaggagggatgcctaaaaacgaagaacattaaaaacatatatttgcaccgtctaatggatttatgaaaaatcattttatcagtttgaaaattatgtattatgattaactaataaggaggacaaacatgatccaaaaacgcaaacgcacagttagctttagactggttctgatgtgcacactgctgtttgtttcactgccgattacaaaaacaagcgcacaagttcaactgcaagaatcaggcggaggcctggttcaagcaggcggatcactgagactgtcatgcgcagcatcaggccttacatttgatacatatgcaatgggctggtttagacaagcaccgggaaaaaaacgcgaatatgttgcagcaatttcatggacaggcatcagcacatattatgcggatattgcaaaaggacgctttacaattagccgtgataatgcgaaaaacacgctgtatctgcaaatggattcactgaaaccggaagatacagcagtctattattgcgcagcacaaaaatcactgaatgttccggcaccgtgggattattggggacaaggcacacaagttacagtttcatcagatccgtgtccgcaatgctgcaaaccgtcactgtcactgcaaccgcctgcactggcggatctgctgctgggctcaaatgcatcactgacatgcacactgtcaggactgaaaaaatctgaaggcgtttcatttacatggcaaccgtcaggcggaaaagatgcagttcaagcatcaccgacaagagattcatgcggctgctattcagtttcaagcattcttccgggatgcgctgatccgtggaataaaggcgaaacattttcatgcacagcagcacattcagaactgaaatcagcactgacagcgacaattacaaaaccgaaagtcaatacatttcgtccgcaagttcatctgcttccgcctccgagcgaagaactggcactgaatgaactggttacacttacatgcctggttagaggcttttcaccgaaagatgttcttgttagatggctgcaaggcggacaagaactgccgagagataaatatctggtttgggaatcactgccggaaccgggacaagcaattccgacatatgcagttacatcagttcttagagttgatgcggaagattggaaacagggcgatacatttagctgcatggttggccatgaagcactgccgctggcatttacacaaaaaacaattgatagactggcaggcaaaccgacacatgttaatgtttcagttgttatggcagaagcagaaggcatctgctataaagatgaactgggtggcatgcgtaaaggcgaagagctgttcactggtttcgtcactattctggtggaactggatggtgatgtcaacggtcataagttttccgtgcgtggcgagggtgaaggtgacgcaactaatggtaaactgacgctgaagttcatctgtactactggtaaactgccggtaccttggccgactctggtaacgacgctgacttatggtgttcagtgctttgctcgttatccggaccacatgaagcagcatgacttcttcaagtccgccatgccggaaggctatgtgcaggaacgcacgatttcctttaaggatgacggcacgtacaaaacgcgtgcggaagtgaaatttgaaggcgataccctggtaaaccgcattgagctgaaaggcattgactttaaagaagacggcaatatcctgggccataagctggaatacaattttaacagccacaatgtttacatcaccgccgataaacaaaaaaatggcattaaagcgaattttaaaattcgccacaacgtggaggatggcagcgtgcagctggctgatcactaccagcaaaacactccaatcggtgatggtcctgttctgctgccagacaatcactatctgagcacgcaaagcgttctgtctaaagatccgaacgagaaacgcgatcacatggttctgctggagttcgtaaccgcagcgggcatcacgcatggtatggatgaactgtacaaataacaccaccatcatcaccattaaaagagcatgagaggacggatttcctgaaggaaatccgtttttttattttgcccgtcttataaatttctttgattacaaagctgttcttttataatatgagataatgccgactgtactttttacagtcggttttctaatgtcactaacctgccccgttagttgaagaaggtttttatattacagctccagatcctctacgccggacgcatcgtggccggcatcaccggcgccacaggtgcggttgctggcgcctatatcgccgacatcaccgatggggaagatcgggctcgccacttcgggctcatgagcgcttgtttcggcgtgggtatggtggcaggccccgtggccgggggactgttgggcgccatctccttgcatgcaccattccttgcggcggcggtgctcaacggcctcaacctactactgggctgcttcctaatgcaggagtcgcataagggagagcgtcgacatggatgagcgatgatgatatccgtttaggctgggcggtgatagcttctcgttcaggcagtacgcctcttttcttttccagacctgagggaggcggaaatggtgtgaggttcccggggaaaagccaaataggcgatcgcgggagtgctttatttgaagatcaggctatcactgcggtcaatagatttcacaatgtgatggctggacagcctgaggaactctcgaacccgaatggaaacaaccagatatttatgaatcagcgcggctcacatggcgttgtgctggcaaatgcaggttcatcctctgtctctatcaatacggcaacaaaattgcctgatggcaggtatgacaataaagctggagcgggttcatttcaagtgaacgatggtaaactgacaggcacgatcaatgccaggtctgtagctgtgctttatcctgatgatattgcaaaagcgcctcatgttttccttgagaattacaaaacaggtgtaacacattctttcaatgatcaactgacgattaccttgcgtgcagatgcgaatacaacaaaagccgtttatcaaatcaataatggaccagacgacaggcgtttaaggatggagatcaattcacaatcggaaaaggagatccaatttggcaaaacatacaccatcatgttaaaaggaacgaacagtgatggtgtaacgaggaccgagaaatacagttttgttaaaagagatccagcgtcggccaaaaccatcggctatcaaaatccgaatcattggagccaggtaaatgcttatatctataaacatgatgggagccgagtaattgaattgaccggatcttggcctggaaaaccaatgactaaaaatgcagacggaatttacacgctgacgctgcctgcggacacggatacaaccaacgcaaaagtgatttttaataatggcagcgcccaagtgcccggtcagaatcagcctggctttgattacgtgctaaatggtttatataatgactcgggcttaagcggttctcttccccattgagggcaaggctagacgggacttaccgaaagaaaccatcaatgatggtttcttttttgttcataaatcagacaaaacttttctcttgcaaaagtttgtgaagtgttgcacaatataaatgtgaaatacttcacaaacaaaaagacatcaaagagaaacataccctgcaaggatgctgatattgtctgcatttgcgccggagcaaaccaaaaacctggtgagacacgccttgaattagtagaaaagaacttgaagattttcaaaggcatcgttagtgaagtcatggcgagcggatttgacggcattttcttagtcgcgacgcgaggctggatggccttccccattatgattcttctcgcttccggcggcatcgggatgcccgcgttgcaggccatgctgtccaggcaggtagatgacgaccatcagggacagcttcaaggatcgctcgcggctcttaccagcctaacttcgatcactggaccgctgatcgtcacggcgatttatgccgcctcggcgagcacatggaacgggttggcatggattgtaggcgccgccctataccttgtctgcctccccgcgttgcgtcgcggtgcatggagccgggccacctactgaagtggatttctttaagagctcctttaacttcctcaccagtagttgtatcggtaccataagtagaagcagcaacccaagtagctttaccagcatccggttcaaccagcatagtaagaatcttactggacatcggcagttcttcgaacagtgcgccaactaccagctctttctgcagttcattcagggcaccggagaacctgcgtgcaatccatcttgttcaatcatgcgaaacgatcctcatcctgtctcttgatccatggattacgcgttaacccgggcccgcggatgcatatgatcagatcttaaggcctaggtctagaggatcgatctgtataataaagaataattattaatctgtagacaaattgtgaaaggatgtacttaaacgctaacggtcagctttattgaacagtaatttaagtatatgtccaatctagggtaagtaaattgagtatcaatataaactttatatgaacataatcaacgaggtgaaatcatgagcaatttgattaacggaaaaataccaaatcaagcgattcaaacattaaaaatcgtaaaagatttatttggaagttcaatagttggagtatatctatttggttcagcagtaaatggtggtttacgcattaacagcgatgtagatgttctagtcgtcgtgaatcatagtttacctcaattaactcgaaaaaaactaacagaaagactaatgactatatcaggaaagattggaaatacggattctgttagaccacttgaagttacggttataaataggagtgaagttgtcccttggcaatatcctccaaaaagagaatttatatacggtgagtggctcaggggtgaatttgagaatggacaaattcaggaaccaagctatgatcctgatttggctattgttttagcacaagcaagaaagaatagtatttctctatttggtcctgattcttcaagtatacttgtctccgtacctttgacagatattcgaagagcaattaaggattctttgccagaactaattgaggggataaaaggtgatgagcgtaatgtaattttaaccctagctcgaatgtggcaaacagtgactactggtgaaattacctcgaaagatgtcgctgcagaatgggctatacctcttttacctaaagagcatgtaactttactggatatagctagaaaaggctatcggggagagtgtgatgataagtgggaaggactatattcaaaggtgaaagcactcgttaagtatatgaaaaattctatagaaacttctctcaattaggctaattttattgcaataacaggtgcttacttttctggagttctttagcaaatttttttattagctgaacttagtattagtggccatactcctccaatccaaagctatttagaaagattactatatcctcaaacaggcggtaaccggcctcttcatcgggaatgcgcgcgaccttcagcatcgccggcatgtccccctggcggacgggaagtatccagctcgaggtcgggccgcgttgctggcgtttttccataggctccgcccccctgacgagcatcacaaaaatcgacgctcaagtcagaggtggcgaaacccgacaggactataaagataccaggcgtttccccctggaagctccctcgtgcgctctcctgttccgaccctgccgcttaccggatacctgtccgcctttctcccttcgggaagcgtggcgctttctcatagctcacgctgtaggtatctcagttcggtgtaggtcgttcgctccaagctgggctgtgtgcacgaaccccccgttcagcccgaccgctgcgccttatccggtaactatcgtcttgagtccaacccggtaagacacgacttatcgccactggcagcagccactggtaacaggattagcagagcgaggtatgtaggcggtgctacagagttcttgaagtggtggcctaactacggctacactagaaggacagtatttggtatctgcgctctgctgaagccagttaccttcggaaaaagagttgatagctcttgatccggcaaacaaaccaccgctggtagcggtggtttttttgtttgcaagcagcagattacgcgcagaaaaaaaggatctcaagaagatcctttgatcttttctacggggtctgacgctcagtggaacgaaaactcacgttaagggattttggtcatgagattatcaaaaaggatcttcacctagatccttttaaattaaaaatgaagttttaaatcaatctaaagtatatatgagtaaacttggtctgacagttaccaatgcttaatcagtgaggcacctatctcagcgatctgtctatttcgttcatccatagttgcctgactccccgtcgtgtagataactacgatacgggagggcttaccatctggccccagtgctgcaatgataccgcgagacccacgctcaccggctccagatttatcagcaataaaccagccagccggaagggccgagcgcagaagtggtcctgcaactttatccgcctccatccagtctattaattgttgccgggaagctagagtaagtagttcgccagttaatagtttgcgcaacgttgttgccattgctgcaggcatcgtggtgtcacgctcgtcgtttggtatggcttcattcagctccggttcccaacgatcaaggcgagttacatgatcccccatgttgtgcaaaaaagcggttagctccttcggtcctccgatcgttgtcagaagtaagttggccgcagtgttatcactcatggttatggcagcactgcataattctcttactgtcatgccatccgtaagatgcttttctgtgactggtgagtactcaaccaagtcattctgagaatagtgtatgcggcgaccgagttgctcttgcccggcgtcaacacgggataataccgcgccacatagcagaactttaaaagtgctcatcattggaaaacgttcttcggggcgaaaactctcaaggatcttaccgctgttgagatccagttcgatgtaacccactcgtgcacccaactgatcttcagcatcttttactttcaccagcgtttctgggtgagcaaaaacaggaaggcaaaatgccgcaaaaaagggaataagggcgacacggaaatgttgaatactcatactcttcctttttcaatattattgaagcatttatcagggttattgtctcatgagcggatacatatttgaatgtatttagaaaaataaacaaataggggttccgcgcacatttccccgaaaagtgccacctgacgtctaagaaaccattattatcatgacattaacctataaaaataggcgtatcacgaggccctttcgtcttcaagaa

SEQ ID NO: 223 - DNA, 20 bp, synthetic
  primer (1)..(20): primer E257
ctgagtcaatttcatcaagg

SEQ ID NO: 224 - DNA, 22 bp, synthetic
  primer (1)..(22): priomer E258
cagaagaaaacattctcgaagc

SEQ ID NO: 225 - DNA, 20 bp, synthetic
  primer (1)..(20): primer E261
gaggtcgcaactgaaaaagc

SEQ ID NO: 226 - DNA, 20 bp, synthetic
  primer (1)..(20): primer E262
atgttcagtctccttactcc

SEQ ID NO: 227 - DNA, 30 bp, synthetic
  primer (1)..(30): primer E372
attataacaugtattcacgaacgaaaatcg

SEQ ID NO: 228 - DNA, 35 bp, synthetic
  primer (1)..(35): primer E373
atcagatttuagaaaacaataaacccttgcatagg

SEQ ID NO: 229 - DNA, 20 bp, synthetic
  primer (1)..(20): primer E374
aaaatctgauacggggcagg

SEQ ID NO: 230 - DNA, 37 bp, synthetic
  primer (1)..(37): primer E375
atgttataauacccattagttcaacaaacgaaaattg